European Patent Specification EP 3 468 573 B1, published August 9, 2023. Title: TREATMENT OF CLOSTRIDIUM DIFFICILE INFECTION. Applicant: Vedanta Biosciences, Inc. Application Not Yet Assigned. The sequence listing filed with the application follows.

SEQUENCE LISTING (159 sequences)

SEQ ID NO: 1 - DNA, 210 bp, Artificial Sequence
  Synthetic Polynucleotide
gcccggagcagttgatgtgaaggatgggtcacctgtggactgcattggaactgtcatacttgagtgccggagggtaagcggaattcctagtgtagcggtgaaatgcgtagatattaggaggaacaccagtggcgaaggcggcttactggacggtaactgacgttgaggctcgaaagcgtggggagcaaacaggattagataccctggtaa

SEQ ID NO: 2 - DNA, 184 bp, Artificial Sequence
  Synthetic Polynucleotide
ctaaccgtggaggtcattggaaactggtcaacttgagtgcagaagagggaagtggaattccatgtgtagcggtgaaatgcgtagagatatggaggaacaccagtggcgaaggcggcttcctggtctgtaactgacactgaggcgcgaaagcgtggggggcaaacaggattagatcccccggtaa

SEQ ID NO: 3 - DNA, 196 bp, Artificial Sequence
  Synthetic Polynucleotide
atgaaagccggggctcaaccccggtactgctttggaaactgtttgacttgagtgcttgagaggtaagtggaattcctagtgtagcgggaaatgtttagatattaggaggacaccagtggcgaaggcggcttactggactgtaactgacgttgtggctcgatttgtggggagcaaacaggattatatcccctggtaa

SEQ ID NO: 4 - DNA, 211 bp, Artificial Sequence
  Synthetic Polynucleotide
cggaaggtctgatgtgaaggttggggcttaccccggactgcattggaaactgtttttctagagtgcccgagaggtaagcggaattcctagtgtagcggtgaaatgctttagatattaggaggaacaccagtggcgaaggcggcttactggacggtaactgacgttgaggctcgaaagcgtggggagcaaacaggattagataccctggtaa

SEQ ID NO: 5 - DNA, 207 bp, Artificial Sequence
  Synthetic Polynucleotide
cgatgtctgagtgaaggctggggcttaccccaggactgcattggaactgtttttctagagtgccggagaggtaagcggaattcctagtgtagcggtgaaatgcgtagatattaggaggaacaccagtggcgaaggcggcttactggacggtaactgacgttgaggctcgaaagcgtggggagcaaacaggattagataccctggtaa

SEQ ID NO: 6 - DNA, 179 bp, Artificial Sequence
  Synthetic Polynucleotide
ttaaccaagaagtgcattggaactgtcagacttgggggaaaaaaagacagtgcaactccatgtgtagcggtggaatgctccatatatatggaagaacaccagtggcgaaggcggctgtctggtctgcaactgacgctgaggctcgaattcatgggtaagaaagtattagtcccttgtaa

SEQ ID NO: 7 - DNA, 214 bp, Artificial Sequence
  Synthetic Polynucleotide
acccgcttggtctgaggtgaggctggggcttaaccccaggactgcattggaaactgttgttctagagtgccggagaggtaagcggaattcctagtgtagcggtgaaatgcgtagatattaggaggaacaccagtggcgaaggcggcttactggacggtaactgacgttgaggctcgaaagcgtggggagcaaacaggattagataccctggtaa

SEQ ID NO: 8 - DNA, 196 bp, Artificial Sequence
  Synthetic Polynucleotide
taggctggggcttaaccccaggactgcattggaaactgtttttctagagtgccggagaggtaagcggaattcctagtgtagcggtgaaatgcgtagatattaggaggaacaccagtggcgaaggcggcttactggacggtaactgacgttgaggctcgaaagcgtggggagcaaacaggattagataccctggtaa

SEQ ID NO: 9 - DNA, 297 bp, Artificial Sequence
  Synthetic Polynucleotide
ttgcattggacactatgtcagctgagtgtcggagaggtaagtggaattcctagtgtagcggtgaaatgcgtagatattaggaggaacaccagtggcgaaggcggcttactgcacgttttctgacgttgaggctcgaaatcgtggggagcaaacaaaaatagataccctggtagtccacgccgtaaacgatgcatactaggtgtcgggtggcaaagccattcggtgccgcagcaaacgcaataagtatgccacctggggagtacgttcgcaagaatgaaactcaaataaattgacgga

SEQ ID NO: 10 - DNA, 209 bp, Artificial Sequence
  Synthetic Polynucleotide
cccgtcgtagatgtgaactgggggctcacctccagcctgcatttgaaactgtagttcttgagtgctggagaggcaatcggaattccgtgtgtagcggtgaaatgcgtagatatacggaggaacaccagtggcgaaggcggattgctggacagtaactgacgctgaggcgcgaaagcgtggggagcaaacaggattagataccctcataa

SEQ ID NO: 11 - DNA, 401 bp, Artificial Sequence
  Synthetic Polynucleotide
acctgatgcagcgacgccgcgtgagtgaagaagtatttcggtatgtaaagctctatcagcagggaagaaaaaagacggtacctgactaagaagccccggctaactacgtgccagcagccgcggtaatacgtagggggcaagcgttatccggaattactgggtgtaaagggtgcgtaggtggcatggtaagtcagaagtgaaagcccggggcttaaccccgggactgcttttgaaactgtcatgctggagtgcaggagaggtaagcggaattcctagtgtagcggtgaaatgcgtagatattaggaggaacaccagtggcgaaggcggcttactggactgtcactgacactgatgcacgaaagcgtggggagcaaacaggattagataccctggaagtccat

SEQ ID NO: 12 - DNA, 355 bp, Artificial Sequence
  Synthetic Polynucleotide
atgggagcgtagatggcgactgggccatatgtgacagccctggtctcaaccccttaactgcatttggaactgagtggctggagtgtcggagaggcaggcggaattcctagtgtagcggtgaaatgcgtagatattaggaggaacaccagtggcgaaggcggcctgctggacgatgactgacgttgaggctcgaaagcgtggggagcaaacaggattagataccctggtagtccacgccgtaaacgatgactactaggtgtcgggtggcaaggacattcggtgccgcagcaaacgcaataagtagtccacctggggagtacgttcgcaagaatgaaactcaaaggaaattgacgga

SEQ ID NO: 13 - DNA, 197 bp, Artificial Sequence
  Synthetic Polynucleotide
cgcagcggagtgtatcctaggctcacctggctgctttcgaactggttttctagatcgtgtagagggggagattcctggtgtagcgtgaaatgcgtagatatctggaggaacaccagtggcgaaggcggcctcctggacggcaactgacgttgaggctcgaaagtgtggggagcaaacaggattagataccctggtaa

SEQ ID NO: 14 - DNA, 1522 bp, Artificial Sequence
  Synthetic Polynucleotide
tcaaagagtttgatcctggctcaggacgaacgctggcggcgcgcctaacacatgcaagtcgaacggagcttacgttttgaagttttcggatggacgaatgtaagcttagtggcggacgggtgagtaacacgtgagcaacctgcctttcagagggggataacagccggaaacggctgctaataccgcatgatgttgcgggggcacatgcccctgcaaccaaaggagcaatccgctgaaagatgggctcgcgtccgattagccagttggcggggtaacggcccaccaaagcgacgatcggtagccggactgagaggttgaacggccacattgggactgagacacggcccagactcctacgggaggcagcagtgggggatattgcacaatgggcgaaagcctgatgcagcgacgccgcgtgagggaagacggtcttcggattgtaaacctctgtctttggggaagaaaatgacggtacccaaagaggaagctccggctaactacgtgccagcagccgcggtaatacgtagggagcaagcgttgtccggaattactgggtgtaaagggagcgtaggcgggatggcaagtagaatgttaaatccatcggctcaaccggtggctgcgttctaaactgccgttcttgagtgaagtagaggcaggcggaattcctagtgtagcggtgaaatgcgtagatattaggaggaacaccagtggcgaaggcggcctgctgggctttaactgacgctgaggctcgaaagcgtggggagcaaacaggattagataccctggtagtccacgccgtaaacgatgattactaggtgtggggggactgaccccttccgtgccgcagttaacacaataagtaatccacctggggagtacggccgcaaggttgaaactcaaaggaattgacgggggcccgcacaagcagtggagtatgtggtttaattcgaagcaacgcgaagaaccttaccaggtcttgacatcggatgcatagcctagagataggtgaagcccttcggggcatccagacaggtggtgcatggttgtcgtcagctcgtgtcgtgagatgttgggttaagtcccgcaacgagcgcaacccttattattagttgctacgcaagagcactctaatgagactgccgttgacaaaacggaggaaggtggggatgacgtcaaatcatcatgccccttatgacctgggctacacacgtactacaatggcactaaaacagagggcggcgacaccgcgaggtgaagcgaatcccgaaaaagtgtctcagttcagattgcaggctgcaacccgcctgcatgaagtcggaattgctagtaatcgcggatcagcatgccgcggtgaatacgttcccgggccttgtacacaccgcccgtcacaccatgggagtcggtaacacccgaagccagtagcctaaccgcaaggggggcgctgtcgaaggtgggattgatgactggggtgaagtcgtaacaaggtagccgtatcggaaggtgcggctggatcacctccttt

SEQ ID NO: 15 - DNA, 1529 bp, Artificial Sequence
  Synthetic Polynucleotide
tacgagagtttgatcctggctcaggatgaacgctggcggcgtgcctaacacatgcaagtcgagcgaagcgctgttttcagaatcttcggaggaagaggacagtgactgagcggcggacgggtgagtaacgcgtgggcaacctgcctcatacagggggataacagttagaaatgactgctaataccgcataagcgcacaggaccgcatggtgtagtgtgaaaaactccggtggtatgagatggacccgcgtctgattaggtagttggtggggtaaaggcctaccaagccgacgatcagtagccgacctgagagggtgaccggccacattgggactgagacacggcccaaactcctacgggaggcagcagtggggaatattgcacaatgggggaaaccctgatgcagcgacgccgcgtgaaggaagaagtatttcggtatgtaaacttctatcagcagggaagaagatgacggtacctgagtaagaagcaccggctaaatacgtgccagcagccgcggtaatacgtatggtgcaagcgttatccggatttactgggtgtaaagggagcgtagacggataggcaagtctggagtgaaaacccagggctcaaccctgggactgctttggaaactgcagatctggagtgccggagaggtaagcggaattcctagtgtagcggtgaaatgcgtagatattaggaggaacaccagtggcgaaggcggcttactggacggtgactgacgttgaggctcgaaagcgtggggagcaaacaggattagataccctggtagtccacgccgtaaacgatgactactaggtgtcggtgtgcaaagcacatcggtgccgcagcaaacgcaataagtagtccacctggggagtacgttcgcaagaatgaaactcaaaggaattgacggggacccgcacaagcggtggagcatgtggtttaattcgaagcaacgcgaagaaccttacctggtcttgacatccggatgacgggcgagtaatgtcgccgtcccttcggggcatccgagacaggtggtgcatggttgtcgtcagctcgtgtcgtgagatgttgggttaagtcccgcaacgagcgcaacccttatcttcagtagccagcatataaggtgggcactctggagagactgccagggagaacctggaggaaggtggggatgacgtcaaatcatcatgccccttatggccagggctacacacgtgctacaatggcgtaaacaaagggaagcgagagggtgacctggagcgaatcccaaaaataacgtctcagttcggattgtagtctgcaactcgactacatgaagctggaatcgctagtaatcgcggatcagcatgccgcggtgaatacgttcccgggtcttgtacacaccgcccgtcacaccatgggagtcagtaacgcccgaagccagtgacccaaccttagaggagggagctgtcgaaggcgggacggataactggggtgaagtcgtaacaaggtagccgtatcggaaggtgcggctggatcacctccttt

SEQ ID NO: 16 - DNA, 1527 bp, Artificial Sequence
  Synthetic Polynucleotide
atgagagtttgatcctggctcaggatgaacgctggcggcgtgcctaacacatgcaagtcgaacgaagcgatttaacggaagttttcggatggaagttgaattgactgagtggcggacgggtgagtaacgcgtgggtaacctgccttgtactgggggacaacagttagaaatgactgctaataccgcataagcgcacagtatcgcatgatacagtgtgaaaaactccggtggtacaagatggacccgcgtctgattagctagttggtaaggtaacggcttaccaaggcgacgatcagtagccgacctgagagggtgaccggccacattgggactgagacacggcccaaactcctacgggaggcagcagtggggaatattgcacaatgggcgaaagcctgatgcagcgacgccgcgtgagtgaagaagtatttcggtatgtaaagctctatcagcagggaagaaaatgacggtacctgactaagaagccccggctaactacgtgccagcagccgcggtaatacgtagggggcaagcgttatccggatttactgggtgtaaagggagcgtagacggtaaagcaagtctgaagtgaaagcccgcggctcaactgcgggactgctttggaaactgtttaactggagtgtcggagaggtaagtggaattcctagtgtagcggtgaaatgcgtagatattaggaggaacaccagtggcgaaggcgacttactggacgataactgacgttgaggctcgaaagcgtggggagcaaacaggattagataccctggtagtccacgccgtaaacgatgaatactaggtgttggggagcaaagctcttcggtgccgtcgcaaacgcagtaagtattccacctggggagtacgttcgcaagaatgaaactcaaaggaattgacggggacccgcacaagcggtggagcatgtggtttaattcgaagcaacgcgaagaaccttaccaggtcttgacatcgatccgacgggggagtaacgtccccttcccttcggggcggagaagacaggtggtgcatggttgtcgtcagctcgtgtcgtgagatgttgggttaagtcccgcaacgagcgcaacccttattctaagtagccagcggttcggccgggaactcttgggagactgccagggataacctggaggaaggtggggatgacgtcaaatcatcatgccccttatgatctgggctacacacgtgctacaatggcgtaaacaaagagaagcaagaccgcgaggtggagcaaatctcaaaaataacgtctcagttcggactgcaggctgcaactcgcctgcacgaagctggaatcgctagtaatcgcgaatcagaatgtcgcggtgaatacgttcccgggtcttgtacacaccgcccgtcacaccatgggagtcagtaacgcccgaagtcagtgacccaaccgcaaggagggagctgccgaaggcgggaccgataactggggtgaagtcgtaacaaggtagccgtatcggaaggtgcggctggatcacctccttt

SEQ ID NO: 17 - DNA, 1530 bp, Artificial Sequence
  Synthetic Polynucleotide
atgagagtttgatcctggctcaggatgaacgctggcggcgtgcctaacacatgcaagtcgaacgaagcaattaaaatgaagttttcggatggatttttgattgactgagtggcggacgggtgagtaacgcgtggataacctgcctcacactgggggataacagttagaaatgactgctaataccgcataagcgcacagtaccgcatggtacggtgtgaaaaactccggtggtgtgagatggatccgcgtctgattagccagttggcggggtaacggcccaccaaagcgacgatcagtagccgacctgagagggtgaccggccacattgggactgagacacggcccaaactcctacgggaggcagcagtggggaatattgcacaatgggcgaaagcctgatgcagcgacgccgcgtgagtgaagaagtatttcggtatgtaaagctctatcagcagggaagaaaatgacggtacctgactaagaagccccggctaactacgtgccagcagccgcggtaatacgtagggggcaagcgttatccggatttactgggtgtaaagggagcgtagacggcgaagcaagtctgaagtgaaaacccagggctcaaccctgggactgctttggaaactgttttgctagagtgtcggagaggtaagtggaattcctagtgtagcggtgaaatgcgtagatattaggaggaacaccagtggcgaaggcggcttactggacgataactgacgttgaggctcgaaagcgtggggagcaaacaggattagataccctggtagtccacgccgtaaacgatgaatgctaggtgttggggggcaaagcccttcggtgccgtcgcaaacgcagtaagcattccacctggggagtacgttcgcaagaatgaaactcaaaggaattgacggggacccgcacaagcggtggagcatgtggtttaattcgaagcaacgcgaagaaccttaccaagtcttgacatcctcttgaccggcgtgtaacggcgccttcccttcggggcaagagagacaggtggtgcatggttgtcgtcagctcgtgtcgtgagatgttgggttaagtcccgcaacgagcgcaacccttatccttagtagccagcaggtaaagctgggcactctagggagactgccagggataacctggaggaaggtggggatgacgtcaaatcatcatgccccttatgatttgggctacacacgtgctacaatggcgtaaacaaagggaagcaagacagtgatgtggagcaaatcccaaaaataacgtcccagttcggactgtagtctgcaacccgactacacgaagctggaatcgctagtaatcgcgaatcagaatgtcgcggtgaatacgttcccgggtcttgtacacaccgcccgtcacaccatgggagtcagcaacgcccgaagtcagtgacccaactcgcaagagagggagctgccgaaggcggggcaggtaactggggtgaagtcgtaacaaggtagccgtatcggaaggtgcggctggatcacctccttt

SEQ ID NO: 18 - DNA, 1528 bp, Artificial Sequence
  Synthetic Polynucleotide
aacgagagtttgatcctggctcaggatgaacgctggcggcgtgcttaacacatgcaagtcgagcgaagcactttggaagattcttcggatgaagacttttgtgactgagcggcggacgggtgagtaacgcgtgggtaacctgcctcatacagggggataacagttagaaatgactgctaataccgcataagaccacggtaccgcatggtacagtggtaaaaactccggtggtatgagatggacccgcgtctgattaggtagttggtggggtaacggcctaccaagccgacgatcagtagccgacctgagagggtgaccggccacattgggactgagacacggcccagactcctacgggaggcagcagtggggaatattgcacaatggaggaaactctgatgcagcgacgccgcgtgaaggatgaagtatttcggtatgtaaacttctatcagcagggaagaaaatgacggtacctgactaagaagccccggctaactacgtgccagcagccgcggtaatacgtagggggcaagcgttatccggatttactgggtgtaaagggagcgtagacggcacggcaagccagatgtgaaagcccggggctcaaccccgggactgcatttggaactgctgagctagagtgtcggagaggcaagtggaattcctagtgtagcggtgaaatgcgtagatattaggaggaacaccagtggcgaaggcggcttgctggacgatgactgacgttgaggctcgaaagcgtggggagcaaacaggattagataccctggtagtccacgccgtaaacgatgactgctaggtgtcgggtggcaaagccattcggtgccgcagctaacgcaataagcagtccacctggggagtacgttcgcaagaatgaaactcaaaggaattgacggggacccgcacaagcggtggagcatgtggtttaattcgaagcaacgcgaagaaccttacctgatcttgacatcccgatgaccgcttcgtaatggaagcttttcttcggaacatcggtgacaggtggtgcatggttgtcgtcagctcgtgtcgtgagatgttgggttaagtcccgcaacgagcgcaacccctatcttcagtagccagcaggttaagctgggcactctggagagactgccagggataacctggaggaaggtggggatgacgtcaaatcatcatgccccttatgaccagggctacacacgtgctacaatggcgtaaacaaagagaagcgaactcgcgagggtaagcaaatctcaaaaataacgtctcagttcggattgtagtctgcaactcgactacatgaagctggaatcgctagtaatcgcagatcagaatgctgcggtgaatacgttcccgggtcttgtacacaccgcccgtcacaccatgggagtcagtaacgcccgaagtcagtgacccaaccgtaaggagggagctgccgaaggtgggaccgataactggggtgaagtcgtaacaaggtagccgtatcggaaggtgcggctggatcacctccttt

SEQ ID NO: 19 - DNA, 1531 bp, Artificial Sequence
  Synthetic Polynucleotide
atcagagagtttgatcctggctcaggatgaacgctggcggcgtgcttaacacatgcaagtcgagcgaagcacttaagtggatctcttcggattgaaacttatttgactgagcggcggacgggtgagtaacgcgtgggtaacctgcctcatacagggggataacagttagaaatggctgctaataccgcataagcgcacaggaccgcatggtctggtgtgaaaaactccggtggtatgagatggacccgcgtctgattagctagttggaggggtaacggcccaccaaggcgacgatcagtagccggcctgagagggtgaacggccacattgggactgagacacggcccagactcctacgggaggcagcagtggggaatattgcacaatgggggaaaccctgatgcagcgacgccgcgtgaaggaagaagtatctcggtatgtaaacttctatcagcagggaagaaaatgacggtacctgactaagaagccccggctaactacgtgccagcagccgcggtaatacgtagggggcaagcgttatccggatttactgggtgtaaagggagcgtagacggaagagcaagtctgatgtgaaaggctggggcttaaccccaggactgcattggaaactgtttttctagagtgccggagaggtaagcggaattcctagtgtagcggtgaaatgcgtagatattaggaggaacaccagtggcgaaggcggcttactggacggtaactgacgttgaggctcgaaagcgtggggagcaaacaggattagataccctggtagtccacgccgtaaacgatgaatactaggtgtcgggtggcaaagccattcggtgccgcagcaaacgcaataagtattccacctggggagtacgttcgcaagaatgaaactcaaaggaattgacggggacccgcacaagcggtggagcatgtggtttaattcgaagcaacgcgaagaaccttaccaagtcttgacatccctctgaccggcccgtaacggggccttcccttcggggcagaggagacaggtggtgcatggttgtcgtcagctcgtgtcgtgagatgttgggttaagtcccgcaacgagcgcaacccctatccttagtagccagcaggtgaagctgggcactctagggagactgccggggataacccggaggaaggcggggacgacgtcaaatcatcatgccccttatgatttgggctacacacgtgctacaatggcgtaaacaaagggaagcgagacagcgatgttgagcaaatcccaaaaataacgtcccagttcggactgcagtctgcaactcgactgcacgaagctggaatcgctagtaatcgcgaatcagaatgtcgcggtgaatacgttcccgggtcttgtacacaccgcccgtcacaccatgggagtcagtaacgcccgaagtcagtgacccaaccttacaggagggagctgccgaaggcgggaccgataactggggtgaagtcgtaacaaggtagccgtatcggaaggtgcggctggatcacctccttt

SEQ ID NO: 20 - DNA, 1528 bp, Artificial Sequence
  Synthetic Polynucleotide
aacgagagtttgatcctggctcaggatgaacgctggcggcgtgcttaacacatgcaagtcgagcgaagcactttggaagattcttcggatgatttcctttgtgactgagcggcggacgggtgagtaacgcgtgggtaacctgcctcatacagggggataacagttagaaatgactgctaataccgcataagaccacggtaccgcatggtacagtggtaaaaactccggtggtatgagatggacccgcgtctgattaggtagttggtggggtaacggcctaccaagccgacgatcagtagccgacctgagagggtgaccggccacattgggactgagacacggcccagactcctacgggaggcagcagtggggaatattgcacaatggaggaaactctgatgcagcgacgccgcgtgaaggatgaagtatttcggtatgtaaacttctatcagcagggaagaaaatgacggtacctgactaagaagccccggctaactacgtgccagcagccgcggtaatacgtagggggcaagcgttatccggatttactgggtgtaaagggagcgtagacggcacggcaagccagatgtgaaagcccggggctcaaccccgggactgcatttggaactgctgagctagagtgtcggagaggcaagtggaattcctagtgtagcggtgaaatgcgtagatattaggaggaacaccagtggcgaaggcggcttgctggacgatgactgacgttgaggctcgaaagcgtggggagcaaacaggattagataccctggtagtccacgccgtaaacgatgactgctaggtgtcgggtggcaaagccattcggtgccgcagctaacgcaataagcagtccacctggggagtacgttcgcaagaatgaaactcaaaggaattgacggggacccgcacaagcggtggagcatgtggtttaattcgaagcaacgcgaagaaccttacctgatcttgacatcccgatgaccgcttcgtaatggaagcttttcttcggaacatcggtgacaggtggtgcatggttgtcgtcagctcgtgtcgtgagatgttgggttaagtcccgcaacgagcgcaacccctatcttcagtagccagcaggttaagctgggcactctggagagactgccagggataacctggaggaaggtggggatgacgtcaaatcatcatgccccttatgaccagggctacacacgtgctacaatggcgtaaacaaagagaagcgaactcgcgagggtaagcaaatctcaaaaataacgtctcagttcggattgtagtctgcaactcgactacatgaagctggaatcgctagtaatcgcagatcagaatgctgcggtgaatacgttcccgggtcttgtacacaccgcccgtcacaccatgggagtcagtaacgcccgaagtcagtgacccaaccgtaaggagggagctgccgaaggtgggaccgataactggggtgaagtcgtaacaaggtagccgtatcggaaggtgcggctggatcacctccttt

SEQ ID NO: 21 - DNA, 1537 bp, Artificial Sequence
  Synthetic Polynucleotide
atggagagtttgatcctggctcaggatgaacgctggcggcatgcctaatacatgcaagtcgaacgaagtttcgaggaagcttgcttccaaagagacttagtggcgaacgggtgagtaacacgtaggtaacctgcccatgtgtccgggataactgctggaaacggtagctaaaaccggataggtatacagagcgcatgctcagtatattaaagcgcccatcaaggcgtgaacatggatggacctgcggcgcattagctagttggtgaggtaacggcccaccaaggcgatgatgcgtagccggcctgagagggtaaacggccacattgggactgagacacggcccaaactcctacgggaggcagcagtagggaattttcgtcaatgggggaaaccctgaacgagcaatgccgcgtgagtgaagaaggtcttcggatcgtaaagctctgttgtaagtgaagaacggctcatagaggaaatgctatgggagtgacggtagcttaccagaaagccacggctaactacgtgccagcagccgcggtaatacgtaggtggcaagcgttatccggaatcattgggcgtaaagggtgcgtaggtggcgtactaagtctgtagtaaaaggcaatggctcaaccattgtaagctatggaaactggtatgctggagtgcagaagagggcgatggaattccatgtgtagcggtaaaatgcgtagatatatggaggaacaccagtggcgaaggcggtcgcctggtctgtaactgacactgaggcacgaaagcgtggggagcaaataggattagataccctagtagtccacgccgtaaacgatgagaactaagtgttggaggaattcagtgctgcagttaacgcaataagttctccgcctggggagtatgcacgcaagtgtgaaactcaaaggaattgacgggggcccgcacaagcggtggagtatgtggtttaattcgaagcaacgcgaagaaccttaccaggccttgacatggaaacaaataccctagagatagggggataattatggatcacacaggtggtgcatggttgtcgtcagctcgtgtcgtgagatgttgggttaagtcccgcaacgagcgcaacccttgtcgcatgttaccagcatcaagttggggactcatgcgagactgccggtgacaaaccggaggaaggtggggatgacgtcaaatcatcatgccccttatggcctgggctacacacgtactacaatggcggccacaaagagcagcgacacagtgatgtgaagcgaatctcataaaggtcgtctcagttcggattgaagtctgcaactcgacttcatgaagtcggaatcgctagtaatcgcagatcagcatgctgcggtgaatacgttctcgggccttgtacacaccgcccgtcaaaccatgggagtcagtaatacccgaagccggtggcataaccgtaaggagtgagccgtcgaaggtaggaccgatgactggggttaagtcgtaacaaggtatccctacgggaacgtggggatggatcacctccttt

SEQ ID NO: 22 - DNA, 476 bp, Artificial Sequence
  Synthetic Polynucleotide
agtaacgcgtgggtaacctgcctcatacagggggataacagttagaaatgactgctaataccgcataagaccacggtaccgcatggtacagtggtaaaaactccggtggtatgagatggacccgcgtctgattaggtagttggtggggtaacggcctaccaagccgacgatcagtagccgacctgagagggtgaccggccacattgggactgagacacggcccagactcctacgggaggcagcagtggggaatattgcacaatggaggaaactctgatgcagcgacgccgcgtgaaggatgaagtatttcggtatgtaaacttctatcagcagggaagaaaatgacggtacctgactaagaagccccggctaactacgtgccagcagccgcggtaatacgtagggggcaagcgttatccggatttactgggtgtaaagggagcgtagacggcacggcaagccagatgtgaaagccc

SEQ ID NO: 23 - DNA, 354 bp, Artificial Sequence
  Synthetic Polynucleotide
caggctggagtgcaggagaggtaagcggaattcctagtgtagcggtgaaatgcgtagatattaggaggaacaccagtggcgaaggcggcttactggactgtaactgacgttgaggctcgaaagcgtggggagcaaacaggattagataccctggtagtccacgcggtaaacgatgattgctaggtgtaggtgggtatggacccatcggtgccgcagctaacgcaataagcaatccacctggggagtacgttcgcaagaatgaaactcaaaggaattgacggggacccgcacaagcggtggagcatgtggtttaattcgaagcaacgcgaagaaccttaccaagtcttgacatcc

SEQ ID NO: 24 - DNA, 190 bp, Artificial Sequence
  Synthetic Polynucleotide
ccggggctcaccccgggactgcatttggaactgctgagctagagtgtcggagaggcaagtggaattcctagtgtagcggtgaaatgcgtagatattaggaggaacaccagtggcgaaggcggcttgctggacgatgactgacgttgaggctcgaaagcgtggggagcaaacaggattagataccctggta

SEQ ID NO: 25 - DNA, 190 bp, Artificial Sequence
  Synthetic Polynucleotide
agggtcaacccctggactgcattggaaactgtcaggctggagtgccggagaggtaagcggaattcctagtgtagcggtgaaatgcgtagatattaggaggaacaccagtggcgaaggcggcttactggacggtaactgacgttgatgctcgaaagcgtggggagcaaacaggattagataacctggtaaa

SEQ ID NO: 26 - DNA, 209 bp, Artificial Sequence
  Synthetic Polynucleotide
gggaagtcggtcttaagtgcggggcttaaccccgtgaggggaccgaaactgtgaagctcgagtgtcggagaggaaagcggaattcctagtgtagcggtgaaatgcgtagatattaggaggaacaccagtggcgaaagcggctttctggacgacaactgacgctgaggcgcgaaagccaggggagcaaacgggattagataccccagtaa

SEQ ID NO: 27 - DNA, 203 bp, Artificial Sequence
  Synthetic Polynucleotide
tagtctgagtgatgcggggcttaaccccgtatggcgttggatactggaagtcttgagtgcaggagaggaaaggggaattcccagtgtagcggtgaaatgcgtagatattgggaggaacaccagtggcgaaggcgcctttctggactgtgtctgacgctgagatgcgaaagccagggtagcaaacgggattagataccacggta

SEQ ID NO: 28 - DNA, 207 bp, Artificial Sequence
  Synthetic Polynucleotide
gatagtcggtcttaagtgcggggcttaccccgtgaggggaccgaaactgtgaagctcgagtgtcggagaggaaagcggaattcctagtgtagcggtgaaatgcgtagatattaggaggaacaccagtggcgaaagcggctttctggacgacaactgacgctgaggcgcgaaagccaggggagcaaacgggattagataccacggtaa

SEQ ID NO: 29 - DNA, 424 bp, Artificial Sequence
  Synthetic Polynucleotide
cgtttgctccacgctttcgagcctcacgtcagttaccgtccagtaagccgccttcgccactggtgttcctcctaatatctacgcatttcaccgctacactaggaattccgcttacctctccggtactctagattgacagtttccaatgcagtcccggggttgagccccgggttttcacatcagacttgccactccgtctacgctccctttacacccagtaaatccggataacgcttgcaccatacgtattaccgcggctgctggcacgtatttagccggtgcttcttagtcaggtaccgtcattttcttccctgctgatagagctttacataccgaaatacttcatcgctcacgcggcgtcgctgcatcagggtttcccccattgtgcaatattccccactgctgcctcccgtaggagtttgga

SEQ ID NO: 30 - DNA, 441 bp, Artificial Sequence
  Synthetic Polynucleotide
tgtcacactttcgagcatcagcgtcagttacagtccagtaagctgccttcgcaatcggagttcttcgtgatatctaagcatttcaccgctacaccacgaattccgcctacctctactgcactcaagacgaccagtatcaactgcaattttacggttgagccgcaaactttcacagctgacttaatagtccgcctacgctccctttaaacccaataaatccggataacgcttggatcctccgtattaccgcggctgctggcacggagttagccgatccttattcgtatggtacatacaaaaagccacacgtggctcactttattcccatataaaagaagtttacaacccatagggcagtcatccttcacgctacttggctggttcagactctcgtccattgaccaatattcctcactgctgcctcccgtaggtagtttggaa

SEQ ID NO: 31 - DNA, 422 bp, Artificial Sequence
  Synthetic Polynucleotide
ccgttgtcacgctttcgtgctcagtgtcagtttcagtccagtaagccgccttcgccactgatgttcctcctaatatctacgcatttcaccgctacactaggaattccgcttacctctcctgcactccagtctgacagtttcaaaagcagtcccagagttaagccctgggttttcacttctgacttgccataccacctacgcaccctttacacccagtaattccggataacgcttgccccctacgtattaccgcggctgctggcacgtagttagccggggcttcttagtcaggtaccgtcattttcttccctgctgatagagctttacataccgaaatacttcttcactcacgcggcgtcgctgcatcagggttccccccattgtgcaatattccccactgctgcctcccgtggaagtttgga

SEQ ID NO: 32 - DNA, 424 bp, Artificial Sequence
  Synthetic Polynucleotide
gcgaatgtcacgcattcgagcctcacgtcagttaccgtccagtaagccgccttcgccactggtgttcctcctaatatctacgcatttcaccgctacactaggaattccgcttacctctccggcactcaagactaacagtttccaatgcagtccaggggttgagcccccgcctttcacatcagacttgccagtccgtctacgctccctttacacccagtaaatccggataacgcttgccccctacgtattaccgcggctgctggcacgtagttagccggggcttcttagtcaggtaccgtcactatcttccctgctgatagaagtttacataccgagatacttcttccttcacgcggcgtcgctgcatcagggtttcccccattgtgcaatattccccactgctgcctcccgtgggagtttggaa

SEQ ID NO: 33 - DNA, 422 bp, Artificial Sequence
  Synthetic Polynucleotide
tgctcacgctttcgcgctcagcgtcagttactgtccagcaatccgccttcgccactggtgttcctccgtatatctacgcatttcaccgctacacacggaattccgattgcctctccagcactcaagaactacagtttcaaatgcaggctggaggttgagcccccagttttcacatctgacttgcaatcccgcctacacgccctttacacccagtaaatccggataacgcttgccacctacgtattaccgcggctgctggcacgtagttagccgtggcttattcgtcaggtaccgtcatttgtttcgtccctgacaaaagaagtttacaacccgaaagccttcttccttcacgcggcgttgctgggtcaggcttgcgcccattgcccaatattccccactgctgcctcccgtggtagtttgga

SEQ ID NO: 34 - DNA, 419 bp, Artificial Sequence
  Synthetic Polynucleotide
tgtccacgctttcgagctcagcgtcagttatcgtccagtaagccgccttcgccactggtgttcctcctaatatctacgcatttcaccgctacactaggaattccgcttacccctccgacactctagtacgacagtttccaatgcagtaccggggttgagccccgggctttcacatcagacttgccgcaccgcctgcgctccctttacacccagtaaatccggataacgcttgcaccatacgtattaccgcggctgctggcacgtatttagccggtgcttcttagtcaggtaccgtcattatcttccctgctgatagagctttacataccgaaatacttcttcgctcacgcggcgtcgctgcatcaggctttcgcccattgtgcaatattccccactgctgactcccgtaggagtttgga

SEQ ID NO: 35 - DNA, 424 bp, Artificial Sequence
  Synthetic Polynucleotide
cgtttctccacgcttcgcgctcagcgtcagttactgtccagcaatccgccttcgccactggtgttcctccgtatatctacgcatttcaccgctacacacggaattccgattgcctctccagcactcaagaactacagtttcaaatgcaggctggaggttgagcccccagttttcacatctgacttgcaatcccgcctacacgccctttacacccagtaaatccggataacgcttgccacctacgtattaccgcggctgctggcacgtagttagccgtggcttattcgtcaggtaccgtcatttgtttcgtccccgacaaaagaagtttacaacccgaaagccttcttccttcacgcggcgttgctgggtcaggcttgcgcccattgcccaatattccccactgctgcctccctgggaagtttgg

SEQ ID NO: 36 - DNA, 445 bp, Artificial Sequence
  Synthetic Polynucleotide
atgtcctgacttcgcgcctcagcgtcagttgtcgtccagaaagccgctttcgccactggtgttcctcctaatatctacgcatttcaccgctacactaggaattccgctttcctctccgacactcgagcttcacagtttcggtcccctcacggggttaagccccgcacttttaagaccgacttgcgatgccgcctgcgcgccctttacgcccaataattccggacaacgcttgccacctacgtattaccgcggctgctggcacgtagttagccgtggctttctcttacggtaccgtcagggataacgggtattgaccgctatcctgttcgtcccatataacagaactttacaacccgaaggccgtcatcgttcacgcggcgttgctccgtcagactttcgtccattgcggaagattccccactgctgcctccctgggaagtttgga

SEQ ID NO: 37 - DNA, 421 bp, Artificial Sequence
  Synthetic Polynucleotide
gtttgctcacgctttcgagctcagcgtcagttatcgtccagtaagccgccttcgccactggtgttcctcctaatatctacgcatttcaccgctacactaggaattccgcttacccctccgacactctagtacgacagtttccaatgcagtaccggggttgagccccgggctttcacatcagacttgccgcaccgcctgcgctccctttacacccagtaaatccggataacgcttgcaccatacgtattaccgcggctgctggcacgtatttagccggtgcttcttagtcaggtaccgtcattatcttccctgctgatagagctttacataccgaaatacttcttcgctcacgcggcgtcgctgcatcaggctttcgcccattgtgcaatattccccactgctgcctcccgtaggagtttgg

SEQ ID NO: 38 - DNA, 424 bp, Artificial Sequence
  Synthetic Polynucleotide
cgttgctcacgcattcgagcctcagcgtcagttaagcccagtaagccgccttcgccactgatgttcctcctaatatctacgcatttcaccgctacactaggaattccgcttacctctacttcactcaagaaccacagtttcaaatgcagtttatgggttaagcccatagttttcacatctgacttgcgatcccgcctacgctccctttacacccagtaattccggacaacgctcgctccctacgtattaccgcggctgctggcacgtagttagccggagcttcctcctcaggtaccgtcttttttcgtccctgaagacagaggtttacaatcctaaaaccttcttccctcacgcggcatcgctgcatcagagtttcctccattgtgcaatattccccactgctgcctcccgtaggagtttggaa

SEQ ID NO: 39 - DNA, 189 bp, Artificial Sequence
  Synthetic Polynucleotide
tgggcttacccataaactgcatttgaaactgtggttcttgagtgaagtagaggtaagcggaattcctagtgtagcggtgaaatgcgtagatattaggaggaacatcagtggcgaaggcggcttactgggctttaactgacgctgaggctcgaaagcgtggggagcaaacaggattagatacccaagtaa

SEQ ID NO: 40 - DNA, 414 bp, Artificial Sequence
  Synthetic Polynucleotide
gtcagcatcgagctcacgtcagttaccgtccagtaagccgccttcgccactggtgttcctcctaatatctacgcatttcaccgctacactaggaattccgcttacctctccggtactctagattgacagtttccaatgcagtcccggggttgagccccgggttttcacatcagacttgccactccgtctacgctccctttacacccagtaaatccggataacgcttgcaccatacgtattaccgcggctgctggcacgtatttagccggtgcttcttagtcaggtaccgtcattttcttccctgctgatagagctttacataccgaaatacttcatcgctcacgcggcgtcgctgcatcagggtttcccccattgtgcaatattccccactgctgcctcccgagggagtttgga

SEQ ID NO: 41 - DNA, 191 bp, Artificial Sequence
  Synthetic Polynucleotide
tcatcgcttacggtggatctgcgccgggtacgggcgggctggagtgcggtaggggagactggaattcccggtgtaacggtggaatgtgtagatatcgggaagaacaccgatggcgaaggcaggtctctgggccgtcactgacgctgaggagcgaaagcgtggggagcgaacaggattagatacaacggtaa

SEQ ID NO: 42 - DNA, 196 bp, Artificial Sequence
  Synthetic Polynucleotide
tgaacccagggcttaactctgggactgcttttgaactgtcagactggagtgcaggagaggtaagcggaattcctagtgtagcggtgaaatgcgtagatattaggaggaacatcagtggcgaaggcggcttactggactgaaactgacactgaggcacgaaagcgtggggagcaaacaggattagataccatggtaa

SEQ ID NO: 43 - DNA, 192 bp, Artificial Sequence
  Synthetic Polynucleotide
accagggcttaactctgggactgcttttgaactgtcagactggagtgcaggagaggtaagcggaattcctagtgtagcggtgaaatgcgtagatattaggaggaacatcagtggcgaaggcggcttactggactgaaactgacactgaggcacgaaagcgtggggagcaaacaggattagataccctggtaa

SEQ ID NO: 44 - DNA, 195 bp, Artificial Sequence
  Synthetic Polynucleotide
gaacccagggcttaactctgggactgcttttgaactgtcagactggagtgcaggagaggtaagcggaattcctagtgtagcggtgaaatgcgtagatattaggaggaacatcagtggcgaaggcggcttactggactgaaactgacactgaggcacgaaagcgtggggagcaaacaggattagataccccggtaa

SEQ ID NO: 45 - DNA, 418 bp, Artificial Sequence
  Synthetic Polynucleotide
gagtcagctttcgagctcagcgtcagttatcgtccagtaagccgccttcgccactggtgttcctcctaatatctacgcatttcaccgctacactaggaattccgcttacccctccgacactctagtacgacagtttccaatgcagtaccggggttgagccccgggctttcacatcagacttgccgcaccgcctgcgctccctttacacccagtaaatccggataacgcttgcaccatacgtattaccgcggctgctggcacgtatttagccggtgcttcttagtcaggtaccgtcattatcttccctgctgatagagctttacataccgaaatacttcttcgctcacgcggcgtcgctgcatcaggctttcgcccattgtgcaatattccccactgctgcctcccgagggagtttgga

SEQ ID NO: 46 - DNA, 416 bp, Artificial Sequence
  Synthetic Polynucleotide
tgtcagctttcgagctcacgtcagttaccgtccagtaagccgccttcgccactggtgttcctcctaatatctacgcatttcaccgctacactaggaattccgcttacctctccggtactctagattgacagtttccaatgcagtcccggggttgagccccgggttttcacatcagacttgccactccgtctacgctccctttacacccagtaaatccggataacgcttgcaccatacgtattaccgcggctgctggcacgtatttagccggtgcttcttagtcaggtaccgtcattttcttccctgctgatagagctttacataccgaaatacttcatcgctcacgcggcgtcgctgcatcagggtttcccccattgtgcaatattccccactgctgcctcccgtaggagtttgga

SEQ ID NO: 47 - DNA, 400 bp, Artificial Sequence
  Synthetic Polynucleotide
cacgtcagttaccgtccagtaagccgccttcgccactggtgttcctcctaatatctacgcatttcaccgctacactaggaattccgcttacctctccggcactcaagacgggcagtttccaatgcagtcccggggttgagccccagcctttcacatcagacttgtccatccgtctacgctccctttacacccagtaaatccggataacgcttgccccctacgtattaccgcggctgctggcacgtagttagccggggcttcttagtcaggtaccgtcattttcttccctgctgatagaagtttacataccgagatacttcttccttcacgcggcgtcgctgcatcagggtttcccccattgtgcaatattccccactgctgcctcccgtaggagtttggg

SEQ ID NO: 48 - DNA, 416 bp, Artificial Sequence
  Synthetic Polynucleotide
gtcagctttcgagctcacgtcagttaccgtccagtaagccgccttcgccactggtgttcctcctaatatctacgcatttcaccgctacactaggaattccgcttacctctccggtactctagattgacagtttccaatgcagtcccggggttgagccccgggttttcacatcagacttgccactccgtctacgctccctttacacccagtaaatccggataacgcttgcaccatacgtattaccgcggctgctggcacgtatttagccggtgcttcttagtcaggtaccgtcattttcttccctgctgatagagctttacataccgaaatacttcatcgctcacgcggcgtcgctgcatcagggtttcccccattgtgcaatattccccactgctgcctcccgtggggagtttgga

SEQ ID NO: 49 - DNA, 421 bp, Artificial Sequence
  Synthetic Polynucleotide
gatgctcagctttcgtgctcagtgtcagtttcagtccagtaagccgccttcgccactgatgttcctcctaatatctacgcatttcaccgctacactaggaattccgcttacctctcctgcactccagtctgacagtttcaaaagcagtcccagagttaagccctgggttttcacttctgacttgccataccacctacgcaccctttacacccagtaattccggataacgcttgccccctacgtattaccgcggctgctggcacgtagttagccggggcttcttagtcaggtaccgtcattttcttccctgctgatagagctttacataccgagatacttcttcactcacgcggcgtcgctgcatcagggtttcccccattgtgcaatattccccactgctgcctcccgaaggaagtttgga

SEQ ID NO: 50 - DNA, 418 bp, Artificial Sequence
  Synthetic Polynucleotide
gtgtcagcttcgtgctcagtgtcagtttcagtccagtaagccgccttcgccactgatgttcctcctaatatctacgcatttcaccgctacactaggaattccgcttacctctcctgcactccagtctgacagtttcaaaagcagtcccagagttaagccctgggttttcacttctgacttgccataccacctacgcaccctttacacccagtaattccggataacgcttgccccctacgtattaccgcggctgctggcacgtagttagccggggcttcttagtcaggtaccgtcattttcttccctgctgatagagctttacataccgagatacttcttcactcacgcggcgtcgctgcatcagggtttcccccattgtgcaatattccccactgctgcctcccgtagggagtttgga

SEQ ID NO: 51 - DNA, 415 bp, Artificial Sequence
  Synthetic Polynucleotide
gtcagcttcgagcctcacgtcagttaccgtccagtaagccgccttcgccactggtgttcctcctaatatctacgcatttcaccgctacactaggaattccgcttacctctccggtactctagattgacagtttccaatgcagtcccggggttgagccccgggttttcacatcagacttgccactccgtctacgctccctttacacccagtaaatccggataacgcttgcaccatacgtattaccgcggctgctggcacgtatttagccggtgcttcttagtcaggtaccgtcattttcttccctgctgatagagctttacataccgaaatacttcatcgctcacgcggcgtcgctgcatcagggtttcccccattgtgcaatattccccactgctgcctcgcgtaggagtttgga

SEQ ID NO: 52 - DNA, 418 bp, Artificial Sequence
  Synthetic Polynucleotide
tgtcagctttcgagctcagcgtcagttatcgtccagtaagccgccttcgccactggtgttcctcctaatatctacgcatttcaccgctacactaggaattccgcttacccctccgacactctagtacgacagtttccaatgcagtaccggggttgagccccgggctttcacatcagacttgccgcaccgcctgcgctccctttacacccagtaaatccggataacgcttgcaccatacgtattaccgcggctgctggcacgtatttagccggtgcttcttagtcaggtaccgtcattatcttccctgctgatagagctttacataccgaaatacttcttcgctcacgcggcgtcgctgcatcaggctttcgcccattgtgcaatattccccactgctgcctcccgaagggagtttgga

SEQ ID NO: 53 - DNA, 416 bp, Artificial Sequence
  Synthetic Polynucleotide
ttcagctttcgagctcagcgtcagttatcgtccagtaagccgccttcgccactggtgttcctcctaatatctacgcatttcaccgctacactaggaattccgcttacccctccgacactctagtacgacagtttccaatgcagtaccggggttgagccccgggctttcacatcagacttgccgcaccgcctgcgctccctttacacccagtaaatccggataacgcttgcaccatacgtattaccgcggctgctggcacgtatttagccggtgcttcttagtcaggtaccgtcattatcttccctgctgatagagctttacataccgaaatacttcttcgctcacgcggcgtcgctgcatcaggctttcgcccattgtgcaatattccccactgctgcctcccgaggggagtttgg

SEQ ID NO: 54 - DNA, 435 bp, Artificial Sequence
  Synthetic Polynucleotide
ttcggtctgctttccccttctcgcgcctcagtgtcagtttctgtctagtaagccgccttcgccactgatgttcctcctaatatctacgcacttcaccgctccacaatgaattccgcttacccctcccgcgctctagtctgacagttttaaaaaaactccccgagagaaaccctgggttttttcttctgacatgcgatatcccacccccaccctttatacacccaaaaatcggataaaaggtgcgacctacgtattataccggctgctggggcgtagatagccgggggttcttatacagggaccgtcattttctttcccgctgatacagctttacataccgaaatacttctttctcacgcggcgtcgctgcatcagggtttcccccattgtgcaatattccccactgctgcctcccgaaggggaagttgggggaaa

SEQ ID NO: 55 - DNA, 418 bp, Artificial Sequence
  Synthetic Polynucleotide
gttcagctttcgagcctcacgtcagttaccgtccagtaagccgccttcgccactggtgttcctcctaatatctacgcatttcaccgctacactaggaattccgcttacctctccggtactctagattgacagtttccaatgcagtcccggggttgagccccgggttttcacatcagacttgccactccgtctacgctccctttacacccagtaaatccggataacgcttgcaccatacgtattaccgcggctgctggcacgtatttagccggtgcttcttagtcaggtaccgtcattttcttccctgctgatagagctttacataccgaaatacttcatcgctcacgcggcgtcgctgcatcagggtttcccccattgtgcaatattccccactgctgcctcccgaggggagtttgga

SEQ ID NO: 56 - DNA, 416 bp, Artificial Sequence
  Synthetic Polynucleotide
gtcagctttcgagctcacgtcagttaccgtccagtaagccgccttcgccactggtgttcctcctaatatctacgcatttcaccgctacactaggaattccgcttacctctccggtactctagattgacagtttccaatgcagtcccggggttgagccccgggttttcacatcagacttgccactccgtctacgctccctttacacccagtaaatccggataacgcttgcaccatacgtattaccgcggctgctggcacgtatttagccggtgcttcttagtcaggtaccgtcattttcttccctgctgatagagctttacataccgaaatacttcatcgctcacgcggcgtcgctgcatcagggtttcccccattgtgcaatattccccactgctgcctcccgaggggagtttgga

SEQ ID NO: 57 - DNA, 417 bp, Artificial Sequence
  Synthetic Polynucleotide
tctcacgctttcgagctcacgtcagtcatcgtccagcaagccgccttcgccactggtgttcctcctaatatctacgcatttcaccgctacactaggaattccacttgcctctccgacactctagctcagcagttccaaatgcagtcccggggttgagccccgggctttcacatctggcttgccgtgccgtctacgctccctttacacccagtaaatccggataacgcttgccccctacgtattaccgcggctgctggcacgtagttagccggggcttcttagtcaggtaccgtcattttcttccctgctgatagaagtttacataccgaaatacttcatccttcacgcggcgtcgctgcatcagagtttcctccattgtgcaatattccccactgctgcctcccgtagggagtttgg

SEQ ID NO: 58 - DNA, 417 bp, Artificial Sequence
  Synthetic Polynucleotide
gtcagctttcgagctcagcgtcagttatcgtccagtaagccgccttcgccactggtgttcctcctaatatctacgcatttcaccgctacactaggaattccacttacccctccgacactctagtacgacagtttccaatgcagtaccggggttgagccccgggctttcacatcagacttgccgcaccgcctgcgctccctttacacccagtaaatccggataacgcttgcaccatacgtattaccgcggctgctggcacgtatttagccggtgcttcttagtcaggtaccgtcattcttcttccctgctgatagagctttacataccgaaatacttcttcgctcacgcggcgtcgctgcatcagggtttcccccattgtgcaatattccccactgctgcctcccgagggagtttgga

SEQ ID NO: 59 - DNA, 419 bp, Artificial Sequence
  Synthetic Polynucleotide
agccccgctttcgagcctcacgtcagttaccgtccagtaagccgccttcgccactggtgttcctcctaatatctacgcatttcaccgctacactaggaattccgcttacctctccggcactcaagacgggcagtttccaatgcagtcccggggttgagccccagcctttcacatcagacttgtccatccgtctacgctccctttacacccagtaaatccggataacgcttgccccctacgtattaccgcggctgctggcacgtagttagccggggcttcttagtcaggtaccgtcattttcttccctgctgatagaagtttacataccgagatacttcttccttcacgcggcgtcgctgcatcagggtttcccccattgtgcaatattccccactgctgcctcccgaaggaagtttgga

SEQ ID NO: 60 - DNA, 419 bp, Artificial Sequence
  Synthetic Polynucleotide
tgctcagctttcgagcctcacgtcagttaccgtccagtaagccgccttcgccactggtgttcttcctaatatctacgcatttcaccgctacactaggaattccgcttacctctccggcactcgagccagacagtttccaatgcagtcccagggttaagccctgggttttcacatcagacttgccttgccgtctacgctccctttacacccagtaaatccggataacgcttgccccctacgtattaccgcggctgctggcacgtagttagccggggcttcttagtcaggtaccgtcattatcttccctgctgatagagctttacataccgaaatacttcttcgctcacgcggcgtcgctgcatcagggtttcccccattgtgcaatattccccactgctgcctcccgaagggagtttgga

SEQ ID NO: 61 - DNA, 421 bp, Artificial Sequence
  Synthetic Polynucleotide
gttgctcagctttcgagctcacgtcagttaccgtccagtaagccgccttcgccactggtgttcttcctaatatctacgcatttcaccgctacactaggaattccgcttacctctccggcactcgagccagacagtttccaatgcagtcccagggttaagccctgggttttcacatcagacttgccttgccgtctacgctccctttacacccagtaaatccggataacgcttgccccctacgtattaccgcggctgctggcacgtagttagccggggcttcttagtcaggtaccgtcattatcttccctgctgatagagctttacataccgaaatacttcttcgctcacgcggcgtcgctgcatcagggtttcccccattgtgcaatattccccactgctgcctcccgaaggaaagtttgga

SEQ ID NO: 62 - DNA, 420 bp, Artificial Sequence
  Synthetic Polynucleotide
tgctcagctttcgagctcagcgtcagttatcgtccagtaagccgccttcgccactggtgttcctcctaatatctacgcatttcaccgctacactaggaattccacttacccctccgacactctagtacgacagtttccaatgcagtaccggggttgagccccgggctttcacatcagacttgccgcaccgcctgcgctccctttacacccagtaaatccggataacgcttgcaccatacgtattaccgcggctgctggcacgtatttagccggtgcttcttagtcaggtaccgtcattcttcttccctgctgatagagctttacataccgaaatacttcttcgctcacgcggcgtcgctgcatcagggtttcccccattgtgcaatattccccactgctgcctcccgaagggagtttgga

SEQ ID NO: 63 - DNA, 446 bp, Artificial Sequence
  Synthetic Polynucleotide
gatgccctggcttcgcgctcagcgtcagttgtcgtccagaaagccgctttcgccactggtgttcctcctaatatctacgcatttcaccgctacactaggaattccgctttcctctccgacactcgagcttcacagtttcggtcccctcacggggttaagccccgcacttttaagaccgacttgcgatgccgcctgcgcgccctttacgcccaataattccggacaacgcttgccacctacgtattaccgcggctgctggcacgtagttagccgtggctttctcttacggtaccgtcagggataacgggtattgaccgctatcctgttcgtcccatataacagaactttacaacccgaaggccgtcatcgttcacgcggcgttgctccgtcagactttcgtccattgcggaagattccccactgctgcctcccggggggagtttgga

SEQ ID NO: 64 - DNA, 419 bp, Artificial Sequence
  Synthetic Polynucleotide
gtcccgctttcgagcctcagcgtcagttatcgtccagtaagccgccttcgccactggtgttcctcctaatatctacgcatttcaccgctacactaggaattccgcttacccctccgacactctagtacgacagtttccaatgcagtaccggggttgagccccgggctttcacatcagacttgccgcaccgcctgcgctccctttacacccagtaaatccggataacgcttgcaccatacgtattaccgcggctgctggcacgtatttagccggtgcttcttagtcaggtaccgtcattatcttccctgctgatagagctttacataccgaaatacttcttcgctcacgcggcgtcgctgcatcaggctttcgcccattgtgcaatattccccactgctgcctcccgaagggaagtttgg

SEQ ID NO: 65 - DNA, 418 bp, Artificial Sequence; identical to SEQ ID NO: 52
  Synthetic Polynucleotide

SEQ ID NO: 66 - DNA, 420 bp, Artificial Sequence; identical to SEQ ID NO: 62
  Synthetic Polynucleotide

SEQ ID NO: 67 - DNA, 417 bp, Artificial Sequence
  Synthetic Polynucleotide
attcagctttcgagctcacgtcagttaccgtccagtaagccgccttcgccactggtgttcctcctaatatctacgcatttcaccgctacactaggaattccgcttacccctccggcactcaagcataccagtttccaatgcagtccaggggttaagcccctgcctttcacatcagacttgatacgccgtctacgctccctttacacccagtaaatccggataacgctcgccccctacgtattaccgcggctgctggcacgtagttagccggggcttcttagtcaggtaccgtcattatcttccctgctgatagaagtttacataccgagatacttcttccttcacgcggcgtcgctgcatcagggtttcccccattgtgcaatattccccactgctgcctcccgagggaagtttgga

SEQ ID NO: 68 - DNA, 416 bp, Artificial Sequence
  Synthetic Polynucleotide
gtgtcagctttcgagctcacgtcagttaccgtccagtaagccgccttcgccactggtgttcttcctaatatctacgcatttcaccgctacactaggaattccgcttacctctccggcactcgagccagacagtttccaatgcagtcccagggttaagccctgggttttcacatcagacttgccttgccgtctacgctccctttacacccagtaaatccggataacgcttgccccctacgtattaccgcggctgctggcacgtagttagccggggcttcttagtcaggtaccgtcattatcttccctgctgatagagctttacataccgaaatacttcttcgctcacgcggcgtcgctgcatcagggtttcccccattgtgcaatattccccactgctgcctcccgagggagtttgg

SEQ ID NO: 69 - DNA, 416 bp, Artificial Sequence
  Synthetic Polynucleotide
gccagcttcgagcctcacgtcagtcatcgtccagtaagccgccttcgccactggtgttcctcctaatatctacgcatttcaccgctacactaggaattccacttacctctccgacactctagctgcacagtttccaaagcagtccacaggttgagcccatgcctttcacttcagacttgcacagccgtctacgctccctttacacccagtaaatccggataacgcttgccccctacgtattaccgcggctgctggcacgtagttagccggggcttcttagtcaggtaccgtcattttcttccctgctgatagaagtttacataccgaaatacttcatccttcacgcggcgtcgctgcatcaggctttcgcccattgtgcaatattccccactgctgcctcccgagggaagtttgga

SEQ ID NO: 70 - DNA, 418 bp, Artificial Sequence
  Synthetic Polynucleotide
tgatcagctttcgagctcacgtcagttaccgtccagtaagccgccttcgccactggtgttcctcctaatatctacgcatttcaccgctacactaggaattccgcttacctctccggtactctagattgacagtttccaatgcagtcccggggttgagccccgggttttcacatcagacttgccactccgtctacgctccctttacacccagtaaatccggataacgcttgcaccatacgtattaccgcggctgctggcacgtatttagccggtgcttcttagtcaggtaccgtcattttcttccctgctgatagagctttacataccgaaatacttcatcgctcacgcggcgtcgctgcatcagggtttcccccattgtgcaatattccccactgctgcctcccggggggagtttgga

SEQ ID NO: 71 - DNA, 420 bp, Artificial Sequence
  Synthetic Polynucleotide
gatgatcagctttcgagctcacgtcagttaccgtccagtaagccgccttcgccactggtgttcctcctaatatctacgcatttcaccgctacactaggaattccgcttacctctccggcactctagaaaaacagtttccaatgcagtcctggggttaagccccagcctttcacatcagacttgctcttccgtctacgctccctttacacccagtaaatccggataacgcttgccccctacgtattaccgcggctgctggcacgtagttagccggggcttcttagtcaggtaccgtcattttcttccctgctgatagaagtttacataccgagatacttcttccttcacgcggcgtcgctgcatcagggtttcccccattgtgcaatattccccactgctgcctcccgggggaagtttgga

SEQ ID NO: 72 - DNA, 418 bp, Artificial Sequence
  Synthetic Polynucleotide
ttgatcagctttcgagctcacgtcagttaccgtccagtaagccgccttcgccactggtgttcctcctaatatctacgcatttcaccgctacactaggaattccgcttacctctccggcactctagaaaaacagtttccaatgcagtcctggggttaagccccagcctttcacatcagacttgctcttccgtctacgctccctttacacccagtaaatccggataacgcttgccccctacgtattaccgcggctgctggcacgtagttagccggggcttcttagtcaggtaccgtcattttcttccctgctgatagaagtttacataccgagatacttcttccttcacgcggcgtcgctgcatcagggtttcccccattgtgcaatattccccactgctgcctcccgaagggagtttgg

SEQ ID NO: 73 - DNA, 421 bp, Artificial Sequence
  Synthetic Polynucleotide
gtatttcagctttcgagctcagcgtcagttatcgtccagtaagccgccttcgccactggtgttcctcctaatatctacgcatttcaccgctacactaggaattccgcttacccctccgacactctagtacgacagtttccaatgcagtaccggggttgagccccgggctttcacatcagacttgccgcaccgcctgcgctccctttacacccagtaaatccggataacgcttgcaccatacgtattaccgcggctgctggcacgtatttagccggtgcttcttagtcaggtaccgtcattatcttccctgctgatagagctttacataccgaaatacttcttcgctcacgcggcgtcgctgcatcaggctttcgcccattgtgcaatattccccactgctgcctcccgaagggagtttgga

SEQ ID NO: 74 - DNA, 419 bp, Artificial Sequence
  Synthetic Polynucleotide
gctcagctttcgagctcagcgtcagttatcgtccagtaagccgccttcgccactggtgttcctcctaatatctacgcatttcaccgctacactaggaattccacttacccctccgacactctagtacgacagtttccaatgcagtaccggggttgagccccgggctttcacatcagacttgccgcaccgcctgcgctccctttacacccagtaaatccggataacgcttgcaccatacgtattaccgcggctgctggcacgtatttagccggtgcttcttagtcaggtaccgtcattcttcttccctgctgatagagctttacataccgaaatacttcttcgctcacgcggcgtcgctgcatcagggtttcccccattgtgcaatattccccactgctgcctcccgaggggagtttgga

SEQ ID NO: 75 - DNA, 417 bp, Artificial Sequence
  Synthetic Polynucleotide
tttcagcttcgagcctcagcgtcagttatcgtccagtaagccgccttcgccactggtgttcctcctaatatctacgcatttcaccgctacactaggaattccgcttacccctccgacactctagtacgacagtttccaatgcagtaccggggttgagccccgggctttcacatcagacttgccgcaccgcctgcgctccctttacacccagtaaatccggataacgcttgcaccatacgtattaccgcggctgctggcacgtatttagccggtgcttcttagtcaggtaccgtcattatcttccctgctgatagagctttacataccgaaatacttcttcgctcacgcggcgtcgctgcatcaggctttcgcccattgtgcaatattccccactgctagctcccgaaggagtttgga

SEQ ID NO: 76 - DNA, 419 bp, Artificial Sequence
  Synthetic Polynucleotide
agctcagctttcgagctcagcgtcagttatcgtccagtaagccgccttcgccactggtgttcctcctaatatctacgcatttcaccgctacactaggaattccgcttacccctccgacactctagtacgacagtttccaatgcagtaccggggttgagccccgggctttcacatcagacttgccgcaccgcctgcgctccctttacacccagtaaatccggataacgcttgcaccatacgtattaccgcggctgctggcacgtatttagccggtgcttcttagtcaggtaccgtcattatcttccctgctgatagagctttacataccgaaatacttcttcgctcacgcggcgtcgctgcatcaggctttcgcccattgtgcaatattccccactgctgcctcccgaagggagtttgga

SEQ ID NO: 77 - DNA, 418 bp, Artificial Sequence
  Synthetic Polynucleotide
gtccagctttcgagcctcagcgtcagttatcgtccagtaagccgccttcgccactggtgttcctcctaatatctacgcatttcaccgctacactaggaattccgcttacccctccgacactctagtacgacagtttccaatgcagtaccggggttgagccccgggctttcacatcagacttgccgcaccgcctgcgctccctttacacccagtaaatccggataacgcttgcaccatacgtattaccgcggctgctggcacgtatttagccggtgcttcttagtcaggtaccgtcattatcttccctgctgatagagctttacataccgaaatacttcttcgctcacgcggcgtcgctgcatcaggctttcgcccattgtgcaatattccccactgctgcctcccgagggagtttgga

SEQ ID NO: 78 - DNA, 193 bp, Artificial Sequence
  Synthetic Polynucleotide
tgagccgggctcaccccggtactgcattggaactgtcgtactagagtgtcggaggggtaagcggaattcctagtgtagcggtgaaatgcgtagatattaggaggaacaccagtggcgaaggcggcttactggacgataactgacgctgaggctcgaaagcgtggggagcaaacaggattagatacaccggtaa

SEQ ID NO: 79 - DNA, 424 bp, Artificial Sequence
  Synthetic Polynucleotide
cacgatgtcagctttcgagctcagcgtcagttatcgtccagtaagccgccttcgccactggtgttcctcctaatatctacgcatttcaccgctacactaggaattccacttacccctccgacactctagtacgacagtttccaatgcagtaccggggttgagccccgggctttcacatcagacttgccgcaccgcctgcgctccctttacacccagtaaatccggataacgcttgcaccatacgtattaccgcggctgctggcacgtatttagccggtgcttcttagtcaggtaccgtcattcttcttccctgctgatagagctttacataccgaaatacttcttcgctcacgcggcgtcgctgcatcagggtttcccccattgtgcaatattccccactgctgcctcccgaggggagtttgga

SEQ ID NO: 80 - DNA, 1524 bp, Artificial Sequence
  Synthetic Polynucleotide
atggagagtttgatcctggctcaggatgaacgctggcggcgtgcctaatacatgcaagtcgaacgcgagcacttgtgctcgagtggcgaacgggtgagtaatacataagtaacctgccctagacagggggataactattggaaacgatagctaagaccgcataggtacggacactgcatggtgaccgtattaaaagtgcctcaaagcactggtagaggatggacttatggcgcattagctggttggcggggtaacggcccaccaaggcgacgatgcgtagccgacctgagagggtgaccggccacactgggactgagacacggcccagactcctacgggaggcagcagtagggaattttcggcaatgggggaaaccctgaccgagcaacgccgcgtgaaggaagaaggttttcggattgtaaacttctgttataaaggaagaacggcggctacaggaaatggtagccgagtgacggtactttattagaaagccacggctaactacgtgccagcagccgcggtaatacgtaggtggcaagcgttatccggaattattgggcgtaaagagggagcaggcggcagcaagggtctgtggtgaaagcctgaagcttaacttcagtaagccatagaaaccaggcagctagagtgcaggagaggatcgtggaattccatgtgtagcggtgaaatgcgtagatatatggaggaacaccagtggcgaaggcgacgatctggcctgcaactgacgctcagtcccgaaagcgtggggagcaaataggattagataccctagtagtccacgccgtaaacgatgagtactaagtgttggatgtcaaagttcagtgctgcagttaacgcaataagtactccgcctgagtagtacgttcgcaagaatgaaactcaaaggaattgacgggggcccgcacaagcggtggagcatgtggtttaattcgaagcaacgcgaagaaccttaccaggtcttgacatactcataaaggctccagagatggagagatagctatatgagatacaggtggtgcatggttgtcgtcagctcgtgtcgtgagatgttgggttaagtcccgcaacgagcgcaacccttatcgttagttaccatcattaagttggggactctagcgagactgccagtgacaagctggaggaaggcggggatgacgtcaaatcatcatgccccttatgacctgggctacacacgtgctacaatggatggtgcagagggaagcgaagccgcgaggtgaagcaaaacccataaaaccattctcagttcggattgtagtctgcaactcgactacatgaagttggaatcgctagtaatcgcgaatcagcatgtcgcggtgaatacgttctcgggccttgtacacaccgcccgtcacaccacgagagttgataacacccgaagccggtggcctaaccgcaaggaaggagctgtctaaggtgggattgatgattggggtgaagtcgtaacaaggtatccctacgggaacgtggggatggatcacctccttt

SEQ ID NO: 81 - DNA, 1528 bp, Artificial Sequence
  Synthetic Polynucleotide
atgagagtttgatcctggctcaggatgaacgctggcggcgtgcctaacacatgcaagtcgaacgaagcaattgaaggaagttttcggatggaattcgattgactgagtggcggacgggtgagtaacgcgtggataacctgcctcacactgggggataacagttagaaatgactgctaataccgcataagcgcacagtaccgcatggtacagtgtgaaaaactccggtggtgtgagatggatccgcgtctgattagccagttggcggggtaacggcccaccaaagcgacgatcagtagccgacctgagagggtgaccggccacattgggactgagacacggcccaaactcctacgggaggcagcagtggggaatattgcacaatgggcgaaagcctgatgcagcgacgccgcgtgagtgaagaagtatttcggtatgtaaagctctatcagcagggaagaaaatgacggtacctgactaagaagccccggctaactacgtgccagcagccgcggtaatacgtagggggcaagcgttatccggatttactgggtgtaaagggagcgtagacggcgaagcaagtctgaagtgaaaacccagggctcaaccctgggactgctttggaaactgttttgctagagtgtcggagaggtaagtggaattcctagtgtagcggtgaaatgcgtagatattaggaggaacaccagtggcgaaggcggcttactggacgataactgacgttgaggctcgaaagcgtggggagcaaacaggattagataccctggtagtccacgccgtaaacgatgaatgctaggtgttggggggcaaagcccttcggtgccgtcgcaaacgcagtaagcattccacctggggagtacgttcgcaagaatgaaactcaaaggaattgacggggacccgcacaagcggtggagcatgtggtttaattcgaagcaacgcgaagaaccttaccaagtcttgacatcctcttgaccggcgtgtaacggcgccttcccttcggggcaagagagacaggtggtgcatggttgtcgtcagctcgtgtcgtgagatgttgggttaagtcccgcaacgagcgcaacccttatccttagtagccagcaggtaaagctgggcactctagggagactgccagggataacctggaggaaggtggggatgacgtcaaatcatcatgccccttatgatttgggctacacacgtgctacaatggcgtaaacaaagggaagcaagacagtgatgtggagcaaatcccaaaaataacgtcccagttcggactgtagtctgcaacccgactacacgaagctggaatcgctagtaatcgcgaatcagaatgtcgcggtgaatacgttcccgggtcttgtacacaccgcccgtcacaccatgggagtcagcaacgcccgaagtcagtgacccaactcgcaagagagggagctgccgaaggcggggcaggtaactggggtgaagtcgtaacaaggtagccgtatcggaaggtgcggctggatcacctccttt

SEQ ID NO: 82 - DNA, 385 bp, Artificial Sequence
  Synthetic Polynucleotide
aattcgacgttgtccggattactgggcgtaaagggagcgtaggcggacttttaagtgagatgtgaaatacccgggctcaacttgggtgctgcatttcaaactggaagtctagagtgcaggagaggagaatggaattcctagtgtagcggtgaaatgcgtagagattaggaagaacaccagtggcgaaggcgattctctggactgtaactgacgctgaggctcgaaagcgtggggagcaaacaggattagataccctggtagtccacgccgtaaacgatgaatactaggtgtaggggttgtcatgacctctgtgccgccgctaacgcattaagtattccgcctggggagtacggtcgcaagattaaaactcaaagaaattgacgga

SEQ ID NO: 83 - DNA, 434 bp, Artificial Sequence
  Synthetic Polynucleotide
acgagcgtatcggattattgggtttaagggagcgtaggtggattgttaagtcagttgtgaaagtttgcggctcaaccgtaaaattgcagttgaaactggcagtcttgagtacagtagaggtgggcggaattcgtggtgtagcggtgaaatgcttagatatcacgaagaactccgattgcgaaggcagctcactagactgtcactgacactgatgctcgaaagtgtgggtatcaaacaggattagataccctggtagtccacacagtaaacgatgaatactcgctgtttgcgatatacagtaagcggccaagcgaaagcattaagtattccacctggggagtacgccggcaacggtgaaactcaaagaaattgacggaagcccgcccaggggggaaaaacatggggtttagttggatgatacggggaggaacctc

SEQ ID NO: 84 - DNA, 1457 bp, Ruminococcus obeum
  misc_feature (65)..(66): n is a, c, g, t or u
  misc_feature (960)..(960): n is a, c, g, t or u
ggcggcgtgcttaacacatgcaagtcgaacgggaaacctttcattgaagcttcggcagatttggnntgtttctagtggcggacgggtgagtaacgcgtgggtaacctgccttatacagggggataacaaccagaaatggttgctaataccgcataagcgcacaggaccgcatggtctggtgtgaaaaactccggtggtataagatggacccgcgttggattagctagttggcagggtaacggcctaccaaggcgacgatccatagccggcctgagagggtgaacggccacattgggactgagacacggcccagactcctacgggaggcagcagtggggaatattgcacaatgggggaaaccctgatgcagcgacgccgcgtgaaggaagaagtatctcggtatgtaaacttctatcagcagggaagatagtgacggtacctgactaagaagccccggctaactacgtgccagcagccgcggtaatacgtagggggcaagcgttatccggatttactgggtgtaaagggagcgtagacggactggcaagtctgatgtgaaaggcgggggctcaacccctggactgcattggaaactgttagtcttgagtgccggagaggtaagcggaattcctagtgtagcggtgaaatgcgtagatattaggaggaacaccagtggcgaaggcggcttactggacggtaactgacgttgaggctcgaaagcgtggggagcaaacaggattagataccctggtagtccacgccgtaaacgatgattactaggtgttggggagcaaagctcttcggtgccgccgcaaacgcattaagtattccacctggggagtacgttcgcaagaatgaaactcaaaggaattgacggggacccgcacaagcggtggagcatgtggtttaattcgaagcaacgcgaagaaccttaccaagtcttgacatccctctgaccgncccttaaccggatctttccttcgggacaggggagacaggtggtgcatggttgtcgtcagctcgtgtcgtgagatgttgggttaagtcccgcaacgagcgcaacccctatccccagtagccagcagtccggctgggcactctgaggagactgccagggataacctggaggaaggcggggatgacgtcaaatcatcatgccccttatgatttgggctacacacgtgctacaatggcgtaaacaaagggaagcaagcctgcgaaggtaagcaaatcccaaaaataacgtcccagttcggactgcagtctgcaactcgactgcacgaagctggaatcgctagtaatcgcggatcagaatgccgcggtgaatacgttcccgggtcttgtacacaccgcccgtcacaccatgggagtcagtaacgcccgaagtcagtgacctaactgcaaagaaggagctgccgaaggcgggaccgatgactggggtgaagtcgtaacaaggt

SEQ ID NO: 85 - DNA, 1398 bp, Ruminococcus obeum
  misc_feature (1083)..(1083): n is a, c, g, t or u
  misc_feature (1207)..(1207): n is a, c, g, t or u
  misc_feature (1233)..(1233): n is a, c, g, t or u
ggcgtgcttaacacatgcaagtcgaacgggaaacttttcattgaagcttcggcagatttggtctgtttctagtggcggacgggtgagtaacgcgtgggtaacctgccttatacagggggataacaaccagaaatggttgctaataccgcataagcgcacaggaccgcatggtctggtgtgaaaaactccggtggtataagatggacccgcgttggattagctagttggcagggtaacggcctaccaaggcgacgatccatagccggcctgagagggtgaacggccacattgggactgagacacgccccagactcctcgggaggcagcagtggggaatattgcacaatgggggaaaccctgatgcagcgacgccgcgtgaaggaagaagtatctcggtatgtaaacttctatcagcagggaagatagtgacggtacctgactaagaagccccgkctaactacgtgccagcagccgcggtaatacgtagggggcaagcgttatccggatttactgggtgtaaagggagcgtagacggactggcaagtctgatgtgaaaggcgggggctcaacccctggactgcattggaaactgttagtcttgagtgccggagaggtaagcggaattcctagtgtagcggtgaaatgcgtagatattaggaggaacaccagtggcgaaggcggcttactggacggtaactgacgttgaggctcgaaagcgtggggagcaaacaggattagataccctggtagtccacgccgcaaacgatgaatactaggtgttggggagcaaagctcttcggtgccgccgcaaacgcattaagtattccacctggggagtacgttcgcaagaatgaaactcaaaggaattgacggggacccgcacaagcggtggagcatgtggtttaattcgaagcaacgcgaagaaccttaccaagtcttgacatccctctgaccgtcccttaaccggatctttccttcgggacaggggagacaggtggtgcatggttgtcgtcagctcgtgtcgtgagatgttgggttaagtcccgcaacgagcgcaacccctatccccagtagccagcagtncggctgggcactctgaggagactgccagggataacctggaggaaggcggggatgacgtcaaatcatcatgccccttatgatttgggctacacacgtgctacaatggcgtaaacaaagggaagcnagcctkcgraggtaagcaaatcccanaaataacgtcccagttcggactgcagtctgcaactcgactgcacgaagctggaatcgctagtaatcgcggatcagaatgccgcggtgaatacgttcccgggtcttgtacacaccgcccgtcacaccatgggagtcagtaacgcccgaagtcagtgacctaactgc

SEQ ID NO: 86 - DNA, 1472 bp, Clostridium disporicum
gctcaggacgaacgctggcggcgtgcctaacacatgcaagtcgagcgagttgattctcttcggagatgaagctagcggcggacgggtgagtaacacgtgggcaacctgcctcatagaggggaatagcctcccgaaagggagattaataccgcataagattgtagcttcgcatgaagtagcaattaaaggagcaatccgctatgagatgggcccgcggcgcattagctagttggtgaggtaacggctcaccaaggcgacgatgcgtagccgacctgagagggtgatcggccacattgggactgagacacggcccagactcctacgggaggcagcagtggggaatattgcacaatgggggaaaccctgatgcagcaacgccgcgtgagtgatgacggccttcgggttgtaaagctctgtcttcagggacgataatgacggtacctgaggaggaagccacggctaactacgtgccagcagccgcggtaatacgtaggtggcgagcgttgtccggatttactgggcgtaaagggagcgtaggcggacttttaagtgagatgtgaaatacccgggctcaacttgggtgctgcatttcaaactggaagtctagagtgcaggagaggagaatggaattcctagtgtagcggtgaaatgcgtagagattaggaagaacaccagtggcgaaggcgattctctggactgtaactgacgctgaggctcgaaagcgtggggagcaaacaggattagataccctggtagtccacgccgtaaacgatgaatactaggtgtaggggttgtcatgacctctgtgccgccgctaacgcattaagtattccgcctggggagtacggtcgcaagattaaaactcaaaggaattgacgggggcccgcacaagcagcggagcatgtggtttaattcgaagcaacgcgaagaaccttacctagacttgacatctcctgaattacccgtaactggggaagccacttcggtggcaggaagacaggtggtgcatggttgtcgtcagctcgtgtcgtgagatgttgggttaagtcccgcaacgagcgcaacccttattgttagttgctaccatttagttgagcactctagcgagactgcccgggttaaccgggaggaaggtggggatgacgtcaaatcatcatgccccttatgtctagggctacacacgtgctacaatggcaagtacaaagagaagcaagaccgcgaggtggagcaaaactcaaaaacttgtctcagttcggattgtaggctgaaactcgcctacatgaagctggagttgctagtaatcgcgaatcagcatgtcgcggtgaatacgttcccgggccttgtacacaccgcccgtcacaccatgagagttggcaatacccaacgtacgtgatctaacccgcaagggaggaagcgtcctaaggtagggtcagcgattggggtgaagtcgtaacaaggtagccgtaggagaa

SEQ ID NO: 87 - DNA, 1529 bp, Clostridium scindens
gagagtttgatcctggctcaggatgaacgctggcggcgtgcctaacacatgcaagtcgaacgaagcgcctggccccgacttcttcggaacgaggagccttgcgactgagtggcggacgggtgagtaacgcgtgggcaacctgccttgcactgggggataacagccagaaatggctgctaataccgcataagaccgaagcgccgcatggcgcggcggccaaagccccggcggtgcaagatgggcccgcgtctgattaggtagttggcggggtaacggcccaccaagccgacgatcagtagccgacctgagagggtgaccggccacattgggactgagacacggcccagactcctacgggaggcagcagtggggaatattgcacaatgggggaaaccctgatgcagcgacgccgcgtgaaggatgaagtatttcggtatgtaaacttctatcagcagggaagaagatgacggtacctgactaagaagccccggctaactacgtgccagcagccgcggtaatacgtagggggcaagcgttatccggatttactgggtgtaaagggagcgtagacggcgatgcaagccagatgtgaaagcccggggctcaaccccgggactgcatttggaactgcgtggctggagtgtcggagaggcaggcggaattcctagtgtagcggtgaaatgcgtagatattaggaggaacaccagtggcgaaggcggcctgctggacgatgactgacgttgaggctcgaaagcgtggggagcaaacaggattagataccctggtagtccacgccgtaaacgatgactactaggtgtcgggtggcaaggccattcggtgccgcagcaaacgcaataagtagtccacctggggagtacgttcgcaagaatgaaactcaaaggaattgacggggacccgcacaagcggtggagcatgtggtttaattcgaagcaacgcgaagaaccttacctgatcttgacatcccgatgccaaagcgcgtaacgcgctctttcttcggaacatcggtgacaggtggtgcatggttgtcgtcagctcgtgtcgtgagatgttgggttaagtcccgcaacgagcgcaacccctatcttcagtagccagcattttggatgggcactctggagagactgccagggagaacctggaggaaggtggggatgacgtcaaatcatcatgccccttatgaccagggctacacacgtgctacaatggcgtaaacaaagggaggcgaacccgcgagggtgggcaaatcccaaaaataacgtctcagttcggattgtagtctgcaactcgactacatgaagttggaatcgctagtaatcgcgaatcagaatgtcgcggtgaatacgttcccgggtcttgtacacaccgcccgtcacaccatgggagtcagtaacgcccgaagccggtgacccaacccgtaagggagggagccgtcgaaggtgggaccgataactggggtgaagtcgtaacaaggtagccgtatcggaaggtgcggctggatcacctccttc

SEQ ID NO: 88 - DNA, 1456 bp, Anaerostipes caccae
gcgcttaatacatgtcaagtcgaacgaagcatttaggattgaagttttcggatggatttcctatatgactgagtggcggacgggtgagtaacgcgtggggaacctgccctatacagggggataacagctggaaacggctgctaataccgcataagcgcacagaatcgcatgattcagtgtgaaaagccctggcagtataggatggtcccgcgtctgattagctggttggtgaggtaacggctcaccaaggcgacgatcagtagccggcttgagagagtgaacggccacattgggactgagacacggcccaaactcctacgggaggcagcagtggggaatattgcacaatgggggtaaaccctgatgcagcgacgccgcgtgagtgaagaagtatttcggtatgtaaagctctatcagcagggaagaaaacagacggtacctgactaagaagccccggctaactacgtgccagcagccgcggtaatacgtagggggcaagcgttatccggaattactgggtgtaaagggtgcgtaggtggcatggtaagtcagaagtgaaagcccggggcttaaccccgggactgcttttgaaactgtcatgctggagtgcaggagaggtaagcggaattcctagtgtagcggtgaaatgcgtagatattaggaggaacaccagtggcgaaggcggcttactggactgtcactgacactgatgcacgaaagcgtggggagcaaacaggattagataccctggtagtccacgccgtaaacgatgaatactaggtgtcggggccgtagaggcttcggtgccgcagcaaacgcagtaagtattccacctggggagtacgttcgcaagaatgaaactcaaaggaattgacggggacccgcacaagcggtggagcatgtggtttaattcgaagcaacgcgaagaaccttacctggtcttgacatcccaatgaccgaaccttaaccggttttttctttcgagacattggagacaggtggtgcatggttgtcgtcagctcgtgtcgtgagatgttgggttaagtcccgcaacgagcgcaacccctatctttagtagccagcatttaaggtgggcactctagagagactgccagggataacctggaggaaggtggggacgacgtcaaatcatcatgccccttatggccagggctacacacgtgctacaatggcgtaaacaaagggaagcgaagtcgtgaggcgaagcaaatcccagaaataacgtctcagttcggattgtagtctgcaactcgactacatgaagctggaatcgctagtaatcgtgaatcagaatgtcacggtgaatacgttcccgggtcttgtacacaccgcccgtcacaccatgggagtcagtaacgcccgaagtcagtgacccaaccgcaaggagggagctgccgaaggtgggaccgataactggggtgaagtcgtaacaagg

SEQ ID NO: 89 - DNA, 1456 bp, Marvinbryantia formatexigens
tggcggcgtgcttaacacatgcaagtcgagcgaagcattttaaatgaagttttcggacggaatttaaaatgactgagcggcggacgggtgagtaacgcgtggataacctgccttatacagggggataacagccagaaatggctgctaataccgcataagcgcacggtaccgcatggtacagtgtgaaaaactccggtggtataagatgggtccgcgttggattaggcagttggcggggtaaaggcccaccaaaccgacgatccatagccggcctgagagggtggacggccacattgggactgagacacggcccagactcctacgggaggcagcagtggggaatattgcacaatgggggaaaccctgatgcagcgacgccgcgtgggtgaagaagtatttcggtatgtaaagccctatcagcagggaagaaaatgacggtacctgaccaagaagccccggctaactacgtgccagcagccgcggtaatacgtagggggcaagcgttatccggatttactgggtgtaaagggagcgtagacggccatgcaagtctggtgtgaaaggcgggggctcaacccccggactgcattggaaactgtatggcttgagtgccggagaggtaagcggaattcctggtgtagcggtgaaatgcgtagatatcaggaggaacaccagtggcgaaggcggcttactggacggtaactgacgttgaggctcgaaagcgtggggagcaaacaggattagataccctggtagtccacgccgtaaacgatgaataccaggtgtcgggggacacggtccttcggtgccgcagcaaacgcactaagtattccacctggggagtacgttcgcaagaatgaaactcaaaggaattgacggggacccgcacaagcggtggagcatgtggtttaattcgaagcaacgcgaagaaccttaccaggtcttgacatccggacgaccggacagtaacgtgtccttcccttcggggcgtccgagacaggtggtgcatggttgtcgtcagctcgtgtcgtgagatgttgggttaagtcccgcaacgagcgcaacccctgttcccagtagccagcattcaggatgggcactctggggagactgccagggataacctggaggaaggcggggatgacgtcaaatcatcatgccccttatgatctgggctacacacgtgctacaatggcgtgaacagagggaagcgaacccgcgagggggagcaaatcccagaaataacgtcccagttcggattgtagtctgcaacccggctacatgaagctggaatcgctagtaatcgcggatcagcatgccgcggtgaatacgttcccgggtcttgtacacaccgcccgtcacaccatgggagtcggaaatgcccgaagtcagtgacccaaccggaaggagggagctgccgaaggcggggccggtaactggggtgaagtcgtaacaa

SEQ ID NO: 90 - DNA, 1568 bp, Lactobacillus mucosae
agagtttgatcctggctcaggatgaacgccggcggtgtgcctaatacatgcaagtcgaacgcgttggcccaactgattgaacgtgcttgcacggacttgacgttggtttaccagcgagtggcggacgggtgagtaacacgtaggtaacctgccccaaagcgggggataacatttggaaacagatgctaataccgcataacaatttgaatcgcatgattcaaatttaaaagatggcttcggctatcactttgggatggacctgcggcgcattagcttgttggtagggtaacggcctaccaaggctgtgatgcgtagccgagttgagagactgatcggccacaatggaactgagacacggtccatactcctacgggaggcagcagtagggaatcttccacaatgggcgcaagcctgatggagcaacaccgcgtgagtgaagaagggtttcggctcgtaaagctctgttgttagagaagaacgtgcgtgagagcaactgttcacgcagtgacggtatctaaccagaaagtcacggctaactacgtgccagcagccgcggtaatacgtaggtggcaagcgttatccggatttattgggcgtaaagcgagcgcaggcggtttgataagtctgatgtgaaagcctttggcttaaccaaagaagtgcatcggaaactgtcagacttgagtgcagaagaggacagtggaactccatgtgtagcggtggaatgcgtagatatatggaagaacaccagtggcgaaggcggctgtctggtctgcaactgacgctgaggctcgaaagcatgggtagcgaacaggattagataccctggtagtccatgccgtaaacgatgagtgctaggtgttggagggtttccgcccttcagtgccgcagctaacgcattaagcactccgcctggggagtacgaccgcaaggttgaaactcaaaggaattgacgggggcccgcacaagcggtggagcatgtggtttaattcgaagctacgcgaagaaccttaccaggtcttgacatcttgcgccaaccctagagatagggcgtttccttcgggaacgcaatgacaggtggtgcatggtcgtcgtcagctcgtgtcgtgagatgttgggttaagtcccgcaacgagcgcaacccttgttactagttgccagcattcagttgggcactctagtgagactgccggtgacaaaccggaggaaggtggggacgacgtcagatcatcatgccccttatgacctgggctacacacgtgctacaatggacggtacaacgagtcgcgaactcgcgagggcaagctaatctcttaaaaccgttctcagttcggactgcaggctgcaactcgcctgcacgaagtcggaatcgctagtaatcgcggatcagcatgccgcggtgaatacgttcccgggccttgtacacaccgcccgtcacaccatgagagtttgcaacacccaaagtcggtggggtaacccttcggggagctagccgcctaaggtggggcagatgattagggtgaagtcgtaacaaggtagccgtaggagaacctgcggctggatcacctcct

SEQ ID NO: 91 - DNA, 1508 bp, Turicibacter sanguinis
agagtttgatcatggctcaggatgaacgctggcggcgtgcctaatacatgcaagtcgagcgaaccacttcggtggtgagcggcgaacgggtgagtaacacgtaggttatctgcccatcagacggggacaacgattggaaacgatcgctaataccggataggacgaaagtttaaaggtgcttcggcaccactgatggatgagcctgcggcgcattagctagttggtagggtaaaggcctaccaaggcgacgatgcgtagccgacctgagagggtgaacggccacactgggactgagacacggcccagactcctacgggaggcagcagtagggaatcttcggcaatgggcgaaagcctgaccgagcaacgccgcgtgaatgatgaaggccttcgggttgtaaaattctgttataagggaagaatggctctagtaggaaatggctagagtgtgacggtaccttatgagaaagccacggctaactacgtgccagcagccgcggtaatacgtaggtggcgagcgttatccggaattattgggcgtaaagagcgcgcaggtggttgattaagtctgatgtgaaagcccacggcttaaccgtggagggtcattggaaactggtcaacttgagtgcagaagagggaagtggaattccatgtgtagcggtgaaatgcgtagagatatggaggaacaccagtggcgaaggcggcttcctggtctgtaactgacactgaggcgcgaaagcgtggggagcaaacaggattagataccctggtagtccacgccgtaaacgatgagtgctaagtgttgggggtcgaacctcagtgctgaagttaacgcattaagcactccgcctggggagtacggtcgcaagactgaaactcaaaggaattgacggggacccgcacaagcggtggagcatgtggtttaattcgaagcaacgcgaagaaccttaccaggtcttgacataccagtgaccgtcctagagataggattttcccttcggggacaatggatacaggtggtgcatggttgtcgtcagctcgtgtcgtgagatgttgggttaagtcccgcaacgagcgcaacccctgtcgttagttgccagcattcagttggggactctaacgagactgccagtgacaaactggaggaaggtggggatgacgtcaaatcatcatgccccttatgacctgggctacacacgtgctacaatggttggtacaaagagaagcgaagcggtgacgtggagcaaacctcataaagccaatctcagttcggattgtaggctgcaactcgcctacatgaagttggaatcgctagtaatcgcgaatcagcatgtcgcggtgaatacgttcccgggtcttgtacacaccgcccgtcacaccacgagagtttacaacacccgaagtcagtggcctaaccgcaaggagggagctgcctaaggtggggtagatgattggggtgaagtcgtaacaaggtatccctaccggaaggtggggttggatcacctcctt

SEQ ID NO: 92 - DNA, 1456 bp, Roseburia faecis
gatgaacgctggcggcgtgcttaacacatgcaagtcgaacgaagcactctatttgattttcttcggaaatgaagattttgtgactgagtggcggacgggtgagtaacgcgtgggtaacctgcctcatacagggggataacagttggaaacgactgctaataccgcataagcgcacaggatcgcatgatccggtgtgaaaaactccggtggtatgagatggacccgcgtctgattagccagttggcagggtaacggcctaccaaagcgacgatcagtagccgacctgagagggtgaccggccacattgggactgagacacggcccaaactcctacgggaggcagcagtggggaatattgcacaatgggggaaaccctgatgcagcgacgccgcgtgagcgaagaagtatttcggtatgtaaagctctatcagcagggaagaagaatgacggtacctgactaagaagcaccggctaaatacgtgccagcagccgcggtaatacgtatggtgcaagcgttatccggatttactgggtgtaaagggagcgcaggcggtgcggcaagtctgatgtgaaagcccggggctcaaccccggtactgcattggaaactgtcgtactagagtgtcggaggggtaagtggaattcctagtgtagcggtgaaatgcgtagatattaggaggaacaccagtggcgaaggcggcttactggacgataactgacgctgaggctcgaaagcgtggggagcaaacaggattagataccctggtagtccacgccgtaaacgatgaatactaggtgtcggggagcattgctcttcggtgccgcagcaaacgcaataagtattccacctggggagtacgttcgcaagaatgaaactcaaaggaattgacggggacccgcacaagcggtggagcatgtggtttaattcgaagcaacgcgaagaaccttaccaagtcttgacatcccgatgacagagtatgtaatgtacyttctcttcggagcatcggtgacaggtggtgcatggttgtcgtcagctcgtgtcgtgagatgttgggttaagtcccgcaacgagcgcaacccctgtccttagtagccagcggttcggccgggcactctagggagactgccagggataacctggaggaaggcggggatgacgtcaaatcatcatgccccttatgacttgggctacacacgtgctacaatggcgtaaacaaagggaagcggagccgtgaggccgagcaaatctcaaaaataacgtctcagttcggactgtagtctgcaacccgactacacgaagctggaatcgctagtaatcgcagatcagaatgctgcggtgaatacgttcccgggtcttgtacacaccgcccgtcacaccatgggagttggaaatgcccgaagtcagtgacccaaccgcaaggagggagctgccgaaggcaggttcgataactggggtg

SEQ ID NO: 93 - DNA, 1465 bp, Flavonifractor plautii
cgctggcggcgtgcttaacacatgcaagtcgaacggggtgctcatgacggaggattcgtccaatggattgagttacctagtggcggacgggtgagtaacgcgtgaggaacctgccttggagaggggaataacactccgaaaggagtgctaataccgcatgaagcagttgggtcgcatggctctgactgccaaagatttatcgctctgagatggcctcgcgtctgattagctagtaggcggggtaacggcccacctaggcgacgatcagtagccggactgagaggttgaccggccacattgggactgagacacggcccagactcctacgggaggcagcagtggggaatattgggcaatgggcgcaagcctgacccagcaacgccgcgtgaaggaagaaggctttcgggttgtaaacttcttttgtcggggacgaaacaaatgacggtacccgacgaataagccacggctaactacgtgccagcagccgcggtaatacgtaggtggcaagcgttatccggatttactgggtgtaaagggcgtgtaggcgggattgcaagtcagatgtgaaaactgggggctcaacctccagcctgcatttgaaactgtagttcttgagtgctggagaggcaatcggaattccgtgtgtagcggtgaaatgcgtagatatacggaggaacaccagtggcgaaggcggattgctggacagtaactgacgctgaggcgcgaaagcgtggggagcaaacaggattagataccctggtagtccacgccgtaaacgatggatactaggtgtggggggtctgaccccctccgtgccgcagttaacacaataagtatcccacctggggagtacgatcgcaaggttgaaactcaaaggaattgacgggggcccgcacaagcggtggagtatgtggtttaattcgaagcaacgcgaagaaccttaccagggcttgacatcccactaacgaggcagagatgcgttaggtgcccttcggggaaagtggagacaggtggtgcatggttgtcgtcagctcgtgtcgtgagatgttgggttaagtcccgcaacgagcgcaacccttattgttagttgctacgcaagagcactctagcgagactgccgttgacaaaacggaggaaggtggggacgacgtcaaatcatcatgccccttatgtcctgggccacacacgtactacaatggtggttaacagagggaggcaataccgcgaggtggagcaaatccctaaaagccatcccagttcggattgcaggctgaaacccgcctgtatgaagttggaatcgctagtaatcgcggatcagcatgccgcggtgaatacgttcccgggccttgtacacaccgcccgtcacaccatgagagtcgggaacacccgaagtccgtagcctaaccgcaaggagggcgcggccgaaggtgggttcgataattggggtgaagtcgtaacaaggtag

SEQ ID NO: 94 - DNA, 1438 bp, Blautia wexlerae
  misc_feature (19)..(19): n is a, c, g, t or u
caagtcgaacgggaattantttattgaaacttcggtcgatttaatttaattctagtggcggacgggtgagtaacgcgtgggtaacctgccttatacagggggataacagtcagaaatggctgctaataccgcataagcgcacagagctgcatggctcagtgtgaaaaactccggtggtataagatggacccgcgttggattagcttgttggtggggtaacggcccaccaaggcgacgatccatagccggcctgagagggtgaacggccacattgggactgagacacggcccagactcctacgggaggcagcagtggggaatattgcacaatgggggaaaccctgatgcagcgacgccgcgtgaaggaagaagtatctcggtatgtaaacttctatcagcagggaagatagtgacggtacctgactaagaagccccggctaactacgtgccagcagccgcggtaatacgtagggggcaagcgttatccggatttactgggtgtaaagggagcgtagacggtgtggcaagtctgatgtgaaaggcatgggctcaacctgtggactgcattggaaactgtcatacttgagtgccggaggggtaagcggaattcctagtgtagcggtgaaatgcgtagatattaggaggaacaccagtggcgaaggcggcttactggacggtaactgacgttgaggctcgaaagcgtggggagcaaacaggattagataccctggtagtccacgccgtaaacgatgaataactaggtgtcgggtggcaaagccattcggtgccgtcgcaaacgcagtaagtattccacctggggagtacgttcgcaagaatgaaactcaaaggaattgacggggacccgcacaagcggtggagcatgtggtttaattcgaagcaacgcgaagaaccttaccaagtcttgacatccgcctgaccgatccttaaccggatctttccttcgggacaggcgagacaggtggtgcatggttgtcgtcagctcgtgtcgtgagatgttgggttaagtcccgcaacgagcgcaacccctatcctcagtagccagcatttaaggtgggcactctggggagactgccagggataacctggaggaaggcggggatgacgtcaaatcatcatgccccttatgatttgggctacacacgtgctacaatggcgtaaacaaagggaagcgagattgtgagatggagcaaatcccaaaaataacgtcccagttcggactgtagtctgcaacccgactacacgaagctggaatcgctagtaatcgcggatcagaatgccgcggtgaatacgttcccgggtcttgtacacaccgcccgtcacaccatgggagtcagtaacgcccgaagtcagtgacctaactgcaaagaaggagctgccgaaggcgggaccgatgactggggtgaagtcgtaacaaggt

SEQ ID NO: 95 - DNA, 1365 bp, Anaerotruncus colihominis
aacggagcttacgttttgaagttttcggatggatgaatgtaagcttagtggcggacgggtgagtaacacgtgagcaacctgcctttcagagggggataacagccggaaacggctgctaataccgcatgatgttgcgggggcacatgcccctgcaaccaaaggagcaatccgctgaaagatgggctcgcgtccgattagccagttggcggggtaacggcccaccaaagcgacgatcggtagccggactgagaggttgaacggccacattgggactgagacacggcccagactcctacgggaggcagcagtgggggatattgcacaatgggcgaaagcctgatgcagcgacgccgcgtgagggaagacggtcttcggattgtaaacctctgtctttggggaagaaaatgacggtacccaaagaggaagctccggctaactacgtgccagcagccgcggtaatacgtagggagcaagcgttgtccggaattactgggtgtaaagggagcgtaggcgggatggcaagtagaatgttaaatccatcggctcaaccggtggctgcgttctaaactgccgttcttgagtgaagtagaggcaggcggaattcctagtgtagcggtgaaatgcgtagatattaggaggaacaccagtggcgaaggcggcctgctgggctttaactgacgctgaggctcgaaagcgtggggagcaaacaggattagataccctggtagtccacgccgtaaacgatgattactaggtgtggggggactgaccccttccgtgccgcagttaacacaataagtaatccacctggggagtacggccgcaaggttgaaactcaaaggaattgacgggggcccgcacaagcagtggagtatgtggtttaattcgaagcaacgcgaagaaccttaccaggtcttgacatcggcgtaatagcctagagagtaggtgaagcccttcggggcatccagacaggtggtgcatggttgtcgtcagctcgtgtcgtgagatgttgggttaagtcccgcaacgagcgcaacccttattattagttgctacgcaagagcactctaatgagactgccgttgacaaaacggaggaaggtggggatgacgtcaaatcatcatgccccttatgacctgggctacacacgtactacaatggcactaaaacagagggcggcgacaccgcgaggtgaagcgaatcccagaaaaagtgtctcagttcagattgcaggctgcaacccgcctgcatgaagtcggaattgctagtaatcgcggatcagcatgccgcggtgaatacgttcccgggccttgtacacaccgcccgtcacaccatgggagtccgggtaacacccgaagccagtag

SEQ ID NO: 96 - DNA, 1404 bp, Ruminococcus faecis
atgcaagtcgaacgaagcaccttgatttgattcttcggatgaagatcttggtgactgagtggcggacgggtgagtaacgcgtgggtaacctgcctcatacagggggataacagttagaaatgactgctaataccgcataagaccacagcaccgcatggtgcaggggtaaaaactccggtggtatgagatggacccgcgtctgattaggtagttggtggggtaacggcctaccaagccgacgatcagtagccgacctgagagggtgaccggccacattgggactgagacacggcccaaactcctacgggaggcagcagtggggaatattgcacaatgggggaaaccctgatgcagcgacgccgcgtgagcgatgaagtatttcggtatgtaaagctctatcagcagggaagaaaatgacggtacctgactaagaagcaccggctaaatacgtgccagcagccgcggtaatacgtatggtgcaagcgttatccggatttactgggtgtaaagggagcgtagacggagtggcaagtctgatgtgaaaacccggggctcaaccccgggactgcattggaaactgtcaatctagagtaccggagaggtaagcggaattcctagtgtagcggtgaaatgcgtagatattaggaggaacaccagtggcgaaggcggcttactggacggtaactgacgttgaggctcgaaagcgtggggagcaaacaggattagataccctggtagtccacgccgtaaacgatgactactaggtgtcgggcagcaaagctgttcggtgccgcagcaaacgcaataagtagtccacctggggagtacgttcgcaagaatgaaactcaaaggaattgacggggacccgcacaagcggtggagcatgtggtttaattcgaagcaacgcgaagaaccttacctgctcttgacatctccctgaccggcaagtaatgttgcctttccttcgggacagggatgacaggtggtgcatggttgtcgtcagctcgtgtcgtgagatgttgggttaagtcccgcaacgagcgcaacccctatctttagtagccagcggtttggccgggcactctagagagactgccagggataacctggaggaaggtggggatgacgtcaaatcatcatgccccttatgagcagggctacacacgtgctacaatggcgtaaacaaagggaggcagaaccgcgaggtcgagcaaatcccaaaaataacgtctcagttcggattgtagtctgcaactcgactacatgaagctggaatcgctagtaatcgcgaatcagaatgtcgcggtgaatacgttcccgggtcttgtacacaccgcccgtcacaccatgggagtcagtaacgcccgaagtcagtgacccaaccgtaaggaggagctgccgaag

SEQ ID NO: 97 - DNA, 1316 bp, Dorea longicatena
taacgcgtgggtaacctgcctcatacagggggataacagttagaaatgactgctaataccgcataagaccacgtaccgcatggtacagtggtaaaaactccggtggtatgagatggacccgcgtctgattaggtagttggtggggtaacggcctaccaagccgacgatcagtagccgacctgagagggtgaccggccacattgggactgagacacggcccagactcctacgggaggcagcagtggggaatattgcacaatggaggaaactctgatgcagcgacgccgcgtgaaggatgaagtatttcggtatgtaaacttctatcagcagggaagaaaatgacggtacctgactaagaagccccggctaactacgtgccagcagccgcggtaatacgtagggggcaagcgttatccggatttactgggtgtaaagggagcgtagacggcacggcaagccagatgtgaaaagcccggggctcaaccccgggactgcatttggaactgctgagctagagtgtcggagaggcaagtggaattcctagtgtagcggtgaaatgcgtagatattaggaggaacaccagtggcgaaggcggcttgctggacgatgactgacgttgaggctcgaaagcgtggggagcaaacaggattagataccctggtagtccacgccgtaaacgatgactgctaggtgtcgggtggcaaagccattcggtgccgcagctaacgcaataagcagtccacctggggagtacgttcgcaagaatgaaactcaaaggaattgacggggacccgcacaagcggtggagcatgtggtttaattcgaagcaacgcgaagaaccttacctgatcttgacatcccgatgaccgcttcgtaatggaagtttttcttcggaacatcggtgacaggtggtgcatggttgtcgtcagctcgtgtcgtgagatgttgggttaagtcccgcaacgagcgcaacccctatcttcagtagccagcaggttaagctgggcactctggagagactgccagggataacctggaggaaggtggggatgacgtcaaatcatcatgccccttatgaccagggctacacacgtgctacaatggcgtaaacaaagagaagcgaactcgcgagggtaagcaaatctcaaaaataacgtctcagttcggattgtagtctgcaactcgactacatgaagctggaatcgctagtaatcgcagatcagaatgctgcggtgaatacgttcccgggtcttgtacacaccgcccgtcacaccatgggagtcataacgcccgaagtcagtgacccaaccgtaagg

SEQ ID NO: 98 - DNA, 1475 bp, Clostridium innocuum
  misc_feature (905)..(905): n is a, c, g, t or u
  misc_feature (942)..(942): n is a, c, g, t or u
atggagagtttgatcctggctcaggatgaacgctggcggcatgcctaatacatgcaagtcgaacgaagtcttcaggaagcttgcttccaaaaagacttagtggcgaacgggtgagtaacacgtaggtaacctgcccatgtgtccgggataactgctggaaacggtagctaaaaccggataggtatacggagcgcatgctctgtatattaaagcgcccttcaaggcgtgaacatggatggacctgcgacgcattagctagttggtgaggtaacggcccaccaaggcgatgatgcgtagccggcctgagagggtaaacggccacattgggactgagacacggcccaaactcctacgggaggcagcagtagggaattttcgtcaatgggggaaaccctgaacgagcaatgccgcgtgagtgaagaaggtcttcggatcgtaaagctctgttgtaagtgaagaacggctcatagaggaaatgctatgggagtgacggtagcttaccagaaagccacggctaactacgtgccagyagccgcggtaatacgtaggtggcaagcgttatccggaatcattgggcgtaaagggtgcgtaggtggcgtactaagtctgtagtaaaaggcaatggctcaaccattgtaagctatggaaactggtatgctggagtgcagaagagggcgatggaattccatgtgtagcggtaaaatgcgtagatatatggaggaacaccagtggcgaaggcggtcgcctggtctgtaactgacactgaggcacgaaagcgtggggagcaaataggattagataccctagtagtccacgccgtaaacgatgagaactaagtgttggagaaattcagtgctgcagttaacgcaataagttctccgcctggggagtatgcacgcaagttngaaactcaaaggaattgacgggggcccgcacaagcgntggagtatgtggtttaattcgaagcaacgcgaagaaccttaccaggccttgacatggaaacaaataccctagagatagggggataattatggatcacacaggtggtgcatggttgtcgtcagctcgtgtcgtgagatgttgggttaagtcccgcaacgagcgcaacccttgtcgcatgttaccagcatcaagttggggactcatgcgagactgccggtgacaaaccggaggaaggtggggatgacgtcaaatcatcatgccccttatggcctgggctacacacgtactacaatggcgaccacaaagagcagcgacttggtgacaagaagcgaatctcataaagatcgtctcagttcggattgaagtctgcaactcgacttcatgaagtcggaatcgctagtaatcgcagatcagcatgctgcggtgaatacgttctcgggccttgtacacaccgcccgtcaaaccatgggagtcagtaatacccgaagccggtggcataaccgtaaggagtgagccgtcgaaggtaggaccga

SEQ ID NO: 99 - DNA, 1492 bp, Blautia hansenii
agagtttgatcctggctcaggatgaacgctggcggcgtgcttaacacatgcaagtcgagcgaagcacttatcattgactcttcggaagatttgatatttgactgagcggcggacgggtgagtaacgcgtgggtaacctgcctcatacaggggaataacagttagaaatggctgctaatgccgcataagcgcacaggaccgcatggtctggtgtgaaaaactgaggtggtatgagatggacccgcgtctgattaggtagttggtggggtaacggcctaccaagccgacgatcagtagccggcctgagagggtgaacggccacattgggactgagacacggcccagactcctacgggaggcagcagtggggaatattgcacaatgggggaaaccctgatgcagcgacgccgcgtgaaggaagaagtatctcggtatgtaaacttctatcagcagggaagaaaatgacggtacctgactaagaagccccggctaactacgtgccagcagccgcggtaatacgtagggggcaagcgttatccggatttactgggtgtaaagggagcgtagacggaagagcaagtctgatgtgaaaggctggggcttaaccccaggactgcattggaaactgtttttctagagtgccggagaggtaagcggaattcctagtgtagcggtgaaatgcgtagatattaggaggaacaccagtggcgaaggcggcttactggacggtaactgacgttgaggctcgaaagcgtggggagcaaacaggattagataccctggtagtccacgccgtaaacgatgaatactaggtgtcggggtgcaaagcagttcggtgccgcagcaaacgcaataagtattccacctggggagtacgttcgcaagaatgaaactcaaaggaattgacggggacccgcacaagcggtggagcatgtggtttaattcgaagcaacgcgaagaaccttaccaagtcttgacatctgcctgaccgttccttaaccggagctttccttcgggacaggcaagacaggtggtgcatggttgtcgtcagctcgtgtcgtgagatgttgggttaagtcccgcaacgagcgcaacccctatccttagtagccagcagtccggctgggcactctagggagactgccggggataacccggaggaaggcggggacgacgtcaaatcatcatgccccttatgatttgggctacacacgtgctacaatggcgtaaacaaagggaagcgaagcggtgacgcttagcaaatctcaaaaataacgtcccagttcggactgcagtctgcaactcgactgcacgaagctggaatcgctagtaatcgcgaatcagaatgtcgcggtgaatacgttcccgggtcttgtacacaccgcccgtcacaccatgggagtcagtaacgcccgaagtcagtgacccaaccttatggagggagctgccgaaggcgggaccgataactggggtgaagtcgtaacaaggtaacc

SEQ ID NO: 100 - DNA, 1473 bp, Bacteroides cellulosilyticus
agagtttgatcctggctcaggatgaacgctagctacaggcttaacacatgcaagtcgaggggcagcatgacctagcaataggttgatggcgaccggcgcacgggtgagtaacacgtatccaacctaccggttattccgggatagcctttcgaaagaaagattaataccggatagtataacgagaaggcatctttttgttattaaagaatttcgataaccgatggggatgcgttccattagtttgttggcggggtaacggcccaccaagacatcgatggataggggttctgagaggaaggtcccccacattggaactgagacacggtccaaactcctacgggaggcagcagtgaggaatattggtcaatggacgagagtctgaaccagccaagtagcgtgaaggatgactgccctatgggttgtaaacttcttttatatgggaataaagtgagccacgtgtggctttttgtatgtaccatacgaataaggatcggctaactccgtgccagcagccgcggtaatacggaggatccgagcgttatccggatttattgggtttaaagggagcgtaggcggactattaagtcagctgtgaaagtttgcggctcaaccgtaaaattgcagttgatactggtcgtcttgagtgcagtagaggtaggcggaattcgtggtgtagcggtgaaatgcttagatatcacgaagaactccgattgcgaaggcagcttactggactgtaactgacgctgatgctcgaaagtgtgggtatcaaacaggattagataccctggtagtccacacagtaaacgatgaatactcgctgtttgcgatatacagcaagcggccaagcgaaagcattaagtattccacctggggagtacgccggcaacggtgaaactcaaaggaattgacgggggcccgcacaagcggaggaacatgtggtttaattcgatgatacgcgaggaaccttacccgggcttaaattgcatctgaataatttggaaacagattagccgcaaggcagatgtgaaggtgctgcatggttgtcgtcagctcgtgccgtgaggtgtcggcttaagtgccataacgagcgcaacccttatctttagttactaacaggtcatgctgaggactctagagagactgccgtcgtaagatgtgaggaaggtggggatgacgtcaaatcagcacggcccttacgtccggggctacacacgtgttacaatggggggtacagaaggcagctacacagcgatgtgatgctaatcccaaaagcctctctcagttcggattggagtctgcaacccgactccatgaagctggattcgctagtaatcgcgcatcagccacggcgcggtgaatacgttcccgggccttgtacacaccgcccgtcaagccatgaaagccgggggtacctgaagtccgtaaccgcaaggagcggcctagggtaaaactggtaattggggctaagtcgta

SEQ ID NO: 101 - DNA, 1459 bp, Bacteroides ovatus
ggctcaggatgaacgctagctacaggcttaacacatgcaagtcgaggggcagcattttagtttgcttgcaaactgaagatggcgaccggcgcacgggtgagtaacacgtatccaacctgccgataactccggaatagcctttcgaaagaaagattaataccggatagcatacgaatatcgcatgatatttttattaaagaatttcggttatcgatggggatgcgttccattagtttgttggcggggtaacggcccaccaagactacgatggataggggttctgagaggaaggtcccccacattggaactgagacacggtccaaactcctacgggaggcagcagtgaggaatattggtcaatgggcgagagcctgaaccagccaagtagcgtgaaggatgaaggctctatgggtcgtaaacttcttttatatgggaataaagttttccacgtgtggaattttgtatgtaccatatgaataaggatcggctaactccgtgccagcagccgcggtaatacggaggatccgagcgttatccggatttattgggtttaaagggagcgtaggtggattgttaagtcagttgtgaaagtttgcggctcaaccgtaaaattgcagttgaaactggcagtcttgagtacagtagaggtgggcggaattcgtggtgtagcggtgaaatgcttagatatcacgaagaactccgattgcgaaggcagctcactagactgttactgacactgatgctcgaaagtgtgggtatcaaacaggattagataccctggtagtccacacagtaaacgatgaatactcgctgtttgcgatatacagtaagcggccaagcgaaagcattaagtattccacctggggagtacgccggcaacggtgaaactcaaaggaattgacgggggcccgcacaagcggaggaacatgtggtttaattcgatgatacgcgaggaaccttacccgggcttaaattgcaacagaatatattggaaacagtatagccgtaaggctgttgtgaaggtgctgcatggttgtcgtcagctcgtgccgtgaggtgtcggcttaagtgccataacgagcgcaacccttatctttagttactaacaggttatgctgaggactctagagagactgccgtcgtaagatgtgaggaaggtggggatgacgtcaaatcagcacggcccttacgtccggggctacacacgtgttacaatggggggtacagaaggcagctacctggcgacaggatgctaatcccaaaaacctctctcagttcggatcgaagtctgcaacccgacttcgtgaagctggattcgctagtaatcgcgcatcagccatggcgcggtgaatacgttcccgggccttgtacacaccgcccgtcaagccatgaaagccgggggtacctgaagtacgtaaccgcaaggagcgtcctagggtaaaactggtaattggggcta

SEQ ID NO: 102 - DNA, 1526 bp, Eubacterium fissicatena
tagagtttgatcctggctcaggatgaacgctggcggcgtgcttaacacatgcaagtcgagcgaagcgctttacttagatttcttcggattgaagagttttgcgactgagcggcggacgggtgagtaacgcgtgggtaacctgcctcatacagggggataacagttagaaatgactgctaataccgcataagaccacagtaccgcatggtacagtgggaaaaactccggtggtatgagatggacccgcgtctgattagctagttggtaaggtaacggcttaccaaggcgacgatcagtagccgacctgagagggtgaccggccacattgggactgagacacggcccaaactcctacgggaggcagcagtggggaatattgcacaatgggggaaaccctgatgcagcgacgccgcgtgaaggatgaagtatttcggtatgtaaacttctatcagcagggaagaaaatgacggtacctgactaagaagccccggctaactacgtgccagcagccgcggtaatacgtagggggcaagcgttatccggatttactgggtgtaaagggagcgtagacggttatgtaagtctgatgtgaaaacccggggctcaaccccgggactgcattggaaactatgtaactagagtgtcggagaggtaagtggaattcctagtgtagcggtgaaatgcgtagatattaggaggaacaccagtggcgaaggcggcttactggacgatcactgacgttgaggctcgaaagcgtggggagcaaacaggattagataccctggtagtccacgccgtaaacgatgaatactaggtgtcgggtggcaaagccattcggtgccgcagcaaacgcaataagtattccacctggggagtacgttcgcaagaatgaaactcaaaggaattgacggggacccgcacaagcggtggagcatgtggtttaattcgaagcaacgcgaagaaccttacctgctcttgacatcccactgaccggcgtgtaatggcgccttcccttcggggcagtggagacaggtggtgcatggttgtcgtcagctcgtgtcgtgagatgttgggttaagtcccgcaacgagcgcaacccttatctttagtagccagcggtttggccgggcactctagagagactgccagggataacctggaggaaggtggggatgacgtcaaatcatcatgccccttatgagcagggctacacacgtgctacaatggcgtaaacaaagggaggcaataccgcgaggttgagcaaatcccaaaaataacgtctcagttcggattgtagtctgcaactcgactacatgaagctggaatcgctagtaatcgcgaatcagaatgtcgcggtgaatacgttcccgggtcttgtacacaccgcccgtcacaccatgggagttggtaacgcccgaagtcagtgacccaaccgtaaggagggagctgccgaaggcgggatcgataactggggtgaagtcgtaacaaggtagccgtatcggaaggtgcggctggatcacctcctt

SEQ ID NO: 103 - DNA, 1493 bp, Blautia coccoides
agagtttgatcctggctcaggatgaacgctggcggcgtgcttaacacatgcaagtcgagcgaagcgctaagacagatttcttcggattgaagtctttgtgactgagcggcggacgggtgagtaacgcgtgggtaacctgcctcatacagggggataacagttagaaatgactgctaataccgcataagcgcacaggaccgcatggtctggtgtgaaaaactccggtggtatgagatggacccgcgtctgattagctagttggaggggtaacggcccaccaaggcgacgatcagtagccggcctgagagggtgaacggccacattgggactgagacacggcccagactcctacgggaggcagcagtggggaatattgcacaatgggggaaaccctgatgcagcgacgccgcgtgaaggaagaagtatctcggtatgtaaacttctatcagcagggaagaaaatgacggtacctgactaagaagccccggctaactacgtgccagcagccgcggtaatacgtagggggcaagcgttatccggatttactgggtgtaaagggagcgtagacggaagagcaagtctgatgtgaaaggctggggcttaaccccaggactgcattggaaactgttgttctagagtgccggagaggtaagcggaattcctagtgtagcggtgaaatgcgtagatattaggaggaacaccagtggcgaaggcggcttactggacggtaactgacgttgaggctcgaaagcgtggggagcaaacaggattagataccctggtagtccacgccgtaaacgatgaatactaggtgtcgggtggcaaagccattcggtgccgcagcaaacgcaataagtattccacctggggagtacgttcgcaagaatgaaactcaaaggaattgacggggacccgcacaagcggtggagcatgtggtttaattcgaagcaacgcgaagaaccttaccaagtcttgacatccctctgaccgtcccgtaacgggggcttcccttcggggcagaggagacaggtggtgcatggttgtcgtcagctcgtgtcgtgagatgttgggttaagtcccgcaacgagcgcaacccttatccttagtagccagcacatgatggtgggcactctagggagactgccggggataacccggaggaaggcggggacgacgtcaaatcatcatgccccttatgatttgggctacacacgtgctacaatggcgtaaacaaagggaagcgagacagcgatgttgagcgaatcccaaaaataacgtcccagttcggactgcagtctgcaactcgactgcacgaagctggaatcgctagtaatcgcggatcagaatgccgcggtgaatacgttcccgggtcttgtacacaccgcccgtcacaccatgggagtcagtaacgcccgaagtcagtgacctaaccgaaaggaaggagctgccgaaggcgggaccgataactggggtgaagtcgtaacaaggtaacc

SEQ ID NO: 104 - DNA, 1262 bp, Blautia faecis
ataacagccagaaatgactgctaataccgcataagcgcacagaaccgcatggttcggtgtgaaaaactccggtggtataagatggacccgcgttggattagctagttggcagggcagcggcctaccaaggcgacgatccatagccggcctgagagggtgaacggccacattgggactgagacacggcccagactcctacgggaggcagcagtggggaatattgcacaatgggggaaaccctgatgcagcgacgccgcgtgaaggaagaagtatctcggtatgtaaacttctatcagcagggaagataatgacggtacctgactaagaagccccggctaactacgtgccagcagccgcggtaatacgtagggggcaagcgttatccggatttactgggtgtaaagggagcgtagacggcgcagcaagtctgatgtgaaaggcaggggcttaacccctggactgcattggaaactgctgtgcttgagtgccggaggggtaagcggaattcctagtgtagcggtgaaatgcgtagatattaggaggaacaccagtggcgaaggcggcttactggacggtaactgacgttgaggctcgaaagcgtggggagcaaacaggattagataccctggtagtccacgccgtaaacgatgaatactaggtgtcagggagcacagctctttggtgccgccgcaaacgcattaagtattccacctggggagtacgttcgcaagaatgaaactcaaaggaattgacggggacccgcacaagcggtggagcatgtggtttaattcgaagcaacgcgaagaaccttaccaaatcttgacatccctctgaccgggacttaaccgtccctttccttcgggacaggggagacaggtggtgcatggttgtcgtcagctcgtgtcgtgagatgttgggttaagtcccgcaacgagcgcaacccctatccttagtagccagcacgcartggtgggcactctgaggagactgccagggataacctggaggaaggcggggatgacgtcaaatcatcatgccccttatgatttgggctacacacgtgctacaatggcgtaaacaaagggaagcgaacccgcgagggtgggcaaatctcaaaaataacgtcccagttcggactgcagtctgcaactcgactgcacgaagctggaatcgctagtaatcgcggatcagaatgccgcggtgaatacgttcccgggtcttgtacacaccgcccgtcacaccatgggagtcagtaacgcccg

SEQ ID NO: 105 - DNA, 1431 bp, Clostridium hathewayi
  misc_feature (191)..(191): n is a, c, g, t or u
  misc_feature (211)..(211): n is a, c, g, t or u
  misc_feature (248)..(248): n is a, c, g, t or u
  misc_feature (979)..(979): n is a, c, g, t or u
ctcaggatgaacgctggcggcgtgcttaacacatgcaagtcgagcgaagcggtttcaatgaagttttcggatggatttgaaattgacttagcggcggacgggtgagtaacgcgtgggtaacctgccttacactgggggataacagttagaaatgactgctaataccgcataagcgcacagggccgcatggnctggtgtgaaaaactccggnggtgtaagatggacccgcgtctgattaggtagttggnggggtaacggcccaccaagccgacgatcagtagccgacctgagagggtgaccggccacattgggactgagacacggcccaaactcctacgggaggcagcagtggggaatattggacaatgggcgaaagcctgatccagcgacgccgcgtgagtgaagaagtatttcggtatgtaaagctctatcagcagggaagaaaatgacggtacctgactaagaagccccggctaactacgtgccagcagccgcggtaatacgtagggggcaagcgttatccggatttactgggtgtaaagggagcgtagacggtttagcaagtctgaagtgaaagcccggggctcaaccccggtactgctttggaaactgttagacttgagtgcaggagaggtaagtggaattcctagtgtagcggtgaaatgcgtagatattaggaggaacaccagtggcgaaggcggcttactggactgtaactgacgttgaggctcgaaagcgtggggagcaaacaggattagataccctggtagtccacgccgtaaacgatgaatactaggtgtcggggggcaaagcccttcggtgccgccgcaaacgcaataagtattccacctggggagtacgttcgcaagaatgaaactcaaaggaattgacggggacccgcacaagcggtggagcatgtggtttaattcgaagcaacgcgaagaaccttaccaagtcttgacatcccactgaaaacacnttaaccgtgatccctcttcggagcagtggagacaggtggtgcatggttgtcgtcagctcgtgtcgtgagatgttgggttaagtcccgcaacgagcgcaacccttatccttagtagccagcgagtagagtcgggcactctggggagactgccagggataacctggaggaaggtggggatgacgtcaaatcatcatgccccttatgatttgggctacacacgtgctacaatggcgtaaacaaagggaggcaaaggagcgatctggagcaaaccccaaaaataacgtctcagttcggattgcaggctgcaactcgcctgcatgaagctggaatcgctagtaatcgcgaatcagaatgtcgcggtgaatacgttcccgggtcttgtacacaccgcccgtcacaccatgggagttggtaacgcccgaagtcagtgacccaaccgaaaggagggagct

SEQ ID NO: 106 - DNA, 1493 bp, Blautia producta
agagtttgatcctggctcaggatgaacgctggcggcgtgcttaacacatgcaagtcgagcgaagcactaagacggatttcttcggattgaagtctttgtgactgagcggcggacgggtgagtaacgcgtgggtaacctgcctcatacagggggataacagttagaaatgactgctaataccgcataagcgcacaggaccgcatggtctggtgtgaaaaactccggtggtatgagatggacccgcgtctgattagctagttggaggggtaacggcccaccaaggcgacgatcagtagccggcctgagagggtgaacggccacattgggactgagacacggcccagactcctacgggaggcagcagtggggaatattgcacaatgggggaaaccctgatgcagcgacgccgcgtgaaggaagaagtatctcggtatgtaaacttctatcagcagggaagaaaatgacggtacctgactaagaagccccggctaactacgtgccagcagccgcggtaatacgtagggggcaagcgttatccggatttactgggtgtaaagggagcgtagacggaagagcaagtctgatgtgaaaggctggggcttaaccccaggactgcattggaaactgttgttctagagtgccggagaggtaagcggaattcctagtgtagcggtgaaatgcgtagatattaggaggaacaccagtggcgaaggcggcttactggacggtaactgacgttgaggctcgaaagcgtggggagcaaacaggattagataccctggtagtccacgccgtaaacgatgaatactaggtgtcgggtggcaaagccattcggtgccgcagcaaacgcaataagtattccacctggggagtacgttcgcaagaatgaaactcaaaggaattgacggggacccgcacaagcggtggagcatgtggtttaattcgaagcaacgcgaagaaccttaccaagtcttgacatccctctgaccgtcccgtaacggggacttcccttcggggcagaggagacaggtggtgcatggttgtcgtcagctcgtgtcgtgagatgttgggttaagtcccgcaacgagcgcaacccttatccttagtagccagcacatgatggtgggcactctagggagactgccggggataacccggaggaaggcggggacgacgtcaaatcatcatgccccttatgatttgggctacacacgtgctacaatggcgtaaacaaagggaagcgagacagcgatgttgagcgaatcccaaaaataacgtcccagttcggactgcagtctgcaactcgactgcacgaagctggaatcgctagtaatcgcggatcagaatgccgcggtgaatacgttcccgggtcttgtacacaccgcccgtcacaccatgggagtcagtaacgcccgaagtcagtgacctaaccgaaaggaaggagctgccgaaggcgggaccgataactggggtgaagtcgtaacaaggtaacc

SEQ ID NO: 107 - DNA, 1515 bp, Anaerostipes hadrus
tggctcaggatgaacgctggcggcgtgcttaacacatgcaagtcgaacgaagctgcttaactgatcttcttcggaattgacgttttgtagactgagtggcggacgggtgagtaacgcgtgggcaacctgccctgtacagggggataacagtcagaaatgactgctaataccgcataagaccacagcaccgcatggtgcaggggtaaaaactccggtggtacaggatggacccgcgtctgattagctggttggtgaggtaacggctcaccaaggcgacgatcagtagccggcttgagagagtgaacggccacattgggactgagacacggcccaaactcctacgggaggcagcagtggggaatattgcacaatgggggaaaccctgatgcagcgacgccgcgtgagtgaagaagtatctcggtatgtaaagctctatcagcagggaagaaaatgacggtacctgactaagaagccccggctaactacgtgccagcagccgcggtaatacgtagggggcaagcgttatccggaattactgggtgtaaagggtgcgtaggtggtatggcaagtcagaagtgaaaacccagggcttaactctgggactgcttttgaaactgtcagactggagtgcaggagaggtaagcggaattcctagtgtagcggtgaaatgcgtagatattaggaggaacatcagtggcgaaggcggcttactggactgaaactgacactgaggcacgaaagcgtggggagcaaacaggattagataccctggtagtccacgccgtaaacgatgaatactaggtgtcggggccgtagaggcttcggtgccgcagccaacgcagtaagtattccacctggggagtacgttcgcaagaatgaaactcaaaggaattgacggggacccgcacaagcggtggagcatgtggtttaattcgaagcaacgcgaagaaccttacctggtcttgacatccttctgaccggtccttaaccggacctttccttcgggacaggagagacaggtggtgcatggttgtcgtcagctcgtgtcgtgagatgttgggttaagtcccgcaacgagcgcaacccctatctttagtagccagcatttcaggtgggcactctagagagactgccagggataacctggaggaaggtggggacgacgtcaaatcatcatgccccttatgaccagggctacacacgtgctacaatggcgtaaacagagggaagcagcctcgtgagagtgagcaaatcccaaaaataacgtctcagttcggattgtagtctgcaactcgactacatgaagctggaatcgctagtaatcgcgaatcagaatgtcgcggtgaatacgttcccgggtcttgtacacaccgcccgtcacaccatgggagtcagtaacgcccgaagtcagtgacccaaccgtaaggagggagctgccgaaggcgggaccgataactggggtgaagtcgtaacaaggtagccgtatcggaaggtgcggctggatcacctcctttc

SEQ ID NO: 108 - DNA, 1523 bp, Eubacterium fissicatena
gtttgatcctggctcaggatgaacgctggcggcgtgcttaacacatgcaagtcgagcgaagcgctttacttagatttcttcggattgaagagttttgcgactgagcggcggacgggtgagtaacgcgtgggtaacctgcctcatacagggggataacagttagaaatgactgctaataccgcataagaccacagtaccgcatggtacagtgggaaaaactccggtggtatgagatggacccgcgtctgattagctagttggtaaggtaacggcttaccaaggcaacgatcagtagccgacctgagagggtgaccggccacattgggactgagacacggcccaaactcctacgggaggcagcagtggggaatattgcacaatgggggaaaccctgatgcagcgacgccgcgtgaaggatgaagtatttcggtatgtaaacttctatcagcagggaagaaaatgacggtacctgactaagaagccccggctaactacgtgccagcagccgcggtaatacgtagggggcaagcgttatccggatttactgggtgtaaagggagcgtagacggttatgtaagtctgatgtgaaaacccggggctcaaccccgggactgcattggaaactatgtaactagagtgtcggagaggtaagtggaattcctagtgtagcggtgaaatgcgtagatattaggaggaacaccagtggcgaaggcggcttactggacgatcactgacgttgaggctcgaaagcgtggggagcaaacaggattagataccctggtagtccacgccgtaaacgatgaatactaggtgtcgggtggcaaagccattcggtgccgcagcaaacgcaataagtattccacctggggagtacgttcgcaagaatgaaactcaaaggaattgacggggacccgcacaagcggtggagcatgtggtttaattcgaagcaacgcgaagaaccttacctgctcttgacatcccactgaccggcgtgtaatggcgccttcccttcggggcagtggagacaggtggtgcatggttgtcgtcagctcgtgtcgtgagatgttgggttaagtcccgcaacgagcgcaacccttatctttagtagccagcggtttggccgggcactctagagagactgccagggataacctggaggaaggtggggatgacgtcaaatcatcatgccccttatgagcagggctacacacgtgctacaatggcgtaaacaaagggaggcaataccgcgaggttgagcaaatcccaaaaataacgtctcagttcggattgtagtctgcaactcgactacatgaagctggaatcgctagtaatcgcgaatcagaatgtcgcggtgaatacgttcccgggtcttgtacacaccgcccgtcacaccatgggagttggtaacgcccgaagtcagtgacccaaccgtaaggagggagctgccgaaggcgggatcgataactggggtgaagtcgtaacaaggtagccgtatcggaaggtgcggctggatcacctccttt

SEQ ID NO: 109 - DNA, 1524 bp, Eubacterium contortum
tttgatcctggctcaggatgaacgctggcgacgtgcttaacacatgcaagtcgagcgaagcactttactttgatttcttcggaatgaaaggttttgtgactgagcggcggacgggtgagtaacgcgtgggtaacctgcctcatacagggggataacagttagaaatgactgctaataccgcataagaccacagtaccgcatggtacagtgggaaaaactccggtggtatgagatggacccgcgtctgattagctagttggtaaggtaacggcttaccaaggcgacgatcagtagccgacctgagagggtgaccggccacattgggactgagacacggcccaaactcctacgggaggcagcagtggggaatattgcacaatgggggaaaccctgatgcagcgacgccgcgtgaaggatgaagtatttcggtatgtaaacttctatcagcagggaagaaaatgacggtacctgactaagaagccccggctaactacgtgccagcagccgcggtaatacgtagggggcaagcgttatccggatttactgggtgtaaagggagcgtagacggttatgtaagtctgatgtgaaaacccggggctcaaccccgggactgcattggaaactatgtaactagagtgtcggagaggtaagtggaattcctagtgtagcggtgaaatgcgtagatattaggaggaacaccagtggcgaaggcggcttactggacgatgactgacgttgaggctcgaaagcgtggggagcaaacaggattagataccctggtagtccacgccgtaaacgatgaatactaggtgtcgggtggcaaagccattcggtgccgcagcaaacgcaataagtattccacctggggagtacgttcgcaagaatgaaactcaaaggaattgacggggacccgcacaagcggtggagcatgtggtttaattcgaagcaacgcgaagaaccttacctgctcttgacatccccctgaccggcgtgtaatggtgcctttccttcgggacaggggagacaggtggtgcatggttgtcgtcagctcgtgtcgtgagatgttgggttaagtcccgcaacgagcgcaacccttatctttagtagccagcggtttggccgggcactctagagagactgccagggataacctggaggaaggtggggatgacgtcaaatcatcatgccccttatgagcagggctacacacgtgctacaatggcgtaaacaaagggaggcgaagccgtgaggtggagcaaatcccaaaaataacgtctcagttcggattgtagtctgcaactcgactacatgaagctggaatcgctagtaatcgcgaatcagaatgtcgcggtgaatacgttcccgggtcttgtacacaccgcccgtcacaccatgggagttggtaacgcccgaagtcagtgacccaaccgcaaggagggagctgccgagggtgggaccgataactggggtgaagtcgtaacaaggtagccgtatcggaaggtgcggctggatcacctcctttct

SEQ ID NO: 110 - DNA, 1390 bp, Clostridium bolteae
ttttaattgactgagtggcggacgggtgagtaacgcgtggataacctgcctcacactgggggataacagttagaaatgactgctaataccgcataagcgcacagtaccgcatggtacagtgtgaaaaactccggtggtgtgagatggatccgcgtctgattagccagttggcggggtaacggcccaccaaagcgacgatcagtagccgacctgagagggtgaccggccacattgggactgagacacggcccaaactcctacgggaggcagcagtggggaatattgcacaatgggcgaaagcctgatgcagcgacgccgcgtgagtgaagaagtatttcggtatgtaaagctctatcagcagggaagaaaatgacggtacctgactaagaagccccggctaactacgtgccagcagccgcggtaatacgtagggggcaagcgttatccggatttactgggtgtaaagggagcgtagacggcgaagcaagtctgaagtgaaaacccagggctcaaccctgggactgctttggaaactgttttgctagagtgtcggagaggtaagtggaattcctagtgtagcggtgaaatgcgtagatattaggaggaacaccagtggcgaaggcggcttactggacgataactgacgttgaggctcgaaagcgtggggagcaaacaggattagataccctggtagtccacgccgtaaacgatgaatgctaggtgttggggggcaaagcccttcggtgccgtcgcaaacgcagtaagcattccacctggggagtacgttcgcaagaatgaaactcaaaggaattgacggggacccgcacaagcggtggagcatgtggtttaattcgaagcaacgcgaagaaccttaccaagtcttgacatcctcttgaccggcgtgtaacggcgccttcccttcggggcaagagagacaggtggtgcatggttgtcgtcagctcgtgtcgtgagatgttgggttaagtcccgcaacgagcgcaacccttatccttagtagccagcaggtaaagctgggcactctagggagactgccagggataacctggaggaaggtggggatgacgtcaaatcatcatgccccttatgatttgggctacacacgtgctacaatggcgtaaacaaagggaagcaagacagtgatgtggagcaaatcccaaaaataacgtcccagttcggactgtagtctgcaacccgactacacgaagctggaatcgctagtaatcgcgaatcagaatgtcgcggtgaatacgttcccgggtcttgtacacaccgcccgtcacaccatgggagtcagcaacgcccgaagtcagtgacccaactcgcaagagagggagctgccgaaggcggggcaggtaactggggtgaagtc

SEQ ID NO: 111 - DNA, 1308 bp, Blautia luti
  misc_feature (702)..(705): n is a, c, g, t or u
gtgggtaacctgccttatacagggggataacagtcagaaatgactgctaataccgcataagcgcacagagctgcatggctccggtgtgaaaaactccggtggtataagatggacccgcgttggattagctagttggtgaggtaacggcccaccaaggcgacgatccatagccggcctgagagggtgaacggccacattgggactgagacacggcccagactcctacgggaggcagcagtggggaatattgcacaatgggggaaaccctgatgcagcgacgccgcgtgaaggaagaagtatctcggtatgtaaacttctatcagcagggaagaaaatgacggtacctgactaagaagccccggctaactacgtgccagcagccgcggtaatacgtagggggcaagcgttatccggatttactgggtgtaaagggagcgtagacggcatggacaagtctgatgtgaaaggctggggctcaaccccgggactgcattggaaactgcccgtcttgagtgccggagaggtaagcggaattcctagtgtagcggtgaaatgcgtagatattaggaggaacaccagtggcgaaggcggcttactggacggtaactgacgttgaggctcgaaagcgtggggagcaaacaggattagataccctggtagtccacgcggtaaacgatgaatcctaggtgtcggggagcaaannnnttcggtgccgccgcaaacgcattaagcattccacctggggagtacgttcgcaagaatgaaactcaaaggaattgacggggacccgcacaagcggtggagcatgtggtttaattcgaagcaacgcgaagaaccttaccaagtcttgacatccctctgaccgagtatgtatggtacttttccttcgggagagagaggagacaggtggtgcatggttgtcgtcagctcgtgtcgtgagatgttgggttaagtcccgcaacgagcgcaacccctatccccagtagccagcggttcggccgggcactctgaggagactgccagggataacctggaggaaggcggggatgacgtcaaatcatcatgccccttatgatttgggctacacacgtgctacaatggcgtaaacaaagggaagcaagcctgcgagggtgggcaaatcccaaaaataacgtcccagttcggactgtagtctgcaacccgactacacgaagctggaatcgctagtaatcgcggatcagaatgccgcggtgaatacgttcccgggtcttgtacacaccgcccgtcacaccatgggagtcagtaacgcccgaagtcagtgacctaact

SEQ ID NO: 112 - DNA, 1489 bp, Acidaminococcus intestini
ctggcggcgtgcttaacacatgcaagtcgaacggagaacttatttcggtaagttcttagtggcgaacgggtgagtaacgcgtgggcaacctgccctccagttggggacaacattccgaaagggatgctaataccgaatgtcctccctcctccgcatggaggagggaggaaagatggcctctgcttgcaagctatcgctggaagatgggcccgcgtctgattagctagttggtggggtaacggctcaccaaggcgatgatcagtagccggtctgagaggatgaacggccacattgggactgagacacggcccaaactcctacgggaggcagcagtggggaatcttccgcaatggacgaaagtctgacggagcaacgccgcgtgagtgatgaaggtcttcggattgtaaaactctgttgttagggacgaaagcaccgtgttcgaacaggtcatggtgttgacggtacctaacgaggaagccacggctaactacgtgccagcagccgcggtaatacgtaggtggcaagcgttgtccggaattattgggcgtaaagagcatgtaggcgggcttttaagtctgacgtgaaaatgcggggcttaaccccgtatggcgttggatactggaagtcttgagtgcaggagaggaaaggggaattcccagtgtagcggtgaaatgcgtagatattgggaggaacaccagtggcgaaggcgcctttctggactgtgtctgacgctgagatgcgaaagccagggtagcaaacgggattagataccccggtagtcctggccgtaaacgatggatactaggtgtaggaggtatcgaccccttctgtgccggagttaacgcaataagtatcccgcctggggactacgatcgcaagattgaaactcaaaggaattgacgggggcccgcacaagcggtggagtatgtggtttaattcgacgcaacgcgaagaaccttaccaaggcttgacattgagtgaaagacctagagataggtccctcccttcggggacacgaaaacaggtggtgcatggctgtcgtcagctcgtgtcgtgagatgttgggttaagtcccgcaacgagcgcaacccctatcctatgttaccagcgcgtaaaggcggggactcataggagactgccagggataacttggaggaaggcggggatgacgtcaagtcatcatgccccttatgtcttgggctacacacgtactacaatggtcggcaacaaagggcagcgaaaccgcgaggtggagcaaatcccagaaacccgaccccagttcggatcgtaggctgcaacccgcctacgtgaagttggaatcgctagtaatcgcaggtcagcatactgcggtgaatacgttcccgggccttgtacacaccgcccgtcacaccacgaaagttggtaacacccgaagccggtgagataaccttttaggagtcagctgtctaaggtggggccgatgattggggtgaagtcgtaacaaggtagc

SEQ ID NO: 113 - DNA, 1500 bp, Ruminococcus albus
agagtttgatcctggctcaggacgaacgctggcggcacgcttaacacatgcaagtcgaacgagcgaaagagtgcttgcactctctagctagtggcggacgggtgagtaacacgtgagcaatctgcctttcggagagggataccaattggaaacgattgttaatacctcataacataacgaagccgcatgactttgttatcaaatgaatttcgccgaaagatgagctcgcgtctgattaggtagttggtgaggtaacggcccaccaagccgacgatcagtagccggactgagaggttgaacggccacattgggactgagacacggcccagactcctacgggaggcagcagtggggaatattgcacaatgggcgaaagcctgatgcagcgatgccgcgtgagggaagaaggttttaggattgtaaacctctgtctttggggacgataatgacggtacccaaggaggaagctccggctaactacgtgccagcagccgcggtaatacgtagggagcgagcgttgtccggaattactgggtgtaaagggagcgtaggcgggattgcaagtcaggtgtgaaatttaggggcttaacccctgaactgcacttgaaactgtagttcttgagtgaagtagaggtaagcggaattcctagtgtagcggtgaaatgcgtagatattaggaggaacatcagtggcgaaggcggcttactgggctttaactgacgctgaggctcgaaagcgtggggagcaaacaggattagataccctggtagtccacgccgtaaacgatgattactaggtgtggggggactgaccccttccgtgccgcagttaacacaataagtaatccacctggggagtacggccgcaaggctgaaactcaaaggaattgacggggacccgcacaagcagtggagtatgtggtttaattcgaagcaacgcgaagaaccttaccaggtcttgacatcgtacgcatagcatagagatatgtgaaatcccttcggggacgtatagacaggtggtgcatggttgtcgtcagctcgtgtcgtgagatgttggggttaagtcccgcaacgagcgcaacccttactgttagttgctacgcaagagcactctagcaggactgccgttgacaaaacggaggaaggtggggatgacgtcaaatcatcatgccccttatgacctgggctacacacgtactacaatggctgttaacagagggaagcaaaacagtgatgtggagcaaaaccctaaaagcagtcttagttcggattgtaggctgcaacccgcctacatgaagtcggaattgctagtaatcgcggatcagcatgccgcggtgaatacgttcccgggccttgtacacaccgcccgtcacgccatgggagtcggtaacacccgaagcctgtgttctaaccgcaaggaggaagcagtcgaaggtgggattgatgactggggtgaagtcgtaacaaggtagccgtatcggaaggtgcggctggatcacct

SEQ ID NO: 114 - DNA, 1521 bp, Eubacterium rectale
agagtttgatcctggctcaggatgaacgctggcggcgtgcttaacacatgcaagtcgaacgaagcactttatttgatttccttcgggactgattattttgtgactgagtggcggacgggtgagtaacgcgtgggtaacctgccttgtacagggggataacagttggaaacggctgctaataccgcataagcgcacggcatcgcatgatgcagtgtgaaaaactccggtggtataagatggacccgcgttggattagctagttggtgaggtaacggcccaccaaggcgacgatccatagccgacctgagagggtgaccggccacattgggactgagacacggcccaaactcctacgggaggcagcagtggggaatattgcacaatgggcgaaagcctgatgcagcgacgccgcgtgagcgaagaagtatttcggtatgtaaagctctatcagcagggaagataatgacggtacctgactaagaagcaccggctaaatacgtgccagcagccgcggtaatacgtatggtgcaagcgttatccggatttactgggtgtaaagggagcgcaggcggtgcggcaagtctgatgtgaaagcccggggctcaaccccggtactgcattggaaactgtcgtactagagtgtcggaggggtaagcggaattcctagtgtagcggtgaaatgcgtagatattaggaggaacaccagtggcgaaggcggcttactggacgataactgacgctgaggctcgaaagcgtggggagcaaacaggattagataccctggtagtccacgccgtaaacgatgaatactaggtgttgggaagcattgcttctcggtgccgtcgcaaacgcagtaagtattccacctggggagtacgttcgcaagaatgaaactcaaaggaattgacggggacccgcacaagcggtggagcatgtggtttaattcgaagcaacgcgaagaaccttaccaagtcttgacatccttctgaccggtacttaaccgtaccttctcttcggagcaggagtgacaggtggtgcatggttgtcgtcagctcgtgtcgtgagatgttgggttaagtcccgcaacgagcgcaacccttatctttagtagccagcggttcggccgggcactctagagagactgccagggataacctggaggaaggcggggatgacgtcaaatcatcatgccccttatgacttgggctacacacgtgctacaatggcgtaaacaaagggaagcaaagctgtgaagccgagcaaatctcaaaaataacgtctcagttcggactgtagtctgcaacccgactacacgaagctggaatcgctagtaatcgcagatcagaatgctgcggtgaatacgttcccgggtcttgtacacaccgcccgtcacaccatgggagttgggaatgcccgaagccagtgacctaaccgaaaggaaggagctgtcgaaggcaggctcgataactggggtgaagtcgtaacaaggtagccgtatcggaaggtgcggctggatcacct

SEQ ID NO: 115 - DNA, 1545 bp, Acidaminococcus fermentans
agagtttgatcctggctcaggacgaacgctggcggcgtgcttaacacatgcaagtcgaacggagaactttcttcggaatgttcttagtggcgaacgggtgagtaacgcgtaggcaacctgccctctggttggggacaacattccgaaagggatgctaataccgaatgagatcctctttccgcatggagagaggatgaaagatggcctctacttgtaagctatcgccagaagatgggcctgcgtctgattagctagtaggtgaggtaacggctcacctaggcgatgatcagtagccggtctgagaggatgaacggccacattgggactgagacacggcccaaactcctacgggaggcagcagtggggaatcttccgcaatggacgaaagtctgacggagcaacgccgcgtgagtgatgaaggccttcgggttgtaaaactctgttgtcagggacgaaagcaccgatctataatacattttggtgttgacggtacctgacgaggaagccacggctaactacgtgccagcagccgcggtaatacgtaggtggcaagcgttgtccggaattattgggcgtaaagagcatgtaggcgggcttttaagtccgacgtgaaaatgcggggcttaaccccgtatggcgttggatactggaagtcttgagtgcaggagaggaaaggggaattcccagtgtagcggtgaaatgcgtagatattgggaggaacaccagtggcgaaggcgcctttctggactgtgtctgacgctgagatgcgaaagccagggtagcaaacgggattagataccccggtagtcctggccgtaaacgatgggtactaggtgtaggaggtatcgaccccttctgtgccggagttaacgcaataagtaccccgcctggggactacgatcgcaagattgaaactcaaaggaattgacgggggcccgcacaagcggtggagtatgtggtttaattcgacgcaacgcgaagaaccttaccaaggcttgacattgagtgaaagacccagagatgggtccccttcttcggaagcacgaaaacaggtggtgcatggctgtcgtcagctcgtgtcgtgagatgttgggttaagtcccgcaacgagcgcaacccttatcctatgttaccagcacgtaatggtggggactcataggagactgccagggataacctggaggaaggcggggatgacgtcaagtcatcatgccccttatgtcttgggctacacacgtactacaatggtcggcaacaaagggcagcgaagccgcgaggcggagccaatcccagaaacccgaccccagttcggatcgcaggctgcaacccgcctgcgtgaagttggaatcgctagtaatcgcaggtcagcatactgcggtgaatacgttcccgggccttgtacacaccgcccgtcacaccacgaaagttggtaacacccgaagccggtgagataaccttttaggagtcagctgtctaaggtggggccgatgattggggtgaagtcgtaacaaggtagccgttcgagaacgagcggctggatcacct

SEQ ID NO: 116 - DNA, 1423 bp, Fusicatenibacter saccharivorans
tggctcaggatgaacgctggcggcgtgcttaacacatgcaagtcgagcgaagcagttaagaagattyttcggatgattcttgactgactgagcggcggacgggtgagtaacgcgtgggtgacctgccccataccgggggataacagctggaaacggctgctaataccgcataagcgcacagagctgcatggctcggtgtgaaaaactccggtggtatgggatgggcccgcgtctgattaggcagttggcggggtaacggcccaccaaaccgacgatcagtagccggcctgagagggcgaccggccacattgggactgagacacggcccaaactcctacgggaggcagcagtggggaatattgcacaatgggggaaaccctgatgcagcgacgccgcgtgagcgaagaagtatttcggtatgtaaagctctatcagcagggaagataatgacggtacctgactaagaagccccggctaactacgtgccagcagccgcggtaatacgtagggggcaagcgttatccggatttactgggtgtaaagggagcgtagacggcaaggcaagtctgatgtgaaaacccagggcttaaccctgggactgcattggaaactgtctggctcgagtgccggagaggtaagcggaattcctagtgtagcggtgaaatgcgtagatattaggaagaacaccagtggcgaaggcggcttactggacggtaactgacgttgaggctcgaaagcgtggggagcaaacaggattagataccctggtagtccacgccgtaaacgatgaatgctaggtgttggggagcaaagctcttcggtgccgccgcaaacgcattaagcattccacctggggagtacgttcgcaagaatgaaactcaaaggaattgacggggacccgcacaagcggtggagcatgtggtttaattcgaagcaacgcgaagaaccttaccaggtcttgacatcccgatgaccggcccgtaacggggccttctcttcggagcattggagacaggtggtgcatggttgtcgtcagctcgtgtcgtgagatgttgggttaagtcccgcaacgagcgcaacccttatcctcagtagccagcaggtaaagctgggcactctgtggagactgccagggataacctggaggaaggtggggatgacgtcaaatcatcatgccccttatgatctgggctacacacgtgctacaatggcgtaaacaaagggaggcaaagccgcgaggtggagcaaatcccaaaaataacgtctcagttcggactgcagtctgcaactcgactgcacgaagctggaatcgctagtaatcgcgaatcagaatgtcgcggtgaatacgttcccgggtcttgtacacaccgcccgtcacaccatgggagttggtaacgcccgaagtcagtgacccaacctttta

SEQ ID NO: 117 - DNA, 1494 bp, Ruminococcus champanellensis
agagtttgatcctggctcaggacgaacgctggcggcacgcctaacacatgcaagtcgaacggagataaagacttcggtttttatcttagtggcggacgggtgagtaacacgtgagcaacctgcctctgagagagggatagcttctggaaacggatggtaatacctcataacatagcggtaccgcatgatactgctatcaaagatttatcgctcagagatgggctcgcgtctgattagctagatggtgaggtaacggctcaccatggcgacgatcagtagccggactgagaggttgaacggccacattgggactgagacacggcccagactcctacgggaggcagcagtggggaatattgcacaatgggcgcaagcctgatgcagcgatgccgcgtggaggaagaaggttttcggattgtaaactcctgtcttaagggacgataatgacggtaccttaggaggaagctccggctaactacgtgccagcagccgcggtaatacgtagggagcgagcgttgtccggaattactgggtgtaaagggagcgtaggcgggattgcaagtcagatgtgaaaactatgggcttaacccatagactgcatttgaaactgtagttcttgagtgaagtagaggtaagcggaattcctagtgtagcggtgaaatgcgtagatattaggaggaacatcggtggcgaaggcggcttactgggcttttactgacgctgaggctcgaaagcgtggggagcaaacaggattagataccctggtagtccacgctgtaaacgatgattactaggtgtggggggactgaccccttccgtgccgcagttaacacaataagtaatccacctggggagtacggccgcaaggttgaaactcaaaggaattgacgggggcccgcacaagcagtggagtatgtggtttaattcgaagcaacgcgaaaaaccttaccaggtcttgacatcgagtgaatgatctagagatagatcagtccttcgggacacaaagacaggtggtgcatggttgtcgtcagctcgtgtcgtgagatgttgggttaagtcccgcaacgagcgcaacccttacctttagttgctacgcaagagcactctagagggactgccgttgacaaaacggaggaaggtggggatgacgtcaaatcatcatgccccttatgacctgggctacacacgtactacaatggcaatgaacagagggaagcaatacagtgatgtggagcaaatccccaaaaattgtcccagttcagattgtaggctgcaactcgcctacatgaagtcggaattgctagtaatcgcagatcagcatgctgcggtgaatacgttcccgggccttgtacacaccgcccgtcacaccatgggagtcggtaacacccgaagccagtagcctaaccgcaaggagggcgctgtcgaaggtgggattgatgactggggtgaagtcgtaacaaggtagccgtatcggaaggtgcggctggatcacct

SEQ ID NO: 118 - DNA, 1533 bp, Bifidobacterium bifidum
tttttgtggagggttcgattctggctcaggatgaacgctggcggcgtgcttaacacatgcaagtcgaacgggatccatcgggctttgcttggtggtgagagtggcgaacgggtgagtaatgcgtgaccgacctgccccatgctccggaatagctcctggaaacgggtggtaatgccggatgttccacatgatcgcatgtgattgtgggaaagattctatcggcgtgggatggggtcgcgtcctatcagcttgttggtgaggtaacggctcaccaaggcttcgacgggtagccggcctgagagggcgaccggccacattgggactgagatacggcccagactcctacgggaggcagcagtggggaatattgcacaatgggcgcaagcctgatgcagcgacgccgcgtgagggatggaggccttcgggttgtaaacctcttttgtttgggagcaagccttcgggtgagtgtacctttcgaataagcgccggctaactacgtgccagcagccgcggtaatacgtagggcgcaagcgttatccggatttattgggcgtaaagggctcgtaggcggctcgtcgcgtccggtgtgaaagtccatcgcttaacggtggatctgcgccgggtacgggcgggctggagtgcggtaggggagactggaattcccggtgtaacggtggaatgtgtagatatcgggaagaacaccgatggcgaaggcaggtctctgggccgtcactgacgctgaggagcgaaagcgtggggagcgaacaggattagataccctggtagtccacgccgtaaacggtggacgctggatgtggggcacgttccacgtgttccgtgtcggagctaacgcgttaagcgtcccgcctggggagtacggccgcaaggctaaaactcaaagaaattgacgggggcccgcacaagcggcggagcatgcggattaattcgatgcaacgcgaagaaccttacctgggcttgacatgttcccgacgacgccagagatggcgtttcccttcggggcgggttcacaggtggtgcatggtcgtcgtcagctcgtgtcgtgagatgttgggttaagtcccgcaacgagcgcaaccctcgccccgtgttgccagcacgttatggtgggaactcacgggggaccgccggggttaactcggaggaaggtggggatgacgtcagatcatcatgccccttacgtccagggcttcacgcatgctacaatggccggtacagcgggatgcgacatggcgacatggagcggatccctgaaaaccggtctcagttcggatcggagcctgcaacccggctccgtgaaggcggagtcgctagtaatcgcggatcagcaacgccgcggtgaatgcgttcccgggccttgtacacaccgcccgtcaagtcatgaaagtgggcagcacccgaagccggtggcctaaccccttgtgggatggagccgtctaaggtgaggctcgtgattgggactaagtcgtaacaaggtagccgtaccggaaggtgcggctggatcacctcctttct

SEQ ID NO: 119 - DNA, 1552 bp, Megasphaera elsdenii
agagtttgatcctggctcaggacgaacgctggcggcgtgcttaacacatgcaagtcgaacgagaagagatgagaagcttgcttcttatcaattcgagtggcaaacgggtgagtaacgcgtaagcaacctgcccttcagatggggacaacagctggaaacggctgctaataccgaatacgttctttttgtcgcatggcagagggaagaaagggaggctcttcggagctttcgctgaaggaggggcttgcgtctgattagctagttggaggggtaacggcccaccaaggcgacgatcagtagccggtctgagaggatgaacggccacattgggactgagacacggcccagactcctacgggaggcagcagtggggaatcttccgcaatggacgaaagtctgacggagcaacgccgcgtgaacgatgacggccttcgggttgtaaagttctgttatacgggacgaatggcgtagcggtcaatacccgttacgagtgacggtaccgtaagagaaagccacggctaactacgtgccagcagccgcggtaatacgtaggtggcaagcgttgtccggaattattgggcgtaaagggcgcgcaggcggcgtcgtaagtcggtcttaaaagtgcggggcttaaccccgtgaggggaccgaaactgcgatgctagagtatcggagaggaaagcggaattcctagtgtagcggtgaaatgcgtagatattaggaggaacaccagtggcgaaagcggctttctggacgacaactgacgctgaggcgcgaaagccaggggagcaaacgggattagataccccggtagtcctggccgtaaacgatggatactaggtgtaggaggtatcgaccccttctgtgccggagttaacgcaataagtatcccgcctggggagtacggccgcaaggctgaaactcaaaggaattgacgggggcccgcacaagcggtggagtatgtggtttaattcgacgcaacgcgaagaaccttaccaagccttgacattgattgctatggatagagatatccagttcctcttcggaggacaagaaaacaggtggtgcacggctgtcgtcagctcgtgtcgtgagatgttgggttaagtcccgcaacgagcgcaacccctatcttctgttaccagcggttcggccggggactcaggagagactgccgcagacaatgcggaggaaggcggggatgacgtcaagtcatcatgccccttatggcttgggctacacacgtactacaatggctcttaatagagggaagcgaaggagcgatccggagcaaaccccaaaaacagagtcccagttcggattgcaggctgcaactcgcctgcatgaagcaggaatcgctagtaatcgcaggtcagcatactgcggtgaatacgttcccgggccttgtacacaccgcccgtcacaccacgaaagtcattcacacccgaagccggtgaggtaaccttttggagccagccgtcgaaggtgggggcgatgattggggtgaagtcgtaacaaggtagccgtatcggaaggtgcggctggatcacct

SEQ ID NO: 120 - DNA, 1479 bp, Dorea formicigenerans
  misc_feature (123)..(125): n is a, c, g, t or u
  misc_feature (220)..(222): n is a, c, g, t or u
  misc_feature (287)..(287): n is a, c, g, t or u
  misc_feature (349)..(350): n is a, c, g, t or u
  misc_feature (517)..(517): n is a, c, g, t or u
  misc_feature (534)..(535): n is a, c, g, t or u
  misc_feature (725)..(725): n is a, c, g, t or u
  misc_feature (918)..(918): n is a, c, g, t or u
  misc_feature (921)..(921): n is a, c, g, t or u
  misc_feature (955)..(956): n is a, c, g, t or u
  misc_feature (1184)..(1185): n is a, c, g, t or u
ttaaacgagagtttgatcctggctcaggatgaacgctggcggcgtgcttaacacatgcaagtcgagcgaagcacataagtttgattcttcggatgaagacttttgtgactgagcggcggacgnnngagtaacgcgtgggtaacctgcctcatacagggggataacagytagaaatggctgctaataccgcataagaccacagtactgcatggtacagtgnnnaaaactccggtggtatgagatggacccgcgtctgattaggtagttggtgaggtaacggcccaccnagccgacgatcagtagccgacctgagagggtgaccggccacattgggactgagacacggccnngactcctacgggaggcagcagtggggaatattgcacaatgggcgaaagcctgatgcagcgacgccgcgtgaaggatgaagtatttcggtatgtaaacttctatcagcagggaagaaaatgacggtacctgactaagaagccccggctaactacgtgccagcagccgnggtaatacgtagggggnnagcgttatccggatttactgggtgtaaagggagcgtagacggctgtgcaagtctgaagtgaaaggcatgggctcaacctgtggactgctttggaaactgtgcagctagagtgtcggagaggtaagtggaattcctagtgtagcggtgaaatgcgtagatattaggaggaacaccagtggcgaaggcggcntactggacgatgactgacgttgaggctcgaaagcgtggggagcaaacaggattagataccctggtagtccacgccgtaaacgatgactgctaggtgtcgggtagcaaagctattcggtgccgcagctaacgcaataagcagtccacctggggagtacgttcgcaagaatgaaactcaaaggaattgacggggnccngcacaagcggtggagcatgtggtttaattcgaannaacgcgaagaaccttacctgatcttgacatcccgatgaccgcttcgtaatggaagyttttcttcggaacatcggtgacaggtggtgcatggttgtcgtcagctcgtgtcgtgagatgttgggttaagtcccgcaacgagcgcaacccttatcttcagtagccagcatttaggatgggcactctggagagactgccagggataacctggaggaaggtggggatgacgtnnaatcatcatgccccttatgaccagggctacacacgtgctacaatggcgtaaacagagggaggcagagccgcgaggccgagcaaatctcaaaaataacgtctcagttcggattgtagtctgcaactcgactacatgaagctggaatcgctagtaatcgcagatcagaatgctgcggtgaatacgttcccgggtcttgtacacaccgcccgtcacaccatgggagtcagtaacgcccgaagtcagtgacccaaccgaaaggagggagctgccgaaggtgggaccgataactggggt

SEQ ID NO: 121 - DNA, 1390 bp, Eisenbergiella tayi
ggtataacttagtggcggacgggtgagtaacgcgtgggaaacctgccctgtaccgggggataacacttagaaataggtgctaataccgcataagcgcacggaaccgcatggttccgtgtgaaaaactccggtggtacaggatggtcccgcgtctgattagccagttggcagggtaacggcctaccaaagcgacgatcagtagccggcctgagagggtgaacggccacattgggactgagacacggcccaaactcctacgggaggcagcagtggggaatattgcacaatgggggaaaccctgatgcagcgacgccgcgtgagtgaagaagtatttcggtatgtaaagctctatcagcagggaagaaaatgacggtacctgactaagaagccccggctaactacgtgccagcagccgcggtaatacgtagggggcaagcgttatccggatttactgggtgtaaagggagcgtagacggcatggcaagccagatgtgaaaacccagggctcaaccttgggattgcatttggaactgccaggctggagtgcaggagaggtaagcggaattcctagtgtagcggtgaaatgcgtagatattaggaggaacaccagtggcgaaggcggcttactggactgtaactgacgttgaggctcgaaagcgtggggagcaaacaggattagataccctggtagtccacgcggtaaacgatgattgctaggtgtaggtgggtatggacccatcggtgccgcagctaacgcaataagcaatccacctggggagtacgttcgcaagaatgaaactcaaaggaattgacggggacccgcacaagcggtggagcatgtggtttaattcgaagcaacgcgaagaaccttaccaagtcttgacatcccaatgacgcacctgtaaagaggtgttcccttcggggcattggagacaggtggtgcatggttgtcgtcagctcgtgtcgtgagatgttgggttaagtcccgcaacgagcgcaacccttattcttagtagccagcaggtaaagctgggcactctaaggagactgccggggataacccggaggaaggcggggatgacgtcaaatcatcatgccccttatgatttgggctacacacgtgctacaatggcgtaaacaaagggaagcgagacagtgatgtggagcaaatcycagaaataacgtctcagttcggattgtagtctgcaactcgactacatgaagctggaatcgctagtaatcgcgaatcagcatgtcgcggtgaatacgttcccgggtcttgtacacaccgcccgtcacaccatgggagttggaaatgcccgaagtctgtgacctaaccgaaagggaggagcagccgaaggcaggtctgataactggggtgaagtcgtaa

SEQ ID NO: 122 - DNA, 1478 bp, Clostridium symbiosum
  misc_feature (349)..(350): n is a, c, g, t or u
  misc_feature (534)..(535): n is a, c, g, t or u
  misc_feature (606)..(606): n is a, c, g, t or u
  misc_feature (618)..(619): n is a, c, g, t or u
  misc_feature (709)..(709): n is a, c, g, t or u
  misc_feature (921)..(921): n is a, c, g, t or u
  misc_feature (955)..(956): n is a, c, g, t or u
  misc_feature (1012)..(1013): n is a, c, g, t or u
  misc_feature (1015)..(1015): n is a, c, g, t or u
  misc_feature (1081)..(1081): n is a, c, g, t or u
  misc_feature (1185)..(1185): n is a, c, g, t or u
  misc_feature (1240)..(1240): n is a, c, g, t or u
  misc_feature (1391)..(1392): n is a, c, g, t or u
  misc_feature (1470)..(1470): n is a, c, g, t or u
  misc_feature (1474)..(1475): n is a, c, g, t or u
aaacatgagagtttgatcctggctcaggatgaacgctggcggcgtgcctaacacatgcaagtcgaacgaagcgatttaacggaagttttcggatggaagttgaattgactgagtggcggacgggtgagtaacgcgtgggtaacctgccttgtactgggggacaacagttagaaatgactgctaataccgcataagcgcacagtattgcatgatacagtgtgaaaaactccggtggtacaagatggacccgcgtctgattagctagttggtaaggtaacggcttaccaaggcgacgatcagtagccgacctgagagggtgaccggccacattgggactgagacacggccnnaactcctacgggaggcagcagtggggaatattgcacaatgggcgaaagcctgatgcagcgacgccgcgtgagtgaagaagtatttcggtatgtaaagctctatcagcagggaagaaaatgacggtacctgactaagaagccccggctaactacgtgccagcagccgcggtaatacgtagggggnnagcgttatccggatttactgggtgtaaagggagcgtagacggtaaagcaagtctgaagtgaaagcccgcgnctcaactgcggnnctgctttggaaactgtttaactggagtgtcggagaggtaagtggaattcctagtgtagcggtgaaatgcgtagatattaggaggaacacnagtggcgaaggcgacttactggacgataactgacgttgaggctcgaaagcgtggggagcaaacaggattagataccctggtagtccacgccgtaaacgatgaatactaggtgttggggagcaaagctcttcggtgccgtcgcaaacgcagtaagtattccacctggggagtacgttcgcaagaatgaaactcaaaggaattgacggggaccngcacaagcggtggagcatgtggtttaattcgaannaacgcgaagaaccttaccaggtcttgacatcgactcgacgggggagtaacgtcccnntnccttcggggcggagaagacaggtggtgcatggttgtcgtcagctcgtgtcgtgagatgttgggttnagtcccgcaacgagcgcaacccttattctaagtagccagcggttcggccgggaactcttgggagactgccagggataacctggaggaaggtggggatgacgtcnaatcatcatgccccttatgatctgggctacacacgtgctacaatggcgtaaacanagagaagcaagaccgcgaggtggagcaaatctcaaaaataacgtctcagttcggactgcaggctgcaactcgcctgcacgaagctggaatcgctagtaatcgcgaatcagaatgtcgcggtgaatacgttcccgggtcttgtacacaccgnncgtcacaccatgggagtcagtaacgcccgaagtcagtgacccaaccgcaaggagggagctgccgaaggcgggaccganaacnnggg

SEQ ID NO: 123 - DNA, 1488 bp, Erysipelatoclostridium ramosum
agagtttgatcctggctcaggatgaacgctggcggcgtgcctaatacatgcaagtcgaacgcgagcacttgtgctcgagtggcgaacgggtgagtaatacataagtaacctgccctagacagggggataactattggaaacgatagctaagaccgcataggtacggacactgcatggtgaccgtattaaaagtgcctcaaagcactggtagaggatggacttatggcgcattagctggttggcggggtaacggcccaccaaggcgacgatgcgtagccgacctgagagggtgaccggccacactgggactgagacacggcccagactcctacgggaggcagcagtagggaattttcggcaatgggggaaaccctgaccgagcaacgccgcgtgaaggaagaaggttttcggattgtaaacttctgttataaaggaagaacggcggctacaggaaatggtagccgagtgacggtactttattagaaagccacggctaactacgtgccagcagccgcggtaatacgtaggtggcaagcgttatccggaattattgggcgtaaagagggagcaggcggcagcaagggtctgtggtgaaagcctgaagcttaacttcagtaagccatagaaaccaggcagctagagtgcaggagaggatcgtggaattccatgtgtagcggtgaaatgcgtagatatatggaggaacaccagtggcgaaggcgacgatctggcctgcaactgacgctcagtcccgaaagcgtggggagcaaataggattagataccctagtagtccacgccgtaaacgatgagtactaagtgttggatgtcaaagttcagtgctgcagttaacgcaataagtactccgcctgagtagtacgttcgcaagaatgaaactcaaaggaattgacgggggcccgcacaagcggtggagcatgtggtttaattcgaagcaacgcgaagaaccttaccaggtcttgacatactcataaaggctccagagatggagagatagctatatgagatacaggtggtgcatggttgtcgtcagctcgtgtcgtgagatgttgggttaagtcccgcaacgagcgcaacccttatcgttagttaccatcattaagttggggactctagcgagactgccagtgacaagctggaggaaggcggggatgacgtcaaatcatcatgccccttatgacctgggctacacacgtgctacaatggatggtgcagagggaagcgaagccgcgaggtgaagcaaaacccataaaaccattctcagttcggattgtagtctgcaactcgactacatgaagttggaatcgctagtaatcgcgaatcagcatgtcgcggtgaatacgttctcgggccttgtacacaccgcccgtcacaccacgagagttgataacacccgaagccggtggcctaaccgcaaggaaggagctgtctaaggtgggattgatgattggggtgaagtcgtaacaaggtaacc

SEQ ID NO: 124 - DNA, 1528 bp, Artificial Sequence
  Synthetic Polynucleotide
atgagagtttgatcctggctcaggatgaacgctggcggcgtgcctaacacatgcaagtcgaacgaagcaattaaaggaagttttcggatggaatttgattgactgagtggcggacgggtgagtaacgcgtggataacctgcctcacactgggggataacagttagaaatgactgctaataccgcataagcgcacagtaccgcatggtacggtgtgaaaaactccggtggtgtgagatggatccgcgtctgattagccagttggcggggtaacggcccaccaaagcgacgatcagtagccgacctgagagggtgaccggccacattgggactgagacacggcccaaactcctacgggaggcagcagtggggaatattgcacaatgggcgaaagcctgatgcagcgacgccgcgtgagtgaagaagtatttcggtatgtaaagctctatcagcagggaagaaaatgacggtacctgactaagaagccccggctaactacgtgccagcagccgcggtaatacgtagggggcaagcgttatccggattcactgggtgtaaagggagcgtagacggcgaagcaagtctgaagtgaaaacccagggctcaaccctgggactgctttggaaactgttttgctagagtgtcggagaggtaagtggaattcctagtgtagcggtgaaatgcgtagatattaggaggaacaccagtggcgaaggcggcttactggacgataactgacgttgaggctcgaaagcgtggggagcaaacaggattagataccctggtagtccacgccgtaaacgatgaatgctaggtgttggggggcaaagcccttcggtgccgtcgcaaacgcagtaagcattccacctggggagtacgttcgcaagaatgaaactcaaaggaattgacggggacccgcacaagcggtggagcatgtggtttaattcgaagcaacgcgaagaaccttaccaagtcttgacatcctcttgaccggcgtgtaacggcgccttcccttcggggcaagagagacaggtggtgcatggttgtcgtcagctcgtgtcgtgagatgttgggttaagtcccgcaacgagcgcaacccttatccttagtagccagcaggtagagctgggcactctagggagactgccagggataacctggaggaaggtggggatgacgtcaaatcatcatgccccttatgatttgggctacacacgtgctacaatggcgtaaacaaagggaagcaagacagtgatgtggagcaaatcccaaaaataacgtcccagttcggactgtagtctgcaacccgactacacgaagctggaatcgctagtaatcgcgaatcagaatgtcgcggtgaatacgttcccgggtcttgtacacaccgcccgtcacaccatgggagtcagcaacgcccgaagtcagtgacccaactcgcaagagagggagctgccgaaggcggggcaggtaactggggtgaagtcgtaacaaggtagccgtatcggaaggtgcggctggatcacctccttt

SEQ ID NO: 125 - DNA, 1530 bp, Artificial Sequence
  Synthetic Polynucleotide
atgagagtttgatcctggctcaggatgaacgctggcggcgtgcctaacacatgcaagtcgaacgaagcaattaaaatgaagttttcggatggatttttgattgactgagtggcggacgggtgagtaacgcgtggataacctgcctcacactgggggataacagttagaaatgactgctaataccgcataagcgcacagtaccgcatggtacggtgtgaaaaactccggtggtgtgggatggatccgcgtctgattagccagttggcggggtaacggcccaccaaagcgacgatcagtagccgacctgagagggtgaccggccacattgggactgagacacggcccaaactcctacgggaggcagcagtggggaatattgcacaatgggcgaaagcctgatgcagcgacgccgcgtgagtgaagaagtatttcggtatgtaaagctctatcagcagggaagaaaatgacggtacctgactaagaagccccggctaactacgtgccagcagccgcggtaatacgtagggggcaagcgttatccggatttactgggtgtaaagggagcgtagacggcgaagcaagtctgaagtgaaaacccagggctcaaccctgggactgctttggaaactgttttgctagagtgtcggagaggtaagtggaattcctagtgtagcggtgaaatgcgtagatattaggaggaacaccagtggcgaaggcggcttactggacgataactgacgttgaggctcgaaagcgtggggagcaaacaggattagataccctggtagtccacgccgtaaacgatgaatgctaggtgttggggggcaaagcccttcggtgccgtcgcaaacgcagtaagcattccacctggggagtacgttcgcaagaatgaaactcaaaggaattgacggggacccgcacaagcggtggagcatgtggtttaattcgaagcaacgcgaagaaccttaccaagtcttgacatcctcttgaccggcgtgtaacggcgccttcccttcggggcaagagagacaggtggtgcatggttgtcgtcagctcgtgtcgtgagatgttgggttaagtcccgcaacgagcgcaacccttatccttagtagccagcaggtaaagctgggcactctagggagactgccagggataacctggaggaaggtggggatgacgtcaaatcatcatgccccttatgatttgggctacacacgtgctacaatggcgtaaacaaagggaagcaagacagtgatgtggagcaaatcccaaaaataacgtcccagttcggactgtagtctgcaacccgactacacgaagctggaatcgctagtaatcgcgaatcagaatgtcgcggtgaatacgttcccgggtcttgtacacaccgcccgtcacaccatgggagtcagcaacgcccgaagtcagtgacccaactcgcaagagagggagctgccgaaggcggggcaggtaactggggtgaagtcgtaacaaggtagccgtatcggaaggtgcggctggatcacctccttt

SEQ ID NO: 126 - DNA, 1528 bp, Artificial Sequence
  Synthetic Polynucleotide
atgagagtttgatcctggctcaggatgaacgctggcggcgtgcctaacacatgcaagtcgaacgaagcaattaaaatgaagttttcggatggatttttgattgactgagtggcggacgggtgagtaacgcgtggataacctgcctcacactgggggataacagttagaaatgactgctaataccgcataagcgcacagtaccgcatggtacggtgtgaaaaactccggtggtgtgagatggatccgcgtctgattagccagttggcggggtaacggcccaccaaagcgacgatcagtagccgacctgagagggtgaccggccacattgggactgagacacggcccaaactcctacgggaggcagcagtggggaatattgcacaatgggcgaaagcctgatgcagcgacgccgcgtgagtgaagaagtatttcggtatgtaaagctctatcagcagggaagaaatgacggtacctgactaagaagccccggctaactacgtgccagcagccgcggtaatacgtagggggcaagcgttatccggatttactgggtgtaaagggagcgtagacggcgaagcaagtctgaagtgaaaacccagggctcaaccctgggactgctttggaaactgttttgctagagtgtcggagaggtaagtggaattcctagtgtagcggtgaaatgcgtagatattaggaggaacaccagtggcgaaggcggcttactggacgataactgacgttgaggctcgaaagcgtggggagcaaacaggattagataccctggtagtccacgccgtaaacgatgaatgctaggtgttgggggcaaagcccttcggtgccgtcgcaaacgcagtaagcattccacctggggagtacgttcgcaagaatgaaactcaaaggaattgacggggacccgcacaagcggtggagcatgtggtttaattcgaagcaacgcgaagaaccttaccaagtcttgacatcctcttgaccggcgtgtaacggcgccttcccttcggggcaagagagacaggtggtgcatggttgtcgtcagctcgtgtcgtgagatgttgggttaagtcccgcaacgagcgcaacccttatccttagtagccagcaggtaaagctgggcactctagggagactgccagggataacctggaggaaggtggggatgacgtcaaatcatcatgccccttatgatttgggctacacacgtgctacaatggcgtaaacaaagggaagcaagacagtgatgtggagcaaatcccaaaaataacgtcccagttcggactgtagtctgcaacccgactacacgaagctggaatcgctagtaatcgcgaatcagaatgtcgcggtgaatacgttcccgggtcttgtacacaccgcccgtcacaccatgggagtcagcaacgcccgaagtcagtgacccaactcgcaagagagggagctgccgaaggcggggcaggtaactggggtgaagtcgtaacaaggtagccgtatcggaaggtgcggctggatcacctccttt

SEQ ID NO: 127 - DNA, 1528 bp, Artificial Sequence
  Synthetic Polynucleotide
atgagagtttgatcctggctcaggatgaacgctggcggcgtgcctaacacatgcaagtcgaacgaagcaattaaaatgaagttttcggatggatttttgattgactgagtggcggacgggtgagtaacgcgtggataacctgcctcacactgggggataacagttagaaatgactgctaataccgcataagcgcacagtaccgcatggtacggtgtgaaaaactccggtggtgtgagatggatccgcgtctgattagccagttggcggggtaacggcccaccaaagcgacgatcagtagccgacctgagagggtgaccggccacattgggactgagacacggcccaaactcctacgggaggcagcagtggggaatattgcacaatgggcgaaagcctgatgcagcgacgccgcgtgagtgaagaagtatttcggtatgtaaagctctatcagcagggaagaaaatgacggtacctgactaagaagccccggctaactacgtgccagcagccgcggtaatacgtagggggcaagcgttatccggatttactgggtgtaaagggagcgtagacggcgaagcaagtctgaagtgaaaacccagggctcaaccctgggactgctttggaaactgttttgctagagtgtcggagaggtaagtggaattcctagtgtagcggtgaaatgcgtagatattaggaggaacaccagtggcgaaggcggcttactggacgataactgacgttgaggctcgaaagcgtggggagcaaacaggattagataccctggtagtccacgccgtaaacgatgaatgctaggtgttgggggcaaagcccttcggtgccgtcgcaaacgcagtaagcattccacctggggagtacgttcgcaagaatgaaactcaaaggaattgacggggacccgcacaagcggtggagcatgtggtttaattcgaagcaacgcgaagaaccttaccaagtcttgacatcctcttgaccggcgtgtaacggcgccttcccttcggggcaggagagacaggtggtgcatggttgtcgtcagctcgtgtcgtgagatgttgggttaagtcccgcaacgagcgcaacccttatccttagtagccagcaggtagagctgggcactctagggagactgccagggataacctggaggaaggtggggatgacgtcaaatcatcatgccccttatgatttgggctacacacgtgctacaatggcgtaaacaaagggaagcaagacagtgatgtggagcaaatcccaaaataacgtcccagttcggactgtagtctgcaacccgactacacgaagctggaatcgctagtaatcgcgaatcagaatgtcgcggtgaatacgttcccgggtcttgtacacaccgcccgtcacaccatgggagtcagcaacgcccgaagtcagtgacccaactcgcaagagagggagctgccgaaggcggggcaggtaactggggtgaagtcgtaacaaggtagccgtatcggaaggtgcggctggatcacctccttt

SEQ ID NO: 128 - DNA, 1528 bp, Artificial Sequence
  Synthetic Polynucleotide
atgagagtttgatcctggctcaggatgaacgctggcggcgtgcctaacacatgcaagtcgaacgaagcaattaaaatgaagttttcggatggattttaattgactgagtggcggacgggtgagtaacgcgtggataacctgcctcacactgggggataacagttagaaatgactgctaataccgcataagcgcacagtaccgcatggtacggtgtgaaaaactccggtggtgtgagatggatccgcgtctgattagccagttggcggggtaacggcccaccaaagcgacgatcagtagccgacctgagagggtgaccggccacattgggactgagacacggcccaaactcctacgggaggcagcagtggggaatattgcacaatgggcgaaagcctgatgcagcgacgccgcgtgagtgaagaagtatttcggtatgtaaagctctatcagcagggaagaaaatgacggtacctgactaagaagccccggctaactacgtgccagcagccgcggtaatacgtagggggcaagcgttatccggatttactgggtgtaaagggagcgtagacggcgaagcaagtctgaagtgaaaacccagggctcaaccctgggactgctttggaaactgttttgctagagtgtcggagaggtaagtggaattcctagtgtagcggtgaaatgcgtagatattaggaggaacaccagtggcgaaggcggcttactggacgataactgacgttgaggctcgaaagcgtggggagcaaacaggattagataccctggtagtccacgccgtaaacgatgaatgctaggtgttggggggcaaagcccttcggtgccgtcgcaaacgcagtaagcattccacctggggagtacgttcgcaagaatgaaactcaaaggaattgacggggacccgcacaagcggtggagcatgtggtttaattcgaagcaacgcgaagaaccttaccaagtcttgacatcctcttgaccggcgtgtaacggcgccttcccttcggggcaagagagacaggtggtgcatggttgtcgtcagctcgtgtcgtgagatgttgggttaagtcccgcaacgagcgcaacccttatccttagtagccagcaggtaaagctgggcactctagggagactgccagggataacctggaggaaggtggggatgacgtcaaatcatcatgccccttatgatttgggctacacacgtgctacaatggcgtaaacaaagggaagcaagacagtgatgtggagcaaatcccaaaataacgtcccagttcggactgtagtctgcaacccgactacacgaagctggaatcgctagtaatcgcgaatcagaatgtcgcggtgaatacgttcccgggtcttgtacacaccgcccgtcacaccatgggagtcagcaacgcccgaagtcagtgacccaactcgcaagagagggagctgccgaaggcggggcaggtaactggggtgaagtcgtaacaaggtagccgtatcggaaggtgcggctggatcacctccttt

SEQ ID NO: 129 - DNA, 1522 bp, Artificial Sequence
  Synthetic Polynucleotide
tcaaagagtttgatcctggctcaggacgaacgctggcggcgcgcctaacacatgcaagtcgaacggagcttacgttttgaagttttcggatggatgaatgtaagcttagtggcggacgggtgagtaacacgtgagcaacctgcctttcagagggggataacagccggaaacggctgctaataccgcatgatgttgcgggggcacatgcccctgcaaccaaaggagcaatccgctgaaagatgggctcgcgtccgattagccagttggcggggtaacggcccaccaaagcgacgatcggtagccggactgagaggttgaacggccacattgggactgagacacggcccagactcctacgggaggcagcagtgggggatattgcacaatgggcgaaagcctgatgcagcgacgccgcgtgagggaagacggtcttcggattgtaaacctctgtctttggggaagaaaatgacggtacccaaagaggaagctccggctaactacgtgccagcagccgcggtaatacgtagggagcaagcgttgtccggaattactgggtgtaaagggagcgtaggcgggatggcaagtagaatgttaaatccatcggctcaaccggtggctgcgttctaaactgccgttcttgagtgaagtagaggcaggcggaattcctagtgtagcggtgaaatgcgtagatattaggaggaacaccagtggcgaaggcggcctgctgggctttaactgacgctgaggctcgaaagcgtggggagcaaacaggattagataccctggtagtccacgccgtaaacgatgattactaggtgtggggggactgaccccttccgtgccgcagttaacacaataagtaatccacctggggagtacggccgcaaggttgaaactcaaaggaattgacgggggcccgcacaagcagtggagtatgtggtttaattcgaagcaacgcgaagaaccttaccaggtcttgacatcggatgcatagcctagagataggtgaagcccttcggggcatccagacaggtggtgcatggttgtcgtcagctcgtgtcgtgagatgttgggttaagtcccgcaacgagcgcaacccttattattagttgctacgcaagagcactctaatgagactgccgttgacaaaacggaggaaggtggggatgacgtcaaatcatcatgccccttatgacctgggctacacacgtactacaatggcactaaaacagagggcggcgacaccgcgaggtgaagcgaatcccgaaaaagtgtctcagttcagattgcaggctgcaacccgcctgcatgaagtcggaattgctagtaatcgcggatcagcatgccgcggtgaatacgttcccgggccttgtacacaccgcccgtcacaccatgggagtcggtaacacccgaagccagtagcctaaccgcaaggggggcgctgtcgaaggtgggattgatgactggggtgaagtcgtaacaaggtagccgtatcggaaggtgcggctggatcacctccttt

SEQ ID NO: 130 - DNA, 1521 bp, Artificial Sequence
  Synthetic Polynucleotide
tcaaagagtttgatcctggctcaggacgaacgctggcggcgcgcctaacacatgcaagtcgaacggagcttacgttttgaagttttcggatggacgaatgtaagcttagtggcggacgggtgagtaacacgtgagcaacctgcctttcagaggggataacagccggaaacggctgctaataccgcatgatgttgcgggggcacatgcccctgcaaccaaaggagcaatccgctgaaagatgggctcgcgtccgattagccagttggcggggtaacggcccaccaaagcgacgatcggtagccggactgagaggttgaacggccacattgggactgagacacggcccagactcctacgggaggcagcagtgggggatattgcacaatgggcgaaagcctgatgcagcgacgccgcgtgagggaagacggtcttcggattgtaaacctctgtctttggggaagaaaatgacggtacccaaagaggaagctccggctaactacgtgccagcagccgcggtaatacgtagggagcaagcgttgtccggaattactgggtgtaaagggagcgtaggcgggatggcaagtagaatgttaaatccatcggctcaaccggtggctgcgttctaaactgccgttcttgagtgaagtagaggcaggcggaattcctagtgtagcggtgaaatgcgtagatattaggaggaacaccagtggcgaaggcggcctgctgggctttaactgacgctgaggctcgaaagcgtggggagcaaacaggattagataccctggtagtccacgccgtaaacgatgattactaggtgtggggggactgaccccttccgtgccgcagttaacacaataagtaatccacctggggagtacggccgcaaggttgaaactcaaaggaattgacgggggcccgcacaagcagtggagtatgtggtttaattcgaagcaacgcgaagaaccttaccaggtcttgacatcggatgcatagcctagagataggtgaagcccttcggggcatccagacaggtggtgcatggttgtcgtcagctcgtgtcgtgagatgttgggttaagtcccgcaacgagcgcaacccttattattagttgctacgcaagagcactctaatgagactgccgttgacaaaacggaggaaggtggggatgacgtcaaatcatcatgccccttatgacctgggctacacacgtactacaatggcactaaaacagagggcggcgacaccgcgaggtgaagcgaatcccgaaaaagtgtctcagttcagattgcaggctgcaacccgcctgcatgaagtcggaattgctagtaatcgcggatcagcatgccgcggtgaatacgttcccgggccttgtacacaccgcccgtcacaccatgggagtcggtaacacccgaagccagtagcctaaccgcaaggggggcgctgtcgaaggtgggattgatgactggggtgaagtcgtaacaaggtagccgtatcggaaggtgcggctggatcacctccttt

SEQ ID NO: 131 - DNA, 1522 bp, Artificial Sequence; identical to SEQ ID NO: 129
  Synthetic Polynucleotide

SEQ ID NO: 132 - DNA, 1529 bp, Artificial Sequence
  Synthetic Polynucleotide
tacgagagtttgatcctggctcaggatgaacgctggcggcgtgcctaacacatgcaagtcgagcgaagcgctgttttcagaatcttcggaggaagaggacagtgactgagcggcggacgggtgagtaacgcgtgggcaacctgcctcatacagggggataacagttagaaatgactgctaataccgcataagcgcacaggaccgcatggtgtagtgtgaaaaactccggtggtatgagatggacccgcgtctgattaggtagttggtggggtaaaggcctaccaagccgacgatcagtagccgacctgagagggtgaccggccacattgggactgagacacggcccaaactcctacgggaggcagcagtggggaatattgcacaatgggggaaaccctgatgcagcgacgccgcgtgaaggaagaagtatttcggtatgtaaacttctatcagcagggaagaaaatgacggtacctgagtaagaagcaccggctaaatacgtgccagcagccgcggtaatacgtatggtgcaagcgttatccggatttactgggtgtaaagggagcgtagacggataggcaagtctggagtgaaaacccagggctcaaccctgggactgctttggaaactgcagatctggagtgccggagaggtaagcggaattcctagtgtagcggtgaaatgcgtagatattaggaggaacaccagtggcgaaggcggcttactggacggtgactgacgttgaggctcgaaagcgtggggagcaaacaggattagataccctggtagtccacgccgtaaacgatgactactaggtgtcggtgtgcaaagcacatcggtgccgcagcaaacgcaataagtagtccacctggggagtacgttcgcaagaatgaaactcaaaggaattgacggggacccgcacaagcggtggagcatgtggtttaattcgaagcaacgcgaagaaccttacctggtcttgacatccggatgacgggcgagtaatgtcgccgtcccttcggggcgtccgagacaggtggtgcatggttgtcgtcagctcgtgtcgtgagatgttgggttaagtcccgcaacgagcgcaacccttatcttcagtagccagcatataaggtgggcactctggagagactgccagggagaacctggaggaaggtggggatgacgtcaaatcatcatgccccttatggccagggctacacacgtgctacaatggcgtaaacaaagggaagcgagagggtgacctggagcgaatcccaaaaataacgtctcagttcggattgtagtctgcaactcgactacatgaagctggaatcgctagtaatcgcggatcagcatgccgcggtgaatacgttcccgggtcttgtacacaccgcccgtcacaccatgggagtcagtaacgcccgaagccagtgacccaaccttagaggagggagctgtcgaaggcgggacggataactggggtgaagtcgtaacaaggtagccgtatcggaaggtgcggctggatcacctccttt

SEQ ID NO: 133 - DNA, 1529 bp, Artificial Sequence
  Synthetic Polynucleotide
tacgagagtttgatcctggctcaggatgaacgctggcggcgtgcctaacacatgcaagtcgagcgaagcgctgttttcagaatcttcggaggaagaggacagtgactgagcggcggacgggtgagtaacgcgtgggcaacctgcctcatacagggggataacagttagaaatgactgctaataccgcataagcgcacaggaccgcatggtgtagtgtgaaaaactccggtggtatgagatggacccgcgtctgattaggtagttggtggggtaaaggcctaccaagccgacgatcagtagccgacctgagagggtgaccggccacattgggactgagacacggcccaaactcctacgggaggcagcagtggggaatattgcacaatgggggaaaccctgatgcagcgacgccgcgtgaaggaagaagtatttcggtatgtaaacttctatcagcagggaagaagatgacggtacctgagtaagaagcaccggctaaatacgtgccagcagccgcggtaatacgtatggtgcaagcgttatccggatttactgggtgtaaagggagcgtagacggataggcaagtctggagtgaaaacccagggctcaaccctgggactgctttggaaactgcagatctggagtgccggagaggtaagcggaattcctagtgtagcggtgaaatgcgtagatattaggaggaacaccagtggcgaaggcggcttactggacggtgactgacgttgaggctcgaaagcgtggggagcaaacaggattagataccctggtagtccacgccgtaaacgatgactactaggtgtcggtgtgcaaagcacatcggtgccgcagcaaacgcaataagtagtccacctggggagtacgttcgcaagaatgaaactcaaaggaattgacggggacccgcacaagcggtggagcatgtggtttaattcgaagcaacgcgaagaaccttacctggtcttgacatccggatgacgggcgagtaatgtcgccgtcccttcggggcatccgagacaggtggtgcatggttgtcgtcagctcgtgtcgtgagatgttgggttaagtcccgcaacgagcgcaacccttatcttcagtagccagcatataaggtgggcactctggagagactgccagggagaacctggaggaaggtggggatgacgtcaaatcatcatgccccttatggccagggctacacacgtgctacaatggcgtaaacaaagggaagcgagagggtgacctgaagcgaatcccaaaaataacgtctcagttcggattgtagtctgcaactcgactacatgaagctggaatcgctagtaatcgcggatcagcatgccgcggtgaatacgttcccgggtcttgtacacaccgcccgtcacaccatgggagtcagtaacgcccgaagccagtgacccaaccttagaggagggagctgtcgaaggcgggacggataactggggtgaagtcgtaacaaggtagccgtatcggaaggtgcggctggatcacctccttt

SEQ ID NO: 134 - DNA, 1529 bp, Artificial Sequence; identical to SEQ ID NO: 15
  Synthetic Polynucleotide

SEQ ID NO: 135 - DNA, 1529 bp, Artificial Sequence; identical to SEQ ID NO: 133
  Synthetic Polynucleotide

SEQ ID NO: 136 - DNA, 1529 bp, Artificial Sequence; identical to SEQ ID NO: 15
  Synthetic Polynucleotide

SEQ ID NO: 137 - DNA, 1527 bp, Artificial Sequence
  Synthetic Polynucleotide
atgagagtttgatcctagctcaggatgaacgctggcggcgtgcctaacacatgcaagtcgaacgaagcaatttaacggaagttttcggatggaagttgaattgactgagtggcggacgggtgagtaacgcgtgggtaacctgccttgtactgggggacaacagttagaaatgactgctaataccgcataagcgcacagtatcgcatgatacagtgtgaaaaactccggtggtacaagatggacccgcgtctgattagctagttggtaaggtaacggcttaccaaggcgacgatcagtagccgacctgagagggtgaccggccacattgggactgagacacggcccaaactcctacgggaggcagcagtggggaatattgcacaatgggcgaaagcctgatgcagcgacgccgcgtgagtgaagaagtatttcggtatgtaaagctctatcagcagggaagaaaatgacggtacctgactaagaagccccggctaactacgtgccagcagccgcggtaatacgtagggggcaagcgttatccggatttactgggtgtaaagggagcgtagacggtaaagcaagtctgaagtgaaagcccgcggctcaactgcgggactgctttggaaactgtttaactggagtgtcggagaggtaagtggaattcctagtgtagcggtgaaatgcgtagatattaggaggaacaccagtggcgaaggcgacttactggacgataactgacgttgaggctcgaaagcgtggggagcaaacaggattagataccctggtagtccacgccgtaaacgatgaatactaggtgttggggagcaaagctcttcggtgccgtcgcaaacgcagtaagtattccacctggggagtacgttcgcaagaatgaaactcaaaggaattgacggggacccgcacaagcggtggagcatgtggtttaattcgaagcaacgcgaagaaccttaccaggtcttgacatcgatccgacgggggagtaacgtccccttcccttcggggcggagaagacaggtggtgcatggttgtcgtcagctcgtgtcgtgagatgttgggttaagtcccgcaacgagcgcaacccttattctaagtagccagcggttcggccgggaactcttgggagactgccagggataacctggaggaaggtggggatgacgtcaaatcatcatgccccttatgatctgggctacacacgtgctacaatggcgtaaacaaagagaagcaagaccgcgaggtggagcaaatctcaaaaataacgtctcagttcggactgcaggctgcaactcgcctgcacgaagctggaatcgctagtaatcgcgaatcagaatgtcgcggtgaatacgttcccgggtcttgtacacaccgcccgtcacaccatgggagtcagtaacgcccgaagtcagtgacccaaccgcaaggagggagctgccgaaggcgggaccgataactggggtgaagtcgtaacaaggtagccgtatcggaaggtgcggctggatcacctccttt

SEQ ID NO: 138 - DNA, 1527 bp, Artificial Sequence
  Synthetic Polynucleotide
atgagagtttgatcctggctcaggatgaacgctggcggcgtgcctaacacatgcaagtcgaacgaagcgatttaacggaaattttcggatggaagttgaattgactgagtggcggacgggtgagtaacgcgtgggtaacctgccttgtactgggggacaacagttagaaatgactgctaataccgcataagcgcacagtatcgcatgatacagtgtgaaaaactccggtggtacaagatggacccgcgtctgattagctagttggtaaggtaacggcttaccaaggcgacgatcagtagccgacctgagagggtgaccggccacattgggactgagacacggcccaaactcctacgggaggcagcagtggggaatattgcacaatgggcgaaagcctgatgcagcgacgccgcgtgagtgaagaagtatttcggtatgtaaagctctatcagcagggaagaaaatgacggtacctgactaagaagccccggctaactacgtgccagcagccgcggtaatacgtagggggcaagcgttatccggatttactgggtgtaaagggagcgtagacggtaaagcaagtctgaagtgaaagcccgcggctcaactgcgggactgctttggaaactgtttaactggagtgtcggagaggtaagtggaattcctagtgtagcggtgaaatgcgtagatattaggaggaacaccagtggcgaaggcgacttactggacgataactgacgttgaggctcgaaagcgtggggagcaaacaggattagataccctggtagtccacgccgtaaacgatgaatactaggtgttggggagcaaagctcttcggtgccgtcgcaaacgcagtaagtattccacctggggagtacgttcgcaagaatgaaactcaaaggaattgacggggacccgcacaagcggtggagcatgtggtttaattcgaagcaacgcgaagaaccttaccaggtcttgacatcgatccgacgggggagtaacgtccccttcccttcggggcggagaagacaggtggtgcatggttgtcgtcagctcgtgtcgtgagatgttgggttaagtcccgcaacgagcgcaacccttattctaagtagccagcggttcggccgggaactcttgggagactgccagggataacctggaggaaggtggggatgacgtcaaatcatcatgccccttatgatctgggctacacacgtgctacaatggcgtaaacaaagagaagcaagaccgcgaggtggagcaaatctcaaaaataacgtctcagttcggactgcaggctgcaactcgcctgcacgaagctggaatcgctagtaatcgcgaatcagaatgtcgcggtgaatacgttcccgggtcttgtacacaccgcccgtcacaccatgggagtcagtaacgcccgaagtcagtgacccaaccgcaaggagggagctgccgaaggcgggaccgataactggggtgaagtcgtaacaaggtagccgtatcggaaggtgcggctggatcacctccttt

SEQ ID NO: 139 - DNA, 1527 bp, Artificial Sequence; identical to SEQ ID NO: 16
  Synthetic Polynucleotide

SEQ ID NO: 140 - DNA, 1527 bp, Artificial Sequence
  Synthetic Polynucleotide
atgagagtttgatcctggctcaggatgaacgctggcggcgtgcctaacacatgcaagtcgaacgaagcgatttaacggaagttttcggatggaagttggattgactgagtggcggacgggtgagtaacgcgtgggtaacctgccttgtactgggggacaacagttagaaatgactgctaataccgcataagcgcacagtatcgcatgatacagtgtgaaaaactccggtggtacaagatggacccgcgtctgattagctagttggtaaggtaacggcttaccaaggcgacgatcagtagccgacctgagagggtgaccggccacattgggactgagacacggcccaaactcctacgggaggcagcagtggggaatattgcacaatgggcgaaagcctgatgcagcgacgccgcgtgagtgaagaagtatttcggtatgtaaagctctatcagcagggaagaaaatgacggtacctgactaagaagccccggctaactacgtgccagcagccgcggtaatacgtagggggcaagcgttatccggatttactgggtgtaaagggagcgtagacggtaaagcaagtctgaagtgaaagcccgcggctcaactgcgggactgctttggaaactgtttaactggagtgtcggagaggtaagtggaattcctagtgtagcggtgaaatgcgtagatattaggaggaacaccagtggcgaaggcgacttactggacgataactgacgttgaggctcgaaagcgtggggagcaaacaggattagataccctggtagtccacgccgtaaacgatgaatactaggtgttggggagcaaagctcttcggtgccgtcgcaaacgcagtaagtattccacctggggagtacgttcgcaagaatgaaactcaaaggaattgacggggacccgcacaagcggtggagcatgtggtttaattcgaagcaacgcgaagaaccttaccaggtcttgacatcgatccgacgggggagtaacgtccccttcccttcggggcggagaagacaggtggtgcatggttgtcgtcagctcgtgtcgtgagatgttgggttaagtcccgcaacgagcgcaacccttattctaagtagccagcggttcggccgggaactcttgggagactgccagggataacctggaggaaggtggggatgacgtcaaatcatcatgccccttatgatctgggctacacacgtgctacaatggcgtaaacaaagagaagcaagaccgcgaggtggagcaaatctcaaaaataacgtctcagttcggactgcaggctgcaactcgcctgcacgaagctggaatcgctagtaatcgcgaatcagaatgtcgcggtgaatacgttcccgggtcttgtacacaccgcccgtcacaccatgggagtcagtaacgcccgaagtcagtgacccaaccgcaaggagggagctgccgaaggcgggaccgataactggggtgaagtcgtaacaaggtagccgtatcggaaggtgcggctggatcacctccttt

SEQ ID NO: 141 - DNA, 1531 bp, Artificial Sequence
  Synthetic Polynucleotide
atcagagagtttgatcctggctcaggatgaacgctggcggcgtgcttaacacatgcaagtcgagcgaagcacttaagtggatctcttcggattgaaacttatttgactgagcggcggacgggtgagtaacgcgtgggtaacctgcctcatacagggggataacagttagaaatggctgctaataccgcataagcgcacaggaccgcatggtctggtgtgaaaaactccggtggtatgagatggacccgcgtctgattagctagttggaggggtaacggcccaccaaggcgacgatcagtagccggcctgagagggtgaacggccacattgggactgagacacggcccagactcctacgggaggcagcagtggggaatattgcacaatgggggaaaccctgatgcagcgacgccgcgtgaaggaagaagtatctcggtatgtaaacttctatcagcagggaagaaaatgacggtacctgactaagaagccccggctaactacgtgccagcagccgcggtaatacgtagggggcaagcgttatccggatttactgggtgtaaagggagcgtagacggaagagcaagtctgatgtgaaaggctggggcttaaccccaggactgcattggaaactgtttttctagagtgccggagaggtaagcggaattcctagtgtagcggtgaaatgcgtagatattaggaggaacaccagtggcgaaggcggcttactggacggtaactgacgttgaggctcgaaagcgtggggagcaaacaggattagataccctggtagtccacgccgtaaacgatgaatactaggtgtcgggtggcaaagccattcggtgccgcagcaaacgcaataagtattccacctggggagtacgttcgcaagaatgaaactcaaaggaattgacggggacccgcacaagcggtggagcatgtggtttaattcgaagcaacgcgaagaaccttaccaagtcttgacatccctctgaccggcccgtaacggggccttcccttcggggcagaggagacaggtggtgcatggttgtcgtcagctcgtgtcgtgagatgttgggttaagtcccgcaacgagcgcaacccctatccttagtagccagcaggtgaagctgggcactctagggagactgccggggataacccggaggaaggcggggacgacgtcaaatcatcatgccccttatgatttgggctacacacgtgctacaatggcgtaaacaaagggaagcgagacagcgatgttgagcaaatcccaaaaataacgtcccagttcggactgcagtctgcaactcgactgcacgaagctggaatcgctagtaatcgcgaatcagaatgtcgcggtgaatacgttcccgggtcttgtacacaccgcccgtcacaccatgggagtcagtaacgcccgaagtcagtgacccaaccttttaggagggagctgccgaaggcgggaccgataactggggtgaagtcgtaacaaggtagccgtatcggaaggtgcggctggatcacctccttt

SEQ ID NO: 142 - DNA, 1531 bp, Artificial Sequence
  Synthetic Polynucleotide
atcagagagtttgatcctggctcaggatgaacgctggcggcgtgcttaacacatgcaagtcgagcgaagcacttaagtggatctcttcggattgaaacttatttgactgagcggcggacgggtgagtaacgcgtgggtaacctgcctcatacagggggataacagttagaaatggctgctaataccgcataagcgcacaggaccgcatggtctggtgtgaaaaactccggtggtatgagatggacccgcgtctgattagctagttggaggggtaacggcccaccaaggcgacgatcagtagccggcctgagagggtgaacggccacattgggactgagacacggcccagactcctacgggaggcagcagtggggaatattgcacaatgggggaaaccctgatgcagcgacgccgcgtgaaggaagaagtatctcggtatgtaaacttctatcagcagggaagaaaatgacggtacctgactaagaagccccggctaactacgtgccagcagccgcggtaatacgtagggggcaagcgttatccggatttactgggtgtaaagggagcgtagacggaagagcaagtctgatgtgaaaggctggggcttaaccccaggactgcattggaaactgtttttctagagtgccggagaggtaagtggaattcctagtgtagcggtgaaatgcgtagatattaggaggaacaccagtggcgaaggcggcttactggacggtaactgacgttgaggctcgaaagcgtggggagcaaacaggattagataccctggtagtccacgccgtaaacgatgaatactaggtgtcgggtggcaaagccattcggtgccgcagcaaacgcaataagtattccacctggggagtacgttcgcaagaatgaaactcaaaggaattgacggggacccgcacaagcggtggagcatgtggtttaattcgaagcaacgcgaagaaccttaccaagtcttgacatccctctgaccggcccgtaacggggccttcccttcggggcagaggagacaggtggtgcatggttgtcgtcagctcgtgtcgtgagatgttgggttaagtcccgcaacgagcgcaacccctatccttagtagccagcaggtgaagctgggcactctagggagactgccggggataacccggaggaaggcggggacgacgtcaaatcatcatgccccttatgatttgggctacacacgtgctacaatggcgtaaacaaagggaagcgggacagcgatgttgagcaaatcccaaaaataacgtcccagttcggactgcagtctgcaactcgactgcacgaagctggaatcgctagtaatcgcgaatcagaatgtcgcggtgaatacgttcccgggtcttgtacacaccgcccgtcacaccatgggagtcagtaacgcccgaagtcagtgacccaaccttacaggagggagctgccgaaggcgggaccgataactggggtgaagtcgtaacaaggtagccgtatcggaaggtgcggctggatcacctccttt

SEQ ID NO: 143 - DNA, 1531 bp, Artificial Sequence
  Synthetic Polynucleotide
atcagagagtttgatcctggctcaggatgaacgctggcggcgtgcttaacacatgcaagtcgagcgaagcacttaagtggatctcttcggattgaagcttatttgactgagcggcggacgggtgagtaacgcgtgggtaacctgcctcatacagggggataacagttagaaatggctgctaataccgcataagcgcacaggaccgcatggtctggtgtgaaaaactccggtggtatgagatggacccgcgtctgattagctagttggaggggtaacggcccaccaaggcgacgatcagtagccggcctgagagggtgaacggccacattgggactgagacacggcccagactcctacgggaggcagcagtggggaatattgcacaatgggggaaaccctgatgcagcgacgccgcgtgaaggaagaagtatctcggtatgtaaacttctatcagcagggaagaaaatgacggtacctgactaagaagccccggctaactacgtgccagcagccgcggtaatacgtagggggcaagcgttatccggatttactgggtgtaaagggagcgtagacggaagagcaagtctgatgtgaaaggctggggcttaaccccaggactgcattggaaactgtttttctagagtgccggagaggtaagcggaattcctagtgtagcggtgaaatgcgtagatattaggaggaacaccagtggcgaaggcggcttactggacggtaactgacgttgaggctcgaaagcgtggggagcaaacaggattagataccctggtagtccacgccgtaaacgatgaatactaggtgtcgggtggcaaagccattcggtgccgcagcaaacgcaataagtattccacctggggagtacgttcgcaagaatgaaactcaaaggaattgacggggacccgcacaagcggtggagcatgtggtttaattcgaagcaacgcgaagaaccttaccaagtcttgacatccctctgaccggcccgtaacggggccttcccttcggggcagaggagacaggtggtgcatggttgtcgtcagctcgtgtcgtgagatgttgggttaagtcccgcaacgagcgcaacccctatccttagtagccagcaggtgaagctgggcactctagggagactgccggggataacccggaggaaggcggggacgacgtcaaatcatcatgccccttatgatttgggctacacacgtgctacaatggcgtaaacaaagggaagcgagacagcgatgttgagcaaatcccaaaaataacgtcccagttcggactgcagtctgcaactcgactgcacgaagctggaatcgctagtaatcgcgaatcagaatgtcgcggtgaatacgttcccgggtcttgtacacaccgcccgtcacaccatgggagtcagtaacgcccgaagtcagtgacccaaccttacaggagggagctgccgaaggcgggaccgataactggggtgaagtcgtaacaaggtagccgtatcggaaggtgcggctggatcacctccttt

SEQ ID NO: 144 - DNA, 1531 bp, Artificial Sequence
  Synthetic Polynucleotide
atcagagagtttgatcctggctcaggatgaacgctggcggcgtgcttaacacatgcaagtcgagcgaagcacttaagcggatctcttcggattgaaacttatttgactgagcggcggacgggtgagtaacgcgtgggtaacctgcctcatacagggggataacagttagaaatggctgctaataccgcataagcgcacaggaccgcatggtctggtgtgaaaaactccggtggtatgagatggacccgcgtctgattagctagttggaggggtaacggcccaccaaggcgacgatcagtagccggcctgagagggtgaacggccacattgggactgagacacggcccagactcctacgggaggcagcagtggggaatattgcacaatgggggaaaccctgatgcagcgacgccgcgtgaaggaagaagtatctcggtatgtaaacttctatcagcagggaagaaaatgacggtacctgactaagaagccccggctaactacgtgccagcagccgcggtaatacgtagggggcaagcgttatccggatttactgggtgtaaagggagcgtagacggaagagcaagtctgatgtgaaaggctggggcttaaccccaggactgcattggaaactgtttttctagagtgccggagaggtaagcggaattcctagtgtagcggtgaaatgcgtagatattaggaggaacaccagtggcgaaggcggcttactggacggtaactgacgttgaggctcgaaagcgtggggagcaaacaggattagataccctggtagtccacgccgtaaacgatgaatactaggtgtcgggtggcaaagccattcggtgccgcagcaaacgcaataagtattccacctggggagtacgttcgcaagaatgaaactcaaaggaattgacggggacccgcacaagcggtggagcatgtggtttaattcgaagcaacgcgaagaaccttaccaagtcttgacatccctctgaccggcccgtaacggggccttcccttcggggcagaggagacaggtggtgcatggttgtcgtcagctcgtgtcgtgagatgttgggttaagtcccgcaacgagcgcaacccctatccttagtagccagcaggtgaagctgggcactctagggagactgccggggataacccggaggaaggcggggacgacgtcaaatcatcatgccccttatgatttgggctacacacgtgctacaatggcgtaaacaaagggaagcgagacagcgatgttgagcaaatcccaaaaataacgtcccagttcggactgcagtctgcaactcgactgcacgaagctggaatcgctagtaatcgcgaatcagaatgtcgcggtgaatacgttcccgggtcttgtacacaccgcccgtcacaccatgggagtcagtaacgcccgaagtcagtgacccaaccttacaggagggagctgccgaaggcgggaccgataactggggtgaagtcgtaacaaggtagccgtatcggaaggtgcggctggatcacctccttt

SEQ ID NO: 145 - DNA, 1531 bp, Artificial Sequence
  Synthetic Polynucleotide
atcagagagtttgatcctggctcaggatgaacgctggcggcgtgcttaacacatgcaagtcgagcgaagcacttaagtggatctcttcggattgaaacttatttgactgagcggcggacgggtgagtaacgcgtgggtaacctgcctcatacagggggataacagttagaaatggctgctaataccgcataagcgcacaggaccgcatggtctggtgtgaaaaactccggtggtatgagatggacccgcgtctgattagctagttggaggggtaacggcccaccaaggcgacgatcagtagccggcctgagagggtgaacggccacattgggactgagacacggcccagactcctacgggaggcagcagtggggaatattgcacaatgggggaaaccctgatgcagcgacgccgcgtgaaggaagaagtatctcggtatgtaaacttctatcagcagggaagaaaatgacggtacctgactaagaagccccggctaactacgtgccagcagccgcggtaatacgtagggggcaagcgttatccggatttactgggtgtaaagggagcgtagacggaagagcaagtctgatgtgaaaggctggggcttaaccccaggactgcattggaaactgtttttctagagtgccggagaggtaagcggaattcctagtgtagcggtgaaatgcgtagatattaggaggaacatcagtggcgaaggcggcttactggacggtaactgacgttgaggctcgaaagcgtggggagcaaacaggattagataccctggtagtccacgccgtaaacgatgaatactaggtgtcgggtggcaaagccattcggtgccgcagcaaacgcaataagtattccacctggggagtacgttcgcaagaatgaaactcaaaggaattgacggggacccgcacaagcggtggagcatgtggtttaattcgaagcaacgcgaagaaccttaccaagtcttgacatccctctgaccggcccgtaacggggccttcccttcggggcagaggagacaggtggtgcatggttgtcgtcagctcgtgtcgtgagatgttgggttaagtcccgcaacgagcgcaacccctatccttagtagccagcaggtgaagctgggcactctagggagactgccggggataacccggaggaaggcggggacgacgtcaaatcatcatgccccttatgatttgggctacacacgtgctacaatggcgtaaacaaagggaagcgagacagcgatgttgagcaaatcccaaaaataacgtcctagttcggactgcagtctgcaactcgactgcacgaagctggaatcgctagtaatcgcgaatcagaatgtcgcggtgaatacgttcccgggtcttgtacacaccgcccgtcacaccatgggagtcagtaacgcccgaagtcagtgacccaaccttacaggagggagctgccgaaggcgggaccgataactggggtgaagtcgtaacaaggtagccgtatcggaaggtgcggctggatcacctccttt

SEQ ID NO: 146 - DNA, 1529 bp, Artificial Sequence
  Synthetic Polynucleotide
aacgagagtttgatcctggctcaggatgaacgctggcggcgtgcttaacacatgcaagtcgagcgaagcacttaagtttgattcttcggatgaagacttttgtgactgagcggcggacgggtgagtaacgcgtgggtaacctgcctcatacagggggataacagttagaaatgactgctaataccgcataagaccacggtaccgcatggtacagtggtaaaaactccggtggtatgagatggacccgcgtctgattaggtagttggtggggtaacggcctaccaagccgacgatcagtagccgacctgagagggtgaccggccacattgggactgagacacggcccagactcctacgggaggcagcagtggggaatattgcacaatggaggaaactctgatgcagcgacgccgcgtgaaggatgaagtatttcggtatgtaaacttctatcagcagggaagaaaatgacggtacctgactaagaagccccggctaactacgtgccagcagccgcggtaatacgtagggggcaagcgttatccggatttactgggtgtaaagggagcgtagacggcacggcaagccagatgtgaaagcccggggctcaaccccgggactgcatttggaactgctgagctagagtgtcggagaggcaagtggaattcctagtgtagcggtgaaatgcgtagatattaggaggaacaccagtggcgaaggcggcttgctggacgatgactgacgttgaggctcgaaagcgtggggagcaaacaggattagataccctggtagtccacgccgtaaacgatgactgctaggtgtcgggtggcaaagccattcggtgccgcagctaacgcaataagcagtccacctggggagtacgttcgcaagaatgaaactcaaaggaattgacggggacccgcacaagcggtggagcatgtggtttaattcgaagcaacgcgaagaaccttacctgatcttgacatcccgatgaccgcttcgtaatggaagtttttcttcggaacatcggtgacaggtggtgcatggttgtcgtcagctcgtgtcgtgagatgttgggttaagtcccgcaacgagcgcaacccctatcttcagtagccagcaggttaagctgggcactctggagagactgccagggataacctggaggaaggtggggatgacgtcaaatcatcatgccccttatgaccagggctacacacgtgctacaatggcgtaaacaaagagaagcgaactcgcgagggtaagcaaatctcaaaaataacgtctcagttcggattgtagtctgcaactcgactacatgaagctggaatcgctagtaatcgcagatcagaatgctgcggtgaatacgttcccgggtcttgtacacaccgcccgtcacaccatgggagtcagtaacgcccgaagtcagtgacccaaccgtaaggagggagctgccgaaggtgggaccgataactggggtgaagtcgtaacaaggtagccgtatcggaaggtgcggctggatcacctccttt

SEQ ID NO: 147 - DNA, 1528 bp, Artificial Sequence
  Synthetic Polynucleotide
aacgagagtttgatcctggctcaggatgaacgctggcggcgtgcttaacacatgcaagtcgagcgaagcactttggaaagattcttcggatgatttcctttgtgactgagcggcggacgggtgagtaacgcgtgggtaacctgcctcatacagggggataacagttagaaatgactgctaataccgcataagaccacggtaccgcatggtacagtggtaaaaactccggtggtatgagatggacccgcgtctgattaggtagttggtggggtaacggcctaccaagccgacgatcagtagccgacctgagagggtgaccggccacattgggactgagacacggcccagactcctacgggaggcagcagtggggaatattgcacaatggaggaaactctgatgcagcgacgccgcgtgaaggatgaagtatttcggtatgtaaacttctatcagcagggaagaaaatgacggtacctgactaagaagccccggctaactacgtgccagcagccgcggtaatacgtagggggcaagcgttatccggatttactgggtgtaaagggagcgtagacggcacggcaagccagatgtgaaagcccggggctcaaccccggactgcatttggaactgctgagctagagtgtcggagaggcaagtggaattcctagtgtagcggtgaaatgcgtagatattaggaggaacaccagtggcgaaggcggcttgctggacgatgactgacgttgaggctcgaaagcgtggggagcaaacaggattagataccctggtagtccacgccgtaaacgatgactgctaggtgtcgggtggcaaagccattcggtgccgcagctaacgcaataagcagtccacctggggagtacgttcgcaagaatgaaactcaaaggaattgacggggacccgcacaagcggtggagcatgtggtttaattcgaagcaacgcgaagaaccttacctgatcttgacatcccgatgaccgcttcgtaatggaagcttttcttcggaacatcggtgacaggtggtgcatggttgtcgtcagctcgtgtcgtgagatgttgggttaagtcccgcaacgagcgcaacccctatcttcagtagccagcaggttaagctgggcactctggagagactgccagggataacctggaggaaggtggggatgacgtcaaatcatcatgccccttatgaccagggctacacacgtgctacaatggcgtaaacaaagagaagcgaactcgcgagggtaagcaaatctcaaaaataacgtctcagttcggattgtagtctgcaactcgactacatgaagctggaatcgctagtaatcgcagatcagaatgctgcggtgaatacgttcccgggtcttgtacacaccgcccgtcacaccatgggagtcagtaacgcccgaagtcagtgacccaaccgtaaggagggagctgccgaaggtgggaccgataactggggtgaagtcgtaacaaggtagccgtatcggaaggtgcggctggatcacctccttt

SEQ ID NO: 148 - DNA, 1529 bp, Artificial Sequence
  Synthetic Polynucleotide
aacgagagtttgatcctggctcaggatgaacgctggcggcgtgcttaacacatgcaagtcgagcgaagcacttaagtttgattcttcggatgaagacttttgtgactgagcggcggacgggtgagtaacgcgtgggtaacctgcctcatacagggggataacagttagaaatgactgctaataccgcataagaccacggtaccgcatggtacagtggtaaaaactccggtggtatgagatggacccgcgtctgattaggtagttggtggggtaacggcctaccaagccgacgatcagtagccgacctgagagggtgaccggccacattgggactgagacacggcccagactcctacgggaggcagcagtggggaatattgcacaatggaggaaactctgatgcagcgacgccgcgtgaaggatgaagtatttcggtatgtaaacttctatcagcagggaagaaaatgacggtacctgactaagaagccccggctaactacgtgccagcagccgcggtaatacgtagggggcaagcgttatccggatttactgggtgtaaagggagcgtagacggcacggcaagccagatgtgaaagcccggggctcaaccccgggactgcatttggaactgctgagctagagtgtcggagaggcaagtggaattcctagtgtagcggtgaaatgcgtagatattaggaggaacaccagtggcgaaggcggcttgctggacgatgactgacgttgaggctcgaaagcgtggggagcaaacaggattagataccctggtagtccacgccgtaaacgatgactgctaggtgtcgggtggcaaagccattcggtgccgcagctaacgcaataagcagtccacctggggagtacgttcgcaagaatgaaactcaaaggaattgacggggacccgcacaagcggtggagcatgtggtttaattcgaagcaacgcgaagaaccttacctgatcttgacatcccgatgaccgcttcgtaatggaagcttttcttcggaacatcggtgacaggtggtgcatggttgtcgtcagctcgtgtcgtgagatgttgggttaagtcccgcaacgagcgcaacccctatcttcagtagccagcaggttaagctgggcactctggagagactgccagggataacctggaggaaggtggggatgacgtcaaatcatcatgccccttatgaccagggctacacacgtgctacaatggcgtaaacaaagagaagcgaactcgcgagggtaagcaaatctcaaaaataacgtctcagttcggattgtagtctgcaactcgactacatgaagctggaatcgctagtaatcgcagatcagaatgctgcggtgaatacgttcccgggtcttgtacacaccgcccgtcacaccatgggagtcagtaacgcccgaagtcagtgacccaaccgtaaggagggagctgccgaaggtgggaccgataactggggtgaagtcgtaacaaggtagccgtatcggaaggtgcggctggatcacctccttt

SEQ ID NO: 149 - DNA, 1529 bp, Artificial Sequence
  Synthetic Polynucleotide
aacgagagtttgatcctggctcaggatgaacgctggcggcgtgcttaacacatgcaagtcgagcgaagcactttggaaagattcttcggatgatttcctttgtgactgagcggcggacgggtgagtaacgcgtgggtaacctgcctcatacagggggataacagttagaaatgactgctaataccgcataagaccacggtaccgcatggtacagtggtaaaaactccggtggtatgagatggacccgcgtctgattaggtagttggtggggtaacggcctaccaagccgacgatcagtagccgacctgagagggtgaccggccacattgggactgagacacggcccagactcctacgggaggcagcagtggggaatattgcacaatggaggaaactctgatgcagcgacgccgcgtgaaggatgaagtatttcggtatgtaaacttctatcagcagggaagaaaatgacggtacctgactaagaagccccggctaactacgtgccagcagccgcggtaatacgtagggggcaagcgttatccggatttactgggtgtaaagggagcgtagacggcacggcaagccagatgtgaaagcccggggctcaaccccgggactgcatttggaactgctgagctagagtgtcggagaggcaagtggaattcctagtgtagcggtgaaatgcgtagatattaggaggaacaccagtggcgaaggcggcttgctggacgatgactgacgttgaggctcgaaagcgtggggagcaaacaggattagataccctggtagtccacgccgtaaacgatgactgctaggtgtcgggtggcaaagccattcggtgccgcagctaacgcaataagcagtccacctggggagtacgttcgcaagaatgaaactcaaaggaattgacggggacccgcacaagcggtggagcatgtggtttaattcgaagcaacgcgaagaaccttacctgatcttgacatcccgatgaccgcttcgtaatggaagcttttcttcggaacatcggtgacaggtggtgcatggttgtcgtcagctcgtgtcgtgagatgttgggttaagtcccgcaacgagcgcaacccctatcttcagtagccagcaggttaagctgggcactctggagagactgccagggataacctggaggaaggtggggatgacgtcaaatcatcatgccccttatgaccagggctacacacgtgctacaatggcgtaaacaaagagaagcgaactcgcgagggtaagcaaatctcaaaaataacgtctcagttcggattgtagtctgcaactcgactacatgaagctggaatcgctagtaatcgcagatcagaatgctgcggtgaatacgttcccgggtcttgtacacaccgcccgtcacaccatgggagtcagtaacgcccgaagtcagtgacccaaccgtaaggagggagctgccgaaggtgggaccgataactggggtgaagtcgtaacaaggtagccgtatcggaaggtgcggctggatcacctccttt

SEQ ID NO: 150 - DNA, 1528 bp, Artificial Sequence
  Synthetic Polynucleotide
aacgagagtttgatcctggctcaggatgaacgctggcggcgtgcttaacacatgcaagtcgagcgaagcgcttaagtttgattcttcggatgaagacttttgtgactgagcggcggacgggtgagtaacgcgtgggtaacctgcctcatacagggggataacagttagaaatgactgctaataccgcataagaccacggtaccgcatggtacagtggtaaaaactccggtggtatgagatggacccgcgtctgattaggtagttggtggggtaacggcctaccaagccgacgatcagtagccgacctgagagggtgaccggccacattgggactgagacacggcccagactcctacgggaggcagcagtggggaatattgcacaatggaggaaactctgatgcagcgacgccgcgtgaaggatgaagtatttcggtatgtaaacttctatcagcagggaagaaaatgacggtacctgactaagaagccccggctaactacgtgccagcagccgcggtaatacgtagggggcaagcgttatccggatttactgggtgtaaagggagcgtagacggcacggcaagccagatgtgaaagcccgggctcaaccccgggactgcatttggaactgctgagctagagtgtcggagaggcaagtggaattcctagtgtagcggtgaaatgcgtagatattaggaggaacaccagtggcgaaggcggcttgctggacgatgactgacgttgaggctcgaaagcgtggggagcaaacaggattagataccctggtagtccacgccgtaaacgatgactgctaggtgtcgggtggcaaagccattcggtgccgcagctaacgcaataagcagtccacctggggagtacgttcgcaagaatgaaactcaaaggaattgacggggacccgcacaagcggtggagcatgtggtttaattcgaagcaacgcgaagaaccttacctgatcttgacatcccgatgaccgcttcgtaatggaagtttttcttcggaacatcggtgacaggtggtgcatggttgtcgtcagctcgtgtcgtgagatgttgggttaagtcccgcaacgagcgcaacccctatcttcagtagccagcaggttaagctgggcactctggagagactgccagggataacctggaggaaggtggggatgacgtcaaatcatcatgccccttatgaccagggctacacacgtgctacaatggcgtaaacaaagagaggcaaactcgcgagggtaagcaaatctcaaaaataacgtctcagttcggattgtagtctgcaactcgactacatgaagctggaatcgctagtaatcgcagatcagaatgctgcggtgaatacgttcccgggtcttgtacacaccgcccgtcacaccatgggagtcagtaacgcccgaagtcagtgacccaaccgtaaggagggagctgccgaaggtgggaccgataactggggtgaagtcgtaacaaggtagccgtatcggaaggtgcggctggatcacctccttt

SEQ ID NO: 151 - DNA, 1529 bp, Artificial Sequence
  Synthetic Polynucleotide
aacgagagtttgatcctggctcaggatgaacgctggcggcgtgcttaacacatgcaagtcgagcgaagcgctttgggaagattcttcggatgatttcctttgtgactgagcggcggacgggtgagtaacgcgtgggtaacctgcctcatacagggggataacagttagaaatgactgctaataccgcataagaccacggtaccgcatggtacagtggtaaaaactccggtggtatgagatggacccgcgtttgattaggtagttggtggggtaacggcctaccaagccgacgatcagtagccgacctgagagggtgaccggccacattgggactgagacacggcccagactcctacgggaggcagcagtggggaatattgcacaatggaggaaactctgatgcagcgacgccgcgtgaaggatgaagtatttcggtatgtaaacttctatcagcagggaagaaaatgacggtacctgactaagaagccccggctaactacgtgccagcagccgcggtaatacgtagggggcaagcgttatccggatttactgggtgtaaagggagcgtagacggcacggcaagccagatgtgaaagcccggggctcaaccccgggactgcatttggaactgctgagctagagtgtcggagaggcaagtggaattcctagtgtagcggtgaaatgcgtagatattaggaggaacaccagtggcgaaggcggcttgctggacgatgactgacgttgaggctcgaaagcgtggggagcaaacaggattagataccctggtagtccacgccgtaaacgatgactgctaggtgtcgggtggcaaagccattcggtgccgcagctaacgcaataagcagtccacctggggagtacgttcgcaagaatgaaactcaaaggaattgacggggacccgcacaagcggtggagcatgtggtttaattcgaagcaacgcgaagaaccttacctgatcttgacatcccgatgactgcttcgtaatggaagtttttcttcggaacatcggtgacaggtggtgcatggttgtcgtcagctcgtgtcgtgagatgttgggttaagtcccgcaacgagcgcaacccctatcttcagtagccagcaggttaagctgggcactctggagagactgccagggataacctggaggaaggtggggatgacgtcaaatcatcatgccccttatgaccagggctacacacgtgctacaatggcgtaaacaaagagaagcgaactcgcgagggtaagcaaatctcaaaaataacgtctcagttcggattgtagtctgcaactcgactacatgaagctggaatcgctagtaatcgcagatcagaatgctgcggtgaatacgttcccgggtcttgtacacaccgcccgtcacaccatgggagtcagtaacgcccgaagtcagtgacccaaccgtaaggagggagctgccgaaggtgggaccgataactggggtgaagtcgtaacaaggtagccgtatcggaaggtgcggctggatcacctccttt

SEQ ID NO: 152 - DNA, 1537 bp, Artificial Sequence
  Synthetic Polynucleotide
atggagagtttgatcctggctcaggatgaacgctggcggcatgcctaatacatgcaagtcgaacgaagtttcgaggaagcttgcttccaaagagacttagtggcgaacgggtgagtaacacgtaggtaacctgcccatgtgtccgggataactgctggaaacggtagctaaaaccggataggtatacagagcgcatgctcagtatattaaagcgcccatcaaggcgtgaacatggatggacctgcggcgcattagctagttggtgaggtaacggctcaccaaggcgatgatgcgtagccggcctgagagggtaaacggccacattgggactgagacacggcccaaactcctacgggaggcagcagtagggaattttcgtcaatgggggaaaccctgaacgagcaatgccgcgtgagtgaagaaggtcttcggatcgtaaagctctgttgtaagtgaagaacggctcatagaggaaatgctatgggagtgacggtagcttaccagaaagccacggctaactacgtgccagcagccgcggtaatacgtaggtggcaagcgttatccggaatcattgggcgtaaagggtgcgtaggtggcgtactaagtctgtagtaaaaggcaatggctcaaccattgtaagctatggaaactggtatgctggagtgcagaagagggcgatggaattccatgtgtagcggtaaaatgcgtagatatatggaggaacaccagtggcgaaggcggtcgcctggtctgtaactgacactgaggcacgaaagcgtggggagcaaataggattagataccctagtagtccacgccgtaaacgatgagaactaagtgttggaggaattcagtgctgcagttaacgcaataagttctccgcctggggagtatgcacgcaagtgtgaaactcaaaggaattgacgggggcccgcacaagcggtggagtatgtggtttaattcgaagcaacgcgaagaaccttaccaggccttgacatggaaacaaataccctagagatagggggataattatggatcacacaggtggtgcatggttgtcgtcagctcgtgtcgtgagatgttgggttaagtcccgcaacgagcgcaacccttgtcgcatgttaccagcatcaagttggggactcatgcgagactgccggtgacaaaccggaggaaggtggggatgacgtcaaatcatcatgccccttatggcctgggctacacacgtactacaatggcggccacaaagagcagcgacacagtgatgtgaagcgaatctcataaaggtcgtctcagttcggattgaagtctgcaactcgacttcatgaagtcggaatcgctagtaatcgcagatcagcatgctgcggtgaatacgttctcgggccttgtacacaccgcccgtcaaaccatgggagtcagtaatacccgaagccggtggcataaccgtaaggagtgagccgtcgaaggtaggaccgatgactggggttaagtcgtaacaaggtatccctacgggaacgtggggatggatcacctccttt

SEQ ID NO: 153 - DNA, 1537 bp, Artificial Sequence; identical to SEQ ID NO: 21
  Synthetic Polynucleotide

SEQ ID NO: 154 - DNA, 1537 bp, Artificial Sequence; identical to SEQ ID NO: 152
  Synthetic Polynucleotide

SEQ ID NO: 155 - DNA, 1537 bp, Artificial Sequence
  Synthetic Polynucleotide
atggagagtttgatcctggctcaggatgaacgctggcggcatgcctaatacatgcaagtcgaacgaagtttcgaggaagcttgcttccaaagagacttagtggcgaacgggtgagtaacacgtaggtaacctgcccatgtgtccgggataactgctggaaacggtagctaaaaccggataggtatacagagcgcatgctcagtatattaaagcgcccatcaaggcgtgaacatggatggacctgcggcgcattagctagttggtgaggtaacggcccaccaaggcgatgatgcgtagccggcctgagagggtaaacggccacattgggactgagacacggcccaaactcctacgggaggcagcagtagggaattttcgtcaatgggggaaaccctgaacgagcaatgccgcgtgagtgaagaaggtcttcggatcgtaaagctctgttgtaagtgaagaacggctcatagaggaaatgctatgggagtgacggtagcttaccagaaagccacggctaactacgtgccagcagccgcggtaatacgtaggtggcaagcgttatccggaatcattgggcgtaaagggtgcgtaggtggcgtactaagtctgtagtaaaaggcaatggctcaaccattgtaagctatggaaactggtatgctggagtgcagaagagggcgatggaattccatgtgtagcggtaaaatgcgtagatatatggaggaacaccagtggcgaaggcggtcgcctggtctgtaactgacactgaggcacgaaagcgtggggagcaaataggattagataccctagtagtccacgccgtaaacgatgagaactaagtgttggaggaattcagtgctgcagttaacgcaataagttctccgcctggggagtatgcacgcaagtgtgaaactcaaaggaattgacgggggcccgcacaagcggtggagtatgtggtttaattcgaagcaacgcgaagaaccttaccaggccttgacatggaaacaaataccctagagatagggggataattatggatcacacaggtggtgcatggttgtcgtcagctcgtgtcgtgagatgttgggttaagtcccgcaacgagcgcaacccttgtcgcatgttaccagcatcaagttggggactcatgcgagactgccggtgacaaaccggaggaaggtggggatgacgtcaaatcatcatgccccttatggcctgggctacacacgtactacaatggcgaccacaaagagcagcgacacagtgatgtgaagcgaatctcataaaggtcgtctcagttcggattgaagtctgcaactcgacttcatgaagtcggaatcgctagtaatcgcagatcagcatgctgcggtgaatacgttctcgggccttgtacacaccgcccgtcaaaccatgggagtcagtaatacccgaagccggtggcataaccgcaaggagtgagccgtcgaaggtaggaccgatgactggggttaagtcgtaacaaggtatccctacgggaacgtggggatggatcacctccttt

SEQ ID NO: 156 - DNA, 1537 bp, Artificial Sequence; identical to SEQ ID NO: 21
  Synthetic Polynucleotide

SEQ ID NO: 157 - DNA, 1529 bp, Artificial Sequence
  Synthetic Polynucleotide
tattgagagtttgatcctggctcaggatgaacgctggcggcgtgcttaacacatgcaagtcgaacggggtgctcatgacggaggattcgtccaacggattgagttacctagtggcggacgggtgagtaacgcgtgaggaacctgccttggagaggggaataacactccgaaaggagtgctaataccgcatgatgcagttgggtcgcatggctctgactgccaaagatttatcgctctgagatggcctcgcgtctgattagctagtaggcggggtaacggcccacctaggcgacgatcagtagccggactgagaggttgaccggccacattgggactgagacacggcccagactcctacgggaggcagcagtggggaatattgggcaatgggcgcaagcctgacccagcaacgccgcgtgaaggaagaaggctttcgggttgtaaacttcttttgtcggggacgaaacaaatgacggtacccgacgaataagccacggctaactacgtgccagcagccgcggtaatacgtaggtggcaagcgttatccggatttactgggtgtaaagggcgtgtaggcgggattgcaagtcagatgtgaaaactgggggctcaacctccagcctgcatttgaaactgtagttcttgagtgctggagaggcaatcggaattccgtgtgtagcggtgaaatgcgtagatatacggaggaacaccagtggcgaaggcggattgctggacagtaactgacgctgaggcgcgaaagcgtggggagcaaacaggattagataccctggtagtccacgccgtaaacgatggatactaggtgtgggggtctgaccccctccgtgccgcagttaacacaataagtatcccacctggggagtacgatcgcaaggttgaaactcaaaggaattgacgggggcccgcacaagcggtggagtatgtggtttaattcgaagcaacgcgaagaaccttaccagggcttgacatcccactaacgaagcagagatgcattaggtgcccttcggggaaagtggagacaggtggtgcatggttgtcgtcagctcgtgtcgtgagatgttgggttaagtcccgcaacgagcgcaacccttattgttagttgctacgcaagagcactctagcgagactgccgttgacaaaacggaggaaggtggggacgacgtcaaatcatcatgccccttatgtcctgggccacacacgtactacaatggtggttaacagagggaggcaataccgcgaggtggagcaaatccctaaaagccatcccagttcggattgcaggctgaaacccgcctgtatgaagttggaatcgctagtaatcgcggatcagcatgccgcggtgaatacgttcccgggccttgtacacaccgcccgtcacaccatgagagtcgggaacacccgaagtccgtagcctaaccgcaaggagggcgcggccgaaggtgggttcgataattggggtgaagtcgtaacaaggtagccgtatcggaaggtgcggctggatcacctccttt

SEQ ID NO: 158 - DNA, 1530 bp, Artificial Sequence
  Synthetic Polynucleotide
tattgagagtttgatcctggctcaggatgaacgctggcggcgtgcttaacacatgcaagtcgaacggggtgctcatgacggaggattcgtccaacggattgagttacctagtggcggacgggtgagtaacgcgtgaggaacctgccttggagaggggaataacactccgaaaggagtgctaataccgcatgatgcagttgggtcgcatggctctgactgccaaagatttatcgctctgagatggcctcgcgtctgattagctagtaggcggggtaacggcccacctaggcgacgatcagtagccggactgagaggttgaccggccacattgggactgagacacggcccagactcctacgggaggcagcagtggggaatattgggcaatgggcgcaagcctgacccagcaacgccgcgtgaaggaagaaggctttcgggttgtaaacttcttttgtcggggacgaaacaaatgacggtacccgacgaataagccacggctaactacgtgccagcagccgcggtaatacgtaggtggcaagcgttatccggatttactgggtgtaaagggcgtgtaggcgggattgcaagtcagatgtgaaaactgggggctcaacctccagcctgcatttgaaactgtagttcttgagtgctggagaggcaatcggaattccgtgtgtagcggtgaaatgcgtagatatacggaggaacaccagtggcgaaggcggattgctggacagtaactgacgctgaggcgcgaaagcgtggggagcaaacaggattagataccctggtagtccacgccgtaaacgatggatactaggtgtggggggtctgaccccctccgtgccgcagttaacacaataagtatcccacctggggagtacgatcgcaaggttgaaactcaaaggaattgacgggggcccgcacaagcggtggagtatgtggtttaattcgaagcaacgcgaagaaccttaccagggcttgacatcccactaacgaagcagagatgcattaggtgcccttcggggaaagtggagacaggtggtgcatggttgtcgtcagctcgtgtcgtgagatgttgggttaagtcccgcaacgagcgcaacccttattgttagttgctacgcaagagcactctagcgagactgccgttgacaaaacggaggaaggtggggacgacgtcaaatcatcatgccccttatgtcctgggccacacacgtactacaatggtggttaacagagggaggcaataccgcgaggtggagcaaatccctaaaagccatcccagttcggattgcaggctgaaacccgcctgtatgaagttggaatcgctagtaatcgcggatcagcatgccgcggtgaatacgttcccgggccttgtacacaccgcccgtcacaccatgagagtcgggaacacccgaagtccgtagcctaaccgcaaggagggcgcggccgaaggtgggttcgataattggggtgaagtcgtaacaaggtagccgtatcggaaggtgcggctggatcacctccttt

SEQ ID NO: 159 - DNA, 1529 bp, Artificial Sequence
  Synthetic Polynucleotide
tattgagagtttgatcctggctcaggatgaacgctggcggcgtgcttaacacatgcaagtcgaacggggtgctcatgacggaggattcgtccaacggattgagttacctagtggcggacgggtgagtaacgcgtgaggaacctgccttggagaggggaataacactccgaaaggagtgctaataccgcataatgcagttgggtcgcatggctctgactgccaaagatttatcgctctgagatggcctcgcgtctgattagctagtaggcggggtaacggcccacctaggcgacgatcagtagccggactgagaggttgaccggccacattgggactgagacacggcccagactcctacgggaggcagcagtggggaatattgggcaatgggcgcaagcctgacccagcaacgccgcgtgaaggaagaaggctttcgggttgtaaacttcttttgtcagggacgaaacaaatgacggtacctgacgaataagccacggctaactacgtgccagcagccgcggtaatacgtaggtggcaagcgttatccggatttactgggtgtaaagggcgtgtaggcgggattgcaagtcagatgtgaaaactgggggctcaacctccagcctgcatttgaaactgtagttcttgagtgctggagaggcaatcggaattccgtgtgtagcggtgaaatgcgtagatatacggaggaacaccagtggcgaaggcggattgctggacagtaactgacgctgaggcgcgaaagcgtggggagcaaacaggattagataccctggtagtccacgccgtaaacgatggatactaggtgtggggggtctgacccctccgtgccgcagttaacacaataagtatcccacctggggagtacgatcgcaaggttgaaactcaaaggaattgacgggggcccgcacaagcggtggagtatgtggtttaattcgaagcaacgcgaagaaccttaccagggcttgacatcccactaacgaagcagagatgcattaggtgcccttcggggaaagtggagacaggtggtgcatggttgtcgtcagctcgtgtcgtgagatgttgggttaagtcccgcaacgagcgcaacccttattgttagttgctacgcaagagcactctagcgagactgccgttgacaaaacggaggaaggtggggacgacgtcaaatcatcatgccccttatgtcctgggccacacacgtactacaatggtggttaacagagggaggcaataccgcgaggtggagcaaatccctaaaagccatcccagttcggattgcaggctgaaacccgcctgtatgaagttggaatcgctagtaatcgcggatcagcatgccgcggtgaatacgttcccgggccttgtacacaccgcccgtcacaccatgagagtcgggaacacccgaagtccgtagcctaaccgcaaggagggcgcggccgaaggtgggttcgataattggggtgaagtcgtaacaaggtagccgtatcggaaggtgcggctggatcacctccttt